European Patent Application EP 4 231 016 A1, published August 23, 2023. Title: Genetically controlled nanoscopy contrast-generating units, genetically controlled structural elements, genetically controlled scaffolds, nanobionaterial based thereon, and use thereof in nanoscopy methods. Applicant: Westmeyer, Gil Gregor Helmholtz Zentrum München - Deutsches Forschungszentrum für Gesundheit und Umwelt GmbH Piovesan, Alberto. The sequence listing filed with the application follows.

SEQUENCE LISTING (239 sequences)

SEQ ID NO: 1 - protein, 68 aa, Mus musculus
MDPETCPCPTGGSCTCSDKCKCKGCKCTNCKKSCCSCCPAGCEKCAKDCVCKGEEGAKAEAEKCSCCQ

SEQ ID NO: 2 - protein, 74 aa, Mus musculus
HHHHHHMDPETCPCPTGGSCTCSDKCKCKGCKCTNCKKSCCSCCPAGCEKCAKDCVCKGEEGAKAEAEKCSCCQ

SEQ ID NO: 3 - protein, 77 aa, Mus musculus
HHHHHHHHHMDPETCPCPTGGSCTCSDKCKCKGCKCTNCKKSCCSCCPAGCEKCAKDCVCKGEEGAKAEAEKCSCCQ

SEQ ID NO: 4 - protein, 147 aa, Mus musculus
MDPETCPCPTGGSCTCSDKCKCKGCKCTNCKKSCCSCCPAGCEKCAKDCVCKGEEGAKAEAEKCSCCQGGGSGGGSGGSADPETCPCPTGGSCTCSDKCKCKGCKCTNCKKSCCSCCPAGCEKCAKDCVCKGEEGAKAEAEKCSCCQ

SEQ ID NO: 5 - protein, 214 aa, Artificial Sequence
  cimeric metallothionein
MDPETCPCPTGGSCTCSDKCKCKGCKCTNCKKSCCSCCPAGCEKCAKDCVCKGEEGAKAEAEKCSCCQGGTGGSTSTTLVKCACEPCLCNVDPSKAIDRNGLYYCSEACADGHTGGSKGCGHTGCNCHGSAGGCDDKCGCAVPCPGGTGCRCTSARSGAAAGEHTTCGCGEHCGCNPCACGREGTPSGRANRRANCSCGAACNCASCGSATAPG

SEQ ID NO: 6 - protein, 300 aa, Pinctada fucata
MKFLAAVAFVAVLSHSTVYSYGPRNRGKMMPMMPPAKKMMNNDMMKMMKPDDAMMKPDKQNQMKPDDMKQMMKMMMDKMMMMDKMMMMDMMMKMMKPDMMMKPDMMMKPDMMMKPDMMMKPDMMMKPDMMMKPDMMMKPDMMMKPDMMMKPDMMMKPDMMMKPDMMMKPDMMMKPDMMMKPDMMMKPDMMMKPDMMMKPDMMMKPDMMMKPDMMMKPDMMMKPDMMMKPDMMMKPDMMMKPDMMMKPDMMMKPDMMMKPDMMMKPDMMMKPDMMMKPDMGMMKPDMGMMMHPTPYNLYQG

SEQ ID NO: 7 - protein, 31 aa, Panax ginseng
CKSGGAWCGFDPHGCCGNCGCLVGFCYGTGC

SEQ ID NO: 8 - protein, 28 aa, Klebsiella pneumoniae
ECPRCDSYYTLHQAQHHLRCHHCDSQRP

SEQ ID NO: 9 - protein, 26 aa, Homo sapiens
EAVCCSDHQHCCPQGYTCVAEGQCQK

SEQ ID NO: 10 - protein, 45 aa, Utricina eques
CYPGQPGCGHCSRPNYCEGARCESGFHDCGSDHWCDASGDRCCCA

SEQ ID NO: 11 - protein, 27 aa, Homo sapiens
LMVKCPNEGCLHKMELRHLEDHQAHCE

SEQ ID NO: 12 - protein, 111 aa, Methylobacterium extorquens
PTTTTKVDIAAFDPDKDGTIDLKEALAAGSAAFDKLDPDKDGTLDAKELKGRVSEADLKKLDPDNDGTLDKKEYLAAVEAQFKAANPDNDGTIDARELASPAGSALVNLIR

SEQ ID NO: 13 - protein, 20 aa, Artificial Sequence
  Synthethic lanthanide binding tag
FIDTNNDGWIEGDELLLEEG

SEQ ID NO: 14 - protein, 119 aa, Ascidia sydneiensis samea
SKVIFALVLVVVLVACINATYVEFEEAYAPVDCKGQCTTPCEPLTACKEKCAESCETSADKKTCRRNCKKADCEPQDKVCDACRMKCHKACRAANCASECPKHEHKSDTCRACMKTNCK

SEQ ID NO: 15 - protein, 88 aa, Escherichia coli
NEHHHETMSEAQPQVISATGEVKGIDLESKKITIHHDPIAAVNWPEMTMRFTITPQTKMSEIKTGDKVAFNFVQQGNLSLLQDIKVSQ

SEQ ID NO: 16 - protein, 10 aa, Artificial Sequence
  Encapsulation signal for the Encapsulin system of Quasibacillus thermotolerans
KGFTVGSLIQ

SEQ ID NO: 17 - protein, 298 aa, Plasmodium falciparum
FNNNLCSKNAKGLNLNKRLLHETQAHVDDAHHAHHVADAHHAHHVADAHHAHHVADAHHAHHAADAHHAHHAADAHHAHHAADAHHAHHAHHAADAHHAHHAADAHHAHHAADAHHAHHAADAHHAHHAADAHHAHHASDAHHAHHAAYAHHAHHASDAHHAADAHHAAYAHHAHHAADAHHAADAHHATDAHHAADAHHAADAHHAADAHHATDAHHAHHAADAHHATDAHHAHHAADAHHAAAHHATDAHHAAAHHATDAHHAAAHHEAATHCLRHGGGGSGGGGSKGFTVGSLIQ

SEQ ID NO: 18 - protein, 212 aa, Artificial Sequence
  Fusion protein consisting of enhanced UnaG(V2L) from Anguilla japonica and MmMT3
MLEKFVGTWKIADSHNFGEYLKAIGAPKELSDGGDATTPTLYISQKDGDKMSVKIENGPPTFLDTQVKFKLGEEFDEFPSDRRKGVKSVVNLVGEKLVYVQKWDGKETTYVREIKDGKLVVTLTMGDVVAVRSYRRATEGGTGGSDPETCPCPTGGSCTCSDKCKCKGCKCTNCKKSCCSCCPAGCEKCAKDCVCKGEEGAKAEAEKCSCCQ

SEQ ID NO: 19 - protein, 182 aa, Homo sapiens
MDKDCEMKRTTLDSPLGKLELSGCEQGLHRIIFLGKGTSAADAVEVPAPAAVLGGPEPLMQATAWLNAYFHQPEAIEEFPVPALHHPVFQQESFTRQVLWKLLKVVKFGEVISYSHLAALAGNPAATAAVKTALSGNPVPILIPCHRVVQGDLDVGGYEGGLAVKEWLLAHEGHRLGKPGLG

SEQ ID NO: 20 - protein, 297 aa, Artificial Sequence
  modified bacterial dehalogenase that forms covalent bonds with chloroalkane derivatives
MAEIGTGFPFDPHYVEVLGERMHYVDVGPRDGTPVLFLHGNPTSSYVWRNIIPHVAPTHRCIAPDLIGMGKSDKPDLGYFFDDHVRFMDAFIEALGLEEVVLVIHDWGSALGFHWAKRNPERVKGIAFMEFIRPIPTWDEWPEFARETFQAFRTTDVGRKLIIDQNVFIEGTLPMGVVRPLTEVEMDHYREPFLNPVDREPLWRFPNELPIAGEPANIVALVEEYMDWLHQSPVPKLLFWGTPGVLIPPAEAARLAKSLPNCKAVDIGPGLNLLQEDNPDLIGSEIARWLSTLEISG

SEQ ID NO: 21 - protein, 404 aa, Artificial Sequence
  Fusion of a synthetic coiled-coil domain (P2), the CGU MmMT3, the QtEnc shell-forming monomer from the Encapsulin system of Q.thermotolerans and a FLAG-epitope
MSPEDKIAQLKEKNAALKEKNQQLKEKIQALKYGGGTGGSDPETCPCPTGGSCTCSDKCKCKGCKCTNCKKSCCSCCPAGCEKCAKDCVCKGEEGAKAEAEKCSCCQGSGPGNKSQLYPDSPLTDQDFNQLDQTVIEAARRQLVGRRFIELYGPLGRGMQSVFNDIFMESHEAKMDFQGSFDTEVESSRRVNYTIPMLYKDFVLYWRDLEQSKALDIPIDFSVAANAARDVAFLEDQMIFHGSKEFDIPGLMNVKGRLTHLIGNWYESGNAFQDIVEARNKLLEMNHNGPYALVLSPELYSLLHRVHKDTNVLEIEHVRELITAGVFQSPVLKGKSGVIVNTGRNNLDLAISEDFETAYLGEEGMNHPFRVYETVVLRIKRPAAICTLIDPEEGSGDYKDDDDK

SEQ ID NO: 22 - protein, 333 aa, Artificial Sequence
  Fusion of synthetic coiled-coil domain P1 (cognate partner of P2), OsO4 post-fixation stable switchable fluorescent protein mEosEM and a human PEST degradation sequence
MVSAIKPDMRIKLRMEGNVNGHHFVIDGEGTGKPYEGKQTMDLEVKEGGPLPFAFDILTTAFHYGNRVFVKYPDNIQDYFKQSFPKGYSWERSMTFEDGGICNARNDITMEGDTFYNKVRFYGTNFPANGPVMQKKTLKWEPSTEKMYVRDGVLTGDIEMALLLEGGAHYRCDFRTTYKAKEKGVKLPGAHFVDHAIEILSHDKDYNKVKLYEHAVAHSGLPDNARRGGGGSGGGGSGPGTGSPEDEIQALEEENAQLEQENAALEEEIAQLEYGSGSETPGTSESATPESAISHGFPPEVEEQAAGTLPMSCAQESGMDRHPAACASARINV

SEQ ID NO: 23 - protein, 195 aa, Artificial Sequence
  Strand 1 to 9 of a Tripartite split superfolderGFP
MRGEELFTGVVPILIELDGDVNGHKFFVRGEGEGDATIGKLSLKFICTTGKLPVPWPTLVTTLTYGVQCFSRYPDHMKRHDFFKSAMPEGYVQERTIYFKDDGTYKTRAEVKFEGDTLVNRIELKGIDFKEDGNILGHKLEYNFNSHKVYITADKQNNGIKANFTIRHNVEDGSVQLADHYQQNTPIGDGPVLLP

SEQ ID NO: 24 - protein, 487 aa, Artificial Sequence
  The shell forming monomer of the Ecapsulin system of Quasibacillus thermotolerans fused to superfolder GFP strands 1 to 9
MNKSQLYPDSPLTDQDFNQLDQTVIEAARRQLVGRRFIELYGPLGRGMQSVFNDIFMESHEAKMDFQGSFDTEVESSRRVNYTIPMLYKDFVLYWRDLEQSKALDIPIDFSVAANAARDVAFLEDQMIFHGSKEFDIPGLMNVKGRLTHLIGNWYESGNAFQDIVEARNKLLEMNHNGPYALVLSPELYSLLHRVHKDTNVLEIEHVRELITAGVFQSPVLKGKSGVIVNTGRNNLDLAISEDFETAYLGEEGMNHPFRVYETVVLRIKRPAAICTLIDPEEGGGGSGPGGSGMRGEELFTGVVPILIELDGDVNGHKFFVRGEGEGDATIGKLSLKFICTTGKLPVPWPTLVTTLTYGVQCFSRYPDHMKRHDFFKSAMPEGYVQERTIYFKDDGTYKTRAEVKFEGDTLVNRIELKGIDFKEDGNILGHKLEYNFNSHKVYITADKQNNGIKANFTIRHNVEDGSVQLADHYQQNTPIGDGPVLL

SEQ ID NO: 25 - protein, 313 aa, Artificial Sequence
  The shell forming monomer of the Ecapsulin system of Quasibacillus thermotolerans fused to superfolderGFP strand 10
MNKSQLYPDSPLTDQDFNQLDQTVIEAARRQLVGRRFIELYGPLGRGMQSVFNDIFMESHEAKMDFQGSFDTEVESSRRVNYTIPMLYKDFVLYWRDLEQSKALDIPIDFSVAANAARDVAFLEDQMIFHGSKEFDIPGLMNVKGRLTHLIGNWYESGNAFQDIVEARNKLLEMNHNGPYALVLSPELYSLLHRVHKDTNVLEIEHVRELITAGVFQSPVLKGKSGVIVNTGRNNLDLAISEDFETAYLGEEGMNHPFRVYETVVLRIKRPAAICTLIDPEEGGGGSGPGGSGTMDLPDNHYLSTQTILLKDL

SEQ ID NO: 26 - protein, 315 aa, Artificial Sequence
  The shell forming monomer of the Ecapsulin system of Quasibacillus thermotolerans fused to superfolderGFP strand 11
MNKSQLYPDSPLTDQDFNQLDQTVIEAARRQLVGRRFIELYGPLGRGMQSVFNDIFMESHEAKMDFQGSFDTEVESSRRVNYTIPMLYKDFVLYWRDLEQSKALDIPIDFSVAANAARDVAFLEDQMIFHGSKEFDIPGLMNVKGRLTHLIGNWYESGNAFQDIVEARNKLLEMNHNGPYALVLSPELYSLLHRVHKDTNVLEIEHVRELITAGVFQSPVLKGKSGVIVNTGRNNLDLAISEDFETAYLGEEGMNHPFRVYETVVLRIKRPAAICTLIDPEEGGGGSGPGGSGSEKRDHMVLLEYVTAAGITDAS

SEQ ID NO: 27 - protein, 432 aa, Artificial Sequence
  The shell forming monomer of the Ecapsulin system of Quasibacillus thermotolerans fused to enhanced UnaG(V2L) from Anguilla japonica and MmMT3
MNKSQLYPDSPLTDQDFNQLDQTVIEAARRQLVGRRFIELYGPLGRGMQSVFNDIFMESHEAKMDFQGSFDTEVESSRRVNYTIPMLYKDFVLYWRDLEQSKALDIPIDFSVAANAARDVAFLEDQMIFHGSKEFDIPGLMNVKGRLTHLIGNWYESGNAFQDIVEARNKLLEMNHNGPYALVLSPELYSLLHRVHKDTNVLEIEHVRELITAGVFQSPVLKGKSGVIVNTGRNNLDLAISEDFETAYLGEEGMNHPFRVYETVVLRIKRPAAICTLIDPEEGGGGSGPGGSGMLEKFVGTWKIADSHNFGEYLKAIGAPKELSDGGDATTPTLYISQKDGDKMSVKIENGPPTFLDTQVKFKLGEEFDEFPSDRRKGVKSVVNLVGEKLVYVQKWDGKETTYVREIKDGKLVVTLTMGDVVAVRSYRRATE

SEQ ID NO: 28 - protein, 437 aa, Artificial Sequence
  The shell forming monomer of the Ecapsulin system of Myxococcus xanthus fused to enhanced UnaG(V2L) from Anguilla japonica and MmMT3
MADFLGHAENPLREEEWARLNETVIQVARRSLVGRRILDIYGPLGAGVQTVPYDEFQGVSPGAVDIVGEQETAMVFTDARKFKTIPIIYKDFLLHWRDIEAARTHNMPLDVSAAAGAAALCAQQEDELIFYGDARLGYEGLMTANGRLTVPLGDWTSPGGGFQAIVEATRKLNEQGHFGPYAVVLSPRLYSQLHRIYEKTGVLEIETIRQLASDGVYQSNRLRGESGVVVSTGRENMDLAVSMDMVAAYLGASRMNHPFRVLEALLLRIKHPDAICTLEGAGATERRGGGGSGPGGSGMLEKFVGTWKIADSHNFGEYLKAIGAPKELSDGGDATTPTLYISQKDGDKMSVKIENGPPTFLDTQVKFKLGEEFDEFPSDRRKGVKSVVNLVGEKLVYVQKWDGKETTYVREIKDGKLVVTLTMGDVVAVRSYRRATE

SEQ ID NO: 29 - protein, 456 aa, Artificial Sequence
  Heme domain of BM3 a natural fusion protein constructed of cytochrome P450 and NADPH-cytochrome P450 reductase domains from Priestia megaterium
MTIKEMPQPKTFGELKNLPLLNTDKPVQALMKIADELGEIFKFEAPGRVTRYLSSQRLIKEACDESRFDKNLSQALKFVRDFAGDGLFTSWTHEKNWKKAHNILLPSFSQQAMKGYHAMMVDIAVQLVQKWERLNADEHIEVPEDMTRLTLDTIGLCGFNYRFNSFYRDQPHPFITSMVRALDEAMNKLQRANPDDPAYDENKRQFQEDIKVMNDLVDKIIADRKASGEQSDDLLTHMLNGKDPETGEPLDDENIRYQIITFLIAGHETTSGLLSFALYFLVKNPHVLQKAAEEAARVLVDPVPSYKQVKQLKYVGMVLNEALRLWPTAPAFSLYAKEDTVLGGEYPLEKGDELMVLIPQLHRDKTIWGDDVEEFRPERFENPSAIPQHAFKPFGNGQRACIGQQFALHEATLVLGMMLKHFDFEDHTNYELDIKETLTLKPEGFVVKAKSKKIPL

SEQ ID NO: 30 - protein, 127 aa, Homo sapiens
MSFSGKYQLQSQENFEAFMKAIGLPEELIQKGKDIKGVSEIVQNGKHFKFTITAGSKVIQNEFTVGEECELETMTGEKVKTVVQLEGDNKLVTTFKNIKSVTELNGDIITNTMTLGDIVFKRISKRI

SEQ ID NO: 31 - protein, 132 aa, Homo sapiens
MAFDSTWKVDRSENYDKFMEKMGVNIVKRKLAAHDNLKLTITQEGNKFTVKESSAFRNIEVVFELGVTFNYNLADGTELRGTWSLEGNKLIGKFKRTDNGNELNTVREIIGDELVQTYVYEGVEAKRIFKKD

SEQ ID NO: 32 - protein, 133 aa, Homo sapiens [sequence omitted]

SEQ ID NO: 33 - protein, 132 aa, Homo sapiens
MCDAFVGTWKLVSSENFDDYMKEVGVGFATRKVAGMAKPNMIISVNGDVITIKSESTFKNTEISFILGQEFDEVTADDRKVKSTITLDGGVLVHVQKWDGKSTTIKRKREDDKLVVECVMKGVTSTRVYERA

SEQ ID NO: 34 - protein, 135 aa, Homo sapiens
MATVQQLEGRWRLVDSKGFDEYMKELGVGIALRKMGAMAKPDCIITCDGKNLTIKTESTLKTTQFSCTLGEKFEETTADGRKTQTVCNFTDGALVQHQEWDGKESTITRKLKDGKLVVECVMNNVTCTRIYEKVE

SEQ ID NO: 35 - protein, 128 aa, Homo sapiens
MAFTGKFEMESEKNYDEFMKLLGISSDVIEKARNFKIVTEVQQDGQDFTWSQHYSGGHTMTNKFTVGKESNIQTMGGKTFKATVQMEGGKLVVNFPNYHQTSEIVGDKLVEVSTIGGVTYERVSKRLA

SEQ ID NO: 36 - protein, 132 aa, Homo sapiens
MVEAFCATWKLTNSQNFDEYMKALGVGFATRQVGNVTKPTVIISQEGDKVVIRTLSTFKNTEISFQLGEEFDETTADDRNCKSVVSLDGDKLVHIQKWDGKETNFVREIKDGKMVMTLTFGDVVAVRHYEKA

SEQ ID NO: 37 - protein, 132 aa, Homo sapiens
MSNKFLGTWKLVSSENFDDYMKALGVGLATRKLGNLAKPTVIISKKGDIITIRTESTFKNTEISFKLGQEFEETTADNRKTKSIVTLQRGSLNQVQRWDGKETTIKRKLVNGKMVAECKMKGVVCTRIYEKV

SEQ ID NO: 38 - protein, 132 aa, Homo sapiens
MVEPFLGTWKLVSSENFEDYMKELGVNFAARNMAGLVKPTVTISVDGKMMTIRTESSFQDTKISFKLGEEFDETTADNRKVKSTITLENGSMIHVQKWLGKETTIKRKIVDEKMVVECKMNNIVSTRIYEKV

SEQ ID NO: 39 - protein, 140 aa, Homo sapiens
MIDQLQGTWKSISCENSEDYMKELGIGRASRKLGRLAKPTVTISTDGDVITIKTKSIFKNNEISFKLGEEFEEITPGGHKTKSKVTLDKESLIQVQDWDGKETTITRKLVDGKMVVESTVNSVICTRTYEKVSSNSVSNS

SEQ ID NO: 40 - protein, 10 aa, Rattus rattus
GCMSCKCVLS

SEQ ID NO: 41 - protein, 36 aa, Rattus norvegicus
CGLCVCPCNKLKSSDAYKKAWGNNQDGVVASQPARV

SEQ ID NO: 42 - protein, 15 aa, Homo sapiens
MGCVQCKDKEATKLT

SEQ ID NO: 43 - protein, 121 aa, Mus musculus
MPSDRPFKQRRSFADRCKEVQQIRDQHPSKIPVIIERYKGEKQLPVLDKTKFLVPDHVNMSELVKIIRRRLQLNPTQAFFLLVNQHSMVSVSTPIADIYEQEKDEDGFLYMVYASQETFGF

SEQ ID NO: 44 - protein, 338 aa, Artificial Sequence
  Consisting of engineered apo-lipoprotein A-1 (MSP1) flanked by DnaE split intein fragments C-intein (AA 103-137) on the N-term and N-Intein (AA 1-102) on the C-term) (Homo sapiens, Nostoc punctiforme):
MIKIATRKYLGKQNVYDIGVGEPHNFALKNGFIASNLKLLDNWDSVTSTFSKLREQLGPVTQEFWDNLEKETEGLRQEMSKDLEEVKAKVQPYLDDFQKKWQEEMELYRQKVEPLRAELQEGARQKLHELQEKLSPLGEEMRDRARAHVDALRTHLAPYSDELRQRLAARLEALKENGGARLAEYHAKATEHLSTLSEKAKPALEDLRQGLLPVLESFKVSFLSALEEYTKKLNTQCLSYETEILTVEYGLLPIGKIVEKRIECTVYSVDNNGNIYTQPVAQWHDRGEQEVFEYCLEDGSLIRATKDHKFMTVDGQMLPIDEIFERELDLMRVDNLPN

SEQ ID NO: 45 - protein, 139 aa, Artificial Sequence
  Designed uranyl binding proteins with 6 binding sites for uranyl ions
MVSRLEERVRDLEAEVDKLRERLDRLEETVQAKGGGGSGGGGSGGGGSGGGGSGGVSRLERVRDLEAEVDKLRERLDRLEETVQAKGGGGSGGGGSGGGGSGGGGSGGVSRLEERVRDLAEVDKLRERLDRLEETVQAK

SEQ ID NO: 46 - protein, 220 aa, Artificial Sequence
  Designed uranyl binding proteins with 6 binding sites for uranyl ions
MQLEDKVEELLSKVYHLENEVDRLRKLIENKGGGGSGGGGSQLEDKVEELESEVDHLRNEVAKKLVGGGGSGGGGSQLEDKVEELLSKVYHLENEVDRLRKLIENKGGGGSGGGGSQLEDKVEELESEVDHLRNEVARLKKLVGGGGSGGGGSQLEDKVEELLSKVYHLENEVDRLRKLIENKGGGGSGGGGSQLEDKVEELESEVDHLRNEVARLKKLV

SEQ ID NO: 47 - protein, 435 aa, Artificial Sequence
  Degron-tagged polyphopsphate kinase 2b of Corynebacterium glutamicum C-terminanlly tagged with the encapsulation signal of Quasibacillus thermotolerans
GVQVETISPGDGRTFPKRGQTCVVHYTGMLEDGKKVDSSRDRNKPFKFMLGKQEVIRGWEEGVAQMSVGQRAKLTISPDYAYGATGHPGIIPPHATLVFDVELLKPEGSGVGKLPIMAETNENDLPVIDLAQIEGYVVDDSDEDDPVLLRPDGTPIETWREDFPYEERVTREDYEKVKRSLQIELLKWQNWTKETGQRHIILFEGRDAAGKGGTIKRFNEHLNPRGARTVALEKPSPRESTSWYFQRYIQHFPAAGEIVFFDRSWYNRSGVERVMGFCTESQHAEFLREVPMLENMILGSGISLTKFWFSVTRKEQRTRFAIRQVDPVRQWKLSPMDLASLDRWDDYTRAKEEQFRYTDTDESPWITIKSNDKKRARINAMRYVLSKFDYTDKDYELVGEPDPKVVLRGRDQIGDGGGGSGGGGSKGFTVGSLIQ

SEQ ID NO: 48 - protein, 305 aa, Corynebacterium glutamicum
VGKLPIMAETNENDLPVIDLAQIEGYVVDDSDEDDPVLLRPDGTPIETWREDFPYEERVTREDYEKVKRSLQIELLKWQNWTKETGQRHIILFEGRDAAGKGGTIKRFNEHLNPRGARTVALEKPSPRESTSWYFQRYIQHFPAAGEIVFFDRSWYNRSGVERVMGFCTESQHAEFLREVPMLENMILGSGISLTKFWFSVTRKEQRTRFAIRQVDPVRQWKLSPMDLASLDRWDDYTRAKEEQFRYTDTDESPWITIKSNDKKRARINAMRYVLSKFDYTDKDYELVGEPDPKVVLRGRDQIGD

SEQ ID NO: 49 - protein, 469 aa, Artificial Sequence
  Phytochelatin synthase 1 of Arabidopsis thaliana with a C-terminal encapsulation signal
MEGFFRLISYFQTQSEPAYCGLASLSVVLNALSIDPGRKWKGPWRWFDESMLDCCEPLEVVKEKGISFGKVVCLAHCSGAKVEAFRTSQSTIDDFRKFVVKCTSSENCHMISTYHRGVFKQTGTGHFSPIGGYNAERDMALILDVARFKYPPHWVPLKLLWEAMDSIDQSTGKRRGFMLISRPHREPGLLYTLSCKDESWIEIAKYLKEDVPRLVSSQHVDSVEKIISVVFKSLPSNFNQFIRWVAEIRITEDSNQNLSAEEKSRLKLKQLVLKEVHETELFKHINKFLSTVGYEDSLTYAAAKACCQGAEILSGSPSKEFCCRETCVKCIKGPDDSEGTVVTGVVVRDGNEQKVDLLVPSTQTECECGPEATYPAGNDVFTALLLALPPQTWSGIKDQALMHEMKQLISMASLPTLLQEEVLHLRRQLQLLKRCQENKEEDDLAAPAYGGGGSGGGGSKGFTVGSLIQ

SEQ ID NO: 50 - protein, 472 aa, Artificial Sequence
  Phytochelatin synthase 2 of Arabidopsis thaliana with a C-terminal encapsulation signal
MSMASLYRRSLSPPAIDFASFEGKQIFNEALQKGTMEGFFGLISYFQTQSEPAFCGLASLSMVLNSLSIDPGRKWKGPWRWFDESMLECCEPLEIVKDKGISFGKVVCLAHSSGAKVEAFRTNQSTIDDFRKYVVKCSTSDNCHMISTYHRQVLKQTGTGHFSPIGGYNAERDMALILDVARFKYPPHWVPLKLLWDAMDSIDQSTGRRRGFMLISRPHREPGLLYTLSCKDESWISIAKYLKEDVPRLVSSQHVDTIERILYVVFKSLPANFNQFIKWMAEIRRTEDVNQNLSSEEKSRLKLKQELLKQVQETKLFKHVDKFLSSVYEDNLPYVAAKVYCDGDEILSGYESDESCCKETCVKCIKGLGEEKVTVVAYPSGNDVFTALLLALPPQTWSGIKDQSLLQEMKQLISMVSHPTLLQQEVLHLRRQLEMLKRCQENKEDEELSAPAGGGGSGGGGSKGFTVGSLIQ

SEQ ID NO: 51 - protein, 296 aa, Bacillus megaterium
SNKYRVRKNVLHLTDTEKRDFVRTVLILKEKGIYDRYIAWHGAAGKFHTPPGSDRNAAHMSSAFLPWHREYLLRFERDLQSINPEVTLPYWEWETDAQMQDPSQSQIWSADFMGGNGNPIKDFIVDTGPFAAGRWTTIDEQGNPSGGLKRNFGATKEAPTLPTRDDVLNALKITQYDTPPWDMTSQNSFRNQLEGFINGPQLHNRVHRWVGGQMGVVPTAPNDPVFFLHHANVDRIWAVWQIIHRNQNYQPMKNGPFGQNFRDPMYPWNTTPEDVMNHRKLGYVYDIELRKSKRSS

SEQ ID NO: 52 - protein, 192 aa, Quasibacillus thermotolerans
MKEELDAFHQIFTTTKEAIERFMAMLTPVIENAEDDHERLYYHHIYEEEEQRLSRLDVLIPLIEKFQDETDEGLFSPSNNAFNRLLQELNLEKFGLHNFIEHVDLALFSFTDEERQTLLKELRKDAYEGYQYVKEKLAEINARFDHDYADPHAHHDEHRDHLADMPSAGSSHEEVQPVAHKKKGFTVGSLIQ

SEQ ID NO: 53 - protein, 128 aa, Bacteriophage Pseudomonas phage
MSKTIVLSVGEATRTLTEIQSTADRQIFEEKVGPLVGRLRLTASLRQNGAKTAYRVNLKLDQADVVDCSTSVCGELPKVRYTQVWSHDVTIVANSTEASRKSLYDLTKSLVATSQVEDLVVNLVPLGR

SEQ ID NO: 54 - protein, 255 aa, Artificial Sequence
  Tandem dimer of The coat protein of the single-stranded RNA bacteriophage Pseudomonas phage binding the PP7 stem loop
MLASKTIVLSVGEATRTLTEIQSTADRQIFEEKVGPLVGRLRLTASLRQNGAKTAYRVNLKLDQADVVDSGLPKVRYTQVWSHDVTIVANSTEASRKSLYDLTKSLVATSQVEDLVVNLVPLGRADPLASKTIVLSVGEATRTLTEIQSTADRQIFEEKVGPLVGRLRLTASLRQNGAKTAYRVNLKLDQADVVDSGLPKVRYTQVWSHDVTIVANSTEASRKSLYDLTKSLVATSQVEDLVVNLVPLGRPPVAT

SEQ ID NO: 55 - RNA, 98 nt, Artificial Sequence
  Synthetically derived RNA aptamer designed to be an RNA mimic of green fluorescent protein (GFP)
gacgcaacugaaugaaauggugaaggacggguccagguguggcugcuucggcagugcagcuuguugaguagagugugagcuccguaacuagucgcguc

SEQ ID NO: 56 - RNA, 25 nt, Artificial Sequence
  Small RNA sequence binding partner of the tandem PCP dimer from Pseudomonas phage
ggagcagacgauauggcgucgcucc

SEQ ID NO: 57 - RNA, 57 nt, Artificial Sequence
  Synthetically derived RNA aptamer designed to be an RNA mimic of red fluorescent protein (RFP)
ggaugcgccuugaaaagccugcuucggcagcuggugaaugacagcuauggcgcaucc

SEQ ID NO: 58 - RNA, 19 nt, Artificial Sequence
  Small synthetic aptamer coordination metal ions in homodimeric form
uugucgcuucgaaaaaguc

SEQ ID NO: 59 - RNA, 55 nt, Artificial Sequence
  Synthetic aptamer that binds a fluorogenic rhodamine dye with fast association and dissociation kinetics
ccuuggacuccgccaauuggaacgcggagaggaaguggcgaaagcgccuccaagg

SEQ ID NO: 60 - protein, 85 aa, Artificial Sequence
  RNA-binding domain that are known to bind single-stranded RNAs. It was found in many eukaryotic proteins
GSMATTKRVLYVGGLAEEVDDKVLHAAFIPFGDITDIQIPLDYETEKHRGFAFVEFELAEDAAAAIDNMNESELFGRTIRVNLAK

SEQ ID NO: 61 - protein, 78 aa, Artificial Sequence
  Protein domain that was first identified in the human binds RNA, and can function in RNA recognition
MSPNLPGQTTVQVRVPYRVVGLVVGPKGATIKRIQQQTHTYIVTPSRDKEPVFEVTGMPENVDRAREEIEMHIAMRTG

SEQ ID NO: 62 - protein, 87 aa, Artificial Sequence
  Zinc finger domain subspecies know to bind RNA
MSGGLAPSKSTVYVSNLPFSLTNNDLYRIFSKYGKVVKVTIMKDKDTRKSKGVAFILFLDKDSAQNCTRAINNKQLFGRVIKASIAI

SEQ ID NO: 63 - protein, 127 aa, Artificial Sequence
  Multifunctional RNA-binding protein that recognizes the K-turn motif in ribosomal RNA
MSKASYVKFEVPQDLADKVLEAVRKAKESGKIKKGTNETTKAVERGQAKLVIIAEDVQPEEIVAHLPLLCDEKKIPYVYVSSKKALGEACGLQVATASAAILEPGEAKDLVDEIIKRVNEIKGKTSS

SEQ ID NO: 64 - protein, 17 aa, Artificial Sequence
  BIV-Tat from the Bovine immunodeficiency virus  binds to a hairpin structure at the 5'-end of all nascent viral mRNAs
SGPRPRGTRGKGRRIRR

SEQ ID NO: 65 - protein, 281 aa, Quasibacillus thermotolerans
NKSQLYPDSPLTDQDFNQLDQTVIEAARRQLVGRRFIELYGPLGRGMQSVFNDIFMESHEAKMDFQGSFDTEVESSRRVNYTIPMLYKDFVLYWRDLEQSKALDIPIDFSVAANAARDVAFLEDQMIFHGSKEFDIPGLMNVKGRLTHLIGNWYESGNAFQDIVEARNKLLEMNHNGPYALVLSPELYSLLHRVHKDTNVLEIEHVRELITAGVFQSPVLKGKSGVIVNTGRNNLDLAISEDFETAYLGEEGMNHPFRVYETVVLRIKRPAAICTLIDPEE

SEQ ID NO: 66 - protein, 287 aa, Myxococcus xanthus
MADFLGHAENPLREEEWARLNETVIQVARRSLVGRRILDIYGPLGAGVQTVPYDEFQGVSPGAVDIVGEQETAMVFTDARKFKTIPIIYKDFLLHWRDIEAARTHNMPLDVSAAAGAAALCAQQEDELIFYGDARLGYEGLMTANGRLTVPLGDWTSPGGGFQAIVEATRKLNEQGHFGPYAVVLSPRLYSQLHRIYEKTGVLEIETIRQLASDGVYQSNRLRGESGVVVSTGRENMDLAVSMDMVAAYLGASRMNHPFRVLEALLLRIKHPDAICTLEGAGATERR

SEQ ID NO: 67 - protein, 264 aa, Thermotoga maritima
MEFLKRSFAPLTEKQWQEIDNRAREIFKTQLYGRKFVDVEGPYGWEYAAHPLGEVEVLSDENEVVKWGLRKSLPLIELRATFTLDLWELDNLERGKPNVDLSSLEETVRKVAEFEDEVIFRGCEKSGVKGLLSFEERKIECGSTPKDLLEAIVRALSIFSKDGIEGPYTLVINTDRWINFLKEEAGHYPLEKRVEECLRGGKIITTPRIEDALVVSERGGDFKLILGQDLSIGYEDREKDAVRLFITETFTFQVVNPEALILLK

SEQ ID NO: 68 - protein, 33 aa, Artificial Sequence
  Synthetic coiled-coil domain which pairs with P2
SPEDEIQALEEENAQLEQENAALEEEIAQLEYG

SEQ ID NO: 69 - protein, 33 aa, Artificial Sequence
  Synthetic coiled-coil domain which pairs with P1
SPEDKIAQLKEKNAALKEKNQQLKEKIQALKYG

SEQ ID NO: 70 - protein, 33 aa, Artificial Sequence
  Synthetic coiled-coil domain which pairs with P4
SPEDEIQQLEEEIAQLEQKNAALKEKNQALKYG

SEQ ID NO: 71 - protein, 33 aa, Artificial Sequence
  Synthetic coiled-coil domain which pairs with P3
SPEDKIAQLKQKIQALKQENQQLEEENAALEYG

SEQ ID NO: 72 - protein, 78 aa, Artificial Sequence
  Synthetic coiled-coil domain which pairs DHD13b
MGTKEDILERQRKIIERAQEIHRRQQEILEELERIIRKPGSSEEAMKRMLKLLEESLRLLKELLELSEESAQLLYEQR

SEQ ID NO: 73 - protein, 83 aa, Artificial Sequence
  Synthetic coiled-coil domain which pairs DHD13a
GTEKRLLEEAERAHREQKEIIKKAQELHRRLEEIVRQSGSSEEAKKEAKKILEEIRELSKRSLELLREILYLSQEQKGSLVPR

SEQ ID NO: 74 - DNA, 16 bp, Artificial Sequence
  engineered DNA sequence promoting ribosomal(translational) read-through after a STOP codon
ctaggcgctcgaagat

SEQ ID NO: 75 - RNA, 15 nt, Artificial Sequence
  engineered RNA motif binding to L7Ae
ccugauuggugaggg

SEQ ID NO: 76 - DNA, 24 bp, Artificial Sequence
  engineered DNA sequence promoting ribosomal(translational) read-through after a STOP codon
caattagctcatccagacattccg

SEQ ID NO: 77 - protein, 861 aa, Rattus norvegicus
MATEEAIIRIPPYHYIHVLDQNSNVSRVEVGPKTYIRQDNERVLFAPVRMVTVPPRHYCIVANPVSRDTQSSVLFDITGQVRLRHADQEIRLAQDPFPLYPGEVLEKDITPLQVVLPNTALHLKALLDFEDKNGDKVMAGDEWLFEGPGTYIPQKEVEVVEIIQATVIKQNQALRLRARKECFDREGKGRVTGEEWLVRSVGAYLPAVFEEVLDLVDAVILTEKTALHLRALQNFRDLRGVLHRTGEEWLVTVQDTEAHVPDVYEEVLGVVPITTLGPRHYCVILDPMGPDGKNQLGQKRVVKGEKSFFLQPGERLERGIQDVYVLSEQQGLLLKALQPLEEGESEEKVSHQAGDCWLIRGPLEYVPSAKVEVVEERQAIPLDQNEGIYVQDVKTGKVRAVIGSTYMLTQDEVLWEKELPSGVEELLNLGHDPLADRGQKGTAKPLQPSAPRNKTRVVSYRVPHNAAVQVYDYRAKRARVVFGPELVTLDPEEQFTVLSLSAGRPKRPHARRALCLLLGPDFFTDVITIETADHARLQLQLAYNWHFELKNRNDPAEAAKLFSVPDFVGDACKAIASRVRGAVASVTFDDFHKNSARIIRMAVFGFEMSEDTGPDGTLLPKARDQAVFPQNGLVVSSVDVQSVEPVDQRTRDALQRSVQLAIEITTNSQEAAAKHEAQRLEQEARGRLERQKILDQSEAEKARKELLELEAMSMAVESTGNAKAEAESRAEAARIEGEGSVLQAKLKAQALAIETEAELERVKKVREMELIYARAQLELEVSKAQQLANVEAKKFKEMTEALGPGTIRDLAVAGPEMQVKLLQSLGLKSTLITDGSSPINLFSTAFGLLGLGSDGQPPAQK

SEQ ID NO: 78 - protein, 978 aa, Artificial Sequence
  Vault forming protein from Rattus norvegicus with SNAP25-derived palmitoylation signal (AA 85-120) inserted in helix-loop-helix region
MATEEAIIRIPPYHYIHVLDQNSNVSRVEVGPKTYIRQDNERVLFAPVRMVTVPPRHYCIVANPVSRDTQSSVLFDITGQVRLRHADQEIRLAQDPFPLYPGEVLEKDITPLQVVLPNTALHLKALLDFEDKNGDKVMAGDEWLFEGPGTYIPQKEVEVVEIIQATVIKQNQALRLRARKECFDREGKGRVTGEEWLVRSVGAYLPAVFEEVLDLVDAVILTEKTALHLRALQNFRDLRGVLHRTGEEWLVTVQDTEAHVPDVYEEVLGVVPITTLGPRHYCVILDPMGPDGKNQLGQKRVVKGEKSFFLQPGERLERGIQDVYVLSEQQGLLLKALQPLEEGESEEKVSHQAGDCWLIRGPLEYVPSAKVEVVEERQAIPLDQNEGIYVQDVKTGKVRAVIGSTYMLTQDEVLWEKELPSGVEELLNLGHDPLADRGQKGTAKPLQPSAPRNKTRVVSYRVPHNAAVQVYDYRAKRARVVFGPELVTLDPEEQFTVLSLSAGRPKRPHARRALCLLLGPDFFTDVITIETADHARLQLQLAYNWHFELKNRNDPAEAAKLFSVPDFVGDACKAIASRVRGAVASVTFDDFHKNSARIIRMAVFGFEGSPEDELAANEEELQQNEQKLAQIKQKLQAIKYGGGGSGGGGSGGGGCGLCVCPCNKLKSSDAYKKAWGNNQDGVVASQPARVGGGGSGGGGSGGGGSPEDEIQQLEEEIAQLEQKNAALKEKNQALKYGKARDQAVFPQNGLVVSSVDVQSVEPVDQRTRDALQRSVQLAIEITTNSQEAAAKHEAQRLEQEARGRLERQKILDQSEAEKARKELLELEAMSMAVESTGNAKAEAESRAEAARIEGEGSVLQAKLKAQALAIETEAELERVKKVREMELIYARAQLELEVSKAQQLANVEAKKFKEMTEALGPGTIRDLAVAGPEMQVKLLQSLGLKSTLITDGSSPINLFSTAFGLLGLGSDGQPPAQK

SEQ ID NO: 79 - protein, 996 aa, Artificial Sequence
  Vault forming protein from Rattus norvegicus with aniparallel coiled-coil domain inserted into helix-loop-helix region
MATEEAIIRIPPYHYIHVLDQNSNVSRVEVGPKTYIRQDNERVLFAPVRMVTVPPRHYCIVANPVSRDTQSSVLFDITGQVRLRHADQEIRLAQDPFPLYPGEVLEKDITPLQVVLPNTALHLKALLDFEDKNGDKVMAGDEWLFEGPGTYIPQKEVEVVEIIQATVIKQNQALRLRARKECFDREGKGRVTGEEWLVRSVGAYLPAVFEEVLDLVDAVILTEKTALHLRALQNFRDLRGVLHRTGEEWLVTVQDTEAHVPDVYEEVLGVVPITTLGPRHYCVILDPMGPDGKNQLGQKRVVKGEKSFFLQPGERLERGIQDVYVLSEQQGLLLKALQPLEEGESEEKVSHQAGDCWLIRGPLEYVPSAKVEVVEERQAIPLDQNEGIYVQDVKTGKVRAVIGSTYMLTQDEVLWEKELPSGVEELLNLGHDPLADRGQKGTAKPLQPSAPRNKTRVVSYRVPHNAAVQVYDYRAKRARVVFGPELVTLDPEEQFTVLSLSAGRPKRPHARRALCLLLGPDFFTDVITIETADHARLQLQLAYNWHFELKNRNDPAEAAKLFSVPDFVGDACKAIASRVRGAVASVTFDDFHKNSARIIRMAVFGFEGSPEDELAANEEELQQNEQKLAQIKQKLQAIKYGGGGSGGGGSGGGGSGGGGKQLEKELKQLEKELQAIEKQLAQLQWKAQARKKKLAQLKKKLQAGGGGSGGGGSGGGGSGGGGSPEDEIQQLEEEIAQLEQKNAALKEKNQALKYGKARDQAVFPQNGLVVSSVDVQSVEPVDQRTRDALQRSVQLAIEITTNSQEAAAKHEAQRLEQEARGRLERQKILDQSEAEKARKELLELEAMSMAVESTGNAKAEAESRAEAARIEGEGSVLQAKLKAQALAIETEAELERVKKVREMELIYARAQLELEVSKAQQLANVEAKKFKEMTEALGPGTIRDLAVAGPEMQVKLLQSLGLKSTLITDGSSPINLFSTAFGLLGLGSDGQPPAQK

SEQ ID NO: 80 - protein, 978 aa, Artificial Sequence
  Vault forming protein from Rattus norvegicus with a shortened aniparallel coiled-coil domain inserted into helix-loop-helix region
MATEEAIIRIPPYHYIHVLDQNSNVSRVEVGPKTYIRQDNERVLFAPVRMVTVPPRHYCIVANPVSRDTQSSVLFDITGQVRLRHADQEIRLAQDPFPLYPGEVLEKDITPLQVVLPNTALHLKALLDFEDKNGDKVMAGDEWLFEGPGTYIPQKEVEVVEIIQATVIKQNQALRLRARKECFDREGKGRVTGEEWLVRSVGAYLPAVFEEVLDLVDAVILTEKTALHLRALQNFRDLRGVLHRTGEEWLVTVQDTEAHVPDVYEEVLGVVPITTLGPRHYCVILDPMGPDGKNQLGQKRVVKGEKSFFLQPGERLERGIQDVYVLSEQQGLLLKALQPLEEGESEEKVSHQAGDCWLIRGPLEYVPSAKVEVVEERQAIPLDQNEGIYVQDVKTGKVRAVIGSTYMLTQDEVLWEKELPSGVEELLNLGHDPLADRGQKGTAKPLQPSAPRNKTRVVSYRVPHNAAVQVYDYRAKRARVVFGPELVTLDPEEQFTVLSLSAGRPKRPHARRALCLLLGPDFFTDVITIETADHARLQLQLAYNWHFELKNRNDPAEAAKLFSVPDFVGDACKAIASRVRGAVASVTFDDFHKNSARIIRMAVFGFEGSPEDELAANEEELQQNEQKLAQIKQKLQAIKYGGGGSGGGGSGGGGKELKQLEKELQAIEKQLAQLQWKAQARKKKLAQLKKGGGGSGGGGSGGGGSPEDEIQQLEEEIAQLEQKNAALKEKNQALKYGKARDQAVFPQNGLVVSSVDVQSVEPVDQRTRDALQRSVQLAIEITTNSQEAAAKHEAQRLEQEARGRLERQKILDQSEAEKARKELLELEAMSMAVESTGNAKAEAESRAEAARIEGEGSVLQAKLKAQALAIETEAELERVKKVREMELIYARAQLELEVSKAQQLANVEAKKFKEMTEALGPGTIRDLAVAGPEMQVKLLQSLGLKSTLITDGSSPINLFSTAFGLLGLGSDGQPPAQK

SEQ ID NO: 81 - protein, 1255 aa, Artificial Sequence
  TEV protease inducible Vault based on caged Gp41-1 split inteins, Version 1
MATEEAIIRIPPYHYIHVLDQNSNVSRVEVGPKTYIRQDNERVLFAPVRMVTVPPRHYCIVANPVSRDTQSSVLFDITGQVRLRHADQEIRLAQDPFPLYPGEVLEKDITPLQVVLPNTALHLKALLDFEDKNGDKVMAGDEWLFEGPGTYIPQKEVEVVEIIQATVIKQNQALRLRARKECFDREGKGRVTGEEWLVRSVGAYLPAVFEEVLDLVDAVILTEKTALHLRALQNFRDLRGVLHRTGEEWLVTVQDTEAHVPDVYEEVLGVVPITTLGPRHYCVILDPMGPDGKNQLGQKRVVKGEKSFFLQPGERLERGIQDVYVLSEQQGLLLKALQPLEEGESEEKVSHQAGDCWLIRGPLEYVPSAKVEVVEERQAIPLDQNEGIYVQDVKTGKVRAVIGSTYMLTQDEVLWEKELPSGVEELLNLGHDPLADRGQKGTAKPLQPSAPRNKTRVVSYRVPHNAAVQVYDYRAKRARVVFGPELVTLDPEEQFTVLSLSAGRPKRPHARRALCLLLGPDFFTDVITIETADHARLQLQLAYNWHFELKNRNDPAEAAKLFSVPDFVGDACKAIASRVRGAVASVTFDDFHKNSARIIRMAVFGFEGSPEDELAANEEELQQNEQKLAQIKQKLQAIKYGGGGSGGGGSGGGGCLDLKTQVQTPQGMKEISNIQVGDLVLSNTGYNEVLNVFPKSKKKSYKITLEDGKEIICSEEHLFPTQTGEMNISGGLKEGMCLYVKEGSGGENLYFQSAMGSHGAAAGSGGMMLKKILKIEELDERELIDIEVSGNHLFYANDGSGATNFSLLKQAGDVEENPGPGSSSKKKSYKITLEDGKEIICSEEHLFPTQTGEMNISGGLKEGMCLYVKEGSGGENLYFQSAMGSHGAAAGSGGMMLKKILKIEELDERELIDIEVSGNHLFYANDILTHNCGLCVCPCNKLKSSDAYKKAWGNNQDGVVASQPARVGGGGSGGGGSGGGGSPEDEIQQLEEEIAQLEQKNAALKEKNQALKYGKARDQAVFPQNGLVVSSVDVQSVEPVDQRTRDALQRSVQLAIEITTNSQEAAAKHEAQRLEQEARGRLERQKILDQSEAEKARKELLELEAMSMAVESTGNAKAEAESRAEAARIEGEGSVLQAKLKAQALAIETEAELERVKKVREMELIYARAQLELEVSKAQQLANVEAKKFKEMTEALGPGTIRDLAVAGPEMQVKLLQSLGLKSTLITDGSSPINLFSTAFGLLGLGSDGQPPAQK

SEQ ID NO: 82 - protein, 1255 aa, Artificial Sequence
  TEV protease inducible Vault based on caged Gp41-1 split inteins, Version 2
MATEEAIIRIPPYHYIHVLDQNSNVSRVEVGPKTYIRQDNERVLFAPVRMVTVPPRHYCIVANPVSRDTQSSVLFDITGQVRLRHADQEIRLAQDPFPLYPGEVLEKDITPLQVVLPNTALHLKALLDFEDKNGDKVMAGDEWLFEGPGTYIPQKEVEVVEIIQATVIKQNQALRLRARKECFDREGKGRVTGEEWLVRSVGAYLPAVFEEVLDLVDAVILTEKTALHLRALQNFRDLRGVLHRTGEEWLVTVQDTEAHVPDVYEEVLGVVPITTLGPRHYCVILDPMGPDGKNQLGQKRVVKGEKSFFLQPGERLERGIQDVYVLSEQQGLLLKALQPLEEGESEEKVSHQAGDCWLIRGPLEYVPSAKVEVVEERQAIPLDQNEGIYVQDVKTGKVRAVIGSTYMLTQDEVLWEKELPSGVEELLNLGHDPLADRGQKGTAKPLQPSAPRNKTRVVSYRVPHNAAVQVYDYRAKRARVVFGPELVTLDPEEQFTVLSLSAGRPKRPHARRALCLLLGPDFFTDVITIETADHARLQLQLAYNWHFELKNRNDPAEAAKLFSVPDFVGDACKAIASRVRGAVASVTFDDFHKNSARIIRMAVFGFEGSPEDELAANEEELQQNEQKLAQIKQKLQAIKYGGGGSGGGGSGGGGCGLCVCPCNKLKCLDLKTQVQTPQGMKEISNIQVGDLVLSNTGYNEVLNVFPKSKKKSYKITLEDGKEIICSEEHLFPTQTGEMNISGGLKEGMCLYVKEGSGGENLYFQSAMGSHGAAAGSGGMMLKKILKIEELDERELIDIEVSGNHLFYANDGSGATNFSLLKQAGDVEENPGPGSSSKKKSYKITLEDGKEIICSEEHLFPTQTGEMNISGGLKEGMCLYVKEGSGGENLYFQSAMGSHGAAAGSGGMMLKKILKIEELDERELIDIEVSGNHLFYANDILTHNSSDAYKKAWGNNQDGVVASQPARVGGGGSGGGGSGGGGSPEDEIQQLEEEIAQLEQKNAALKEKNQALKYGKARDQAVFPQNGLVVSSVDVQSVEPVDQRTRDALQRSVQLAIEITTNSQEAAAKHEAQRLEQEARGRLERQKILDQSEAEKARKELLELEAMSMAVESTGNAKAEAESRAEAARIEGEGSVLQAKLKAQALAIETEAELERVKKVREMELIYARAQLELEVSKAQQLANVEAKKFKEMTEALGPGTIRDLAVAGPEMQVKLLQSLGLKSTLITDGSSPINLFSTAFGLLGLGSDGQPPAQK

SEQ ID NO: 83 - protein, 241 aa, Artificial Sequence
  MmMT3 fused to endogenous vault cargo protein mINT
MDPETCPCPTGGSCTCSDKCKCKGCKCTNCKKSCCSCCPAGCEKCAKDCVCKGEEGAKAEAEKCSCCQGGGSGGGGSGGGDDEGRQSPVSWTSLFALQTEDGFWKLTPELGLILKLNVNALLNSLEEKGIRSLGTKGRERLLDLIATLLVLQFLYTKLEQEGMAAKSLIKMDDVLISRNIPWAFENIKKAREWARRTEGQYPSICQRLELGKDWESATKQLLGIQHQGNTSLHRILHYSQG

SEQ ID NO: 84 - protein, 996 aa, Artificial Sequence
  MmMT3 inserted into rat Vault Helix-Loop-Helix motif
MATEEAIIRIPPYHYIHVLDQNSNVSRVEVGPKTYIRQDNERVLFAPVRMVTVPPRHYCIVANPVSRDTQSSVLFDITGQVRLRHADQEIRLAQDPFPLYPGEVLEKDITPLQVVLPNTALHLKALLDFEDKNGDKVMAGDEWLFEGPGTYIPQKEVEVVEIIQATVIKQNQALRLRARKECFDREGKGRVTGEEWLVRSVGAYLPAVFEEVLDLVDAVILTEKTALHLRALQNFRDLRGVLHRTGEEWLVTVQDTEAHVPDVYEEVLGVVPITTLGPRHYCVILDPMGPDGKNQLGQKRVVKGEKSFFLQPGERLERGIQDVYVLSEQQGLLLKALQPLEEGESEEKVSHQAGDCWLIRGPLEYVPSAKVEVVEERQAIPLDQNEGIYVQDVKTGKVRAVIGSTYMLTQDEVLWEKELPSGVEELLNLGGGGSPEDKLQAIKYELAQNEEELAQIEEKLAANKEGGSGGGGSGGDPETCPCPTGGSCTCSDKCKCKGCKCTNCKKSCCSCCPAGCEKCAKDCVCKGEEGAKAEAEKCSCCQGGSGGGGSGGPEDENAALEEKIAQLKQKNAALKEEIQALEYSAPRNKTRVVSYRVPHNAAVQVYDYRAKRARVVFGPELVTLDPEEQFTVLSLSAGRPKRPHARRALCLLLGPDFFTDVITIETADHARLQLQLAYNWHFELKNRNDPAEAAKLFSVPDFVGDACKAIASRVRGAVASVTFDDFHKNSARIIRMAVFGFEMSEDTGPDGTLLPKARDQAVFPQNGLVVSSVDVQSVEPVDQRTRDALQRSVQLAIEITTNSQEAAAKHEAQRLEQEARGRLERQKILDQSEAEKARKELLELEAMSMAVESTGNAKAEAESRAEAARIEGEGSVLQAKLKAQALAIETEAELERVKKVREMELIYARAQLELEVSKAQQLANVEAKKFKEMTEALGPGTIRDLAVAGPEMQVKLLQSLGLKSTLITDGSSPINLFSTAFGLLGLGSDGQPPAQK

SEQ ID NO: 85 - protein, 1125 aa, Artificial Sequence
  Rat Vault with N-terminal anti-parallel coiled-coil domain stabilizing the holo-vault configuration and MT3 and His6-tag in the HLH domain
MADIEQELERLKASIRRLEQEVNQERARMAALQTLLAKGGSGGATEEAIIRIPPYHYIHVLDQNSNVSRVEVGPKTYIRQDNERVLFAPVRMVTVPPRHYCIVANPVSRDTQSSVLFDITGQVRLRHADQEIRLAQDPFPLYPGEVLEKDITPLQVVLPNTALHLKALLDFEDKNGDKVMAGDEWLFEGPGTYIPQKEVEVVEIIQATVIKQNQALRLRARKECFDREGKGRVTGEEWLVRSVGAYLPAVFEEVLDLVDAVILTEKTALHLRALQNFRDLRGVLHRTGEEWLVTVQDTEAHVPDVYEEVLGVVPITTLGPRHYCVILDPMGPDGKNQLGQKRVVKGEKSFFLQPGERLERGIQDVYVLSEQQGLLLKALQPLEEGESEEKVSHQAGDCWLIRGPLEYVPSAKVEVVEERQAIPLDQNEGIYVQDVKTGKVRAVIGSTYMLTQDEVLWEKELPSGVEELLNLGGGGSPEDKLQAIKYELAQNEEELAQIEEKLAANKEGGSGGGGSGGDPETCPCPTGGSCTCSDKCKCKGCKCTNCKKSCCSCCPAGCEKCAKDCVCKGEEGAKAEAEKCSCCQGGSGGGGSGGPEDENAALEEKIAQLKQKNAALKEEIQALEYSAPRNKTRVVSYRVPHNAAVQVYDYRAKRARVVFGPELVTLDPEEQFTVLSLSAGRPKRPHARRALCLLLGPDFFTDVITIETADHARLQLQLAYNWHFELKNRNDPAEAAKLFSVPDFVGDACKAIASRVRGAVASVTFDDFHKNSARIIRMAVFGFEGSPEDELAANEEELQQNEQKLAQIKQKLQAIKYGGGGSGGGGSGGGGHHHHHHGGGGSGGGGSGGGGSPEDEIQQLEEEIAQLEQKNAALKEKNQALKYGKARDQAVFPQNGLVVSSVDVQSVEPVDQRTRDALQRSVQLAIEITTNSQEAAAKHEAQRLEQEARGRLERQKILDQSEAEKARKELLELEAMSMAVESTGNAKAEAESRAEAARIEGEGSVLQAKLKAQALAIETEAELERVKKVREMELIYARAQLELEVSKAQQLANVEAKKFKEMTEALGPGTIRDLAVAGPEMQVKLLQSLGLKSTLITDGSSPINLFSTAFGLLGLGSDGQPPAQK

SEQ ID NO: 86 - protein, 187 aa, Artificial Sequence
  Synthetic Hyperstable de novo TIM barrel varian
MDILIVNATDVDEMLKQVEILRRLGAKQIAVVSDDWRILQEALKKGGDILIVNATDVDEMLKQVEILRRLGAKQIAVVSDDWRILQEALKKGGDILIVNATDVDEMLKQVEILRRLGAKQIAVVSDDWRILQEALKKGGDILIVNATDVDEMLKQVEILRRLGAKQIAVVSDDWRILQEALKKGGLE

SEQ ID NO: 87 - protein, 456 aa, Sus scrofa
MNLDIHCEQLSDARWTELLPLLQQYEVVRLDDCGLTEEHCKDIGSALRANPSLTELCLRTNELGDAGVHLVLQGLQSPTCKIQKLSLQNCSLTEAGCGVLPSTLRSLPTLRELHLSDNPLGDAGLRLLCEGLLDPQCHLEKLQLEYCRLTAASCEPLASVLRATRALKELTVSNNDIGEAGARVLGQGLADSACQLETLRLENCGLTPANCKDLCGIVASQASLRELDLGSNGLGDAGIAELCPGLLSPASRLKTLWLWECDITASGCRDLCRVLQAKETLKELSLAGNKLGDEGARLLCESLLQPGCQLESLWVKSCSLTAACCQHVSLMLTQNKHLLELQLSSNKLGDSGIQELCQALSQPGTTLRVLCLGDCEVTNSGCSSLASLLLANRSLRELDLSNNCVGDPGVLQLLGSLEQPGCALEQLVLYDTYWTEEVEDRLQALEGSKPGLRVIS

SEQ ID NO: 88 - protein, 242 aa, Pseudomonas aeruginosa
TYCVAMHLADGLVFASDSRTNAGIDHIATFRKLFTFGTPGERLLVVQTAGNLATSQSVINLLQQRIRRDGASLLNVPSVYDATALVAETTREVMARDSGNLAGNTDLSCSFMVGGQIAGGPPALYSIYPQGNFIQATPDTPFLQLGESKYGKPILDRNLTFDTPLEQALRCALVSFDSTIRSNLSVGMPLDLLVYHRDSLILPEGYRVTEDDAYFSAIRRQWSAGLHDMLERLPSPPSAYNI

SEQ ID NO: 89 - protein, 249 aa, Bacteriophage S16
MAVQGPWVGSSYVAETGQNWASLAANELRVTERPFWISSFIGRSKEEIWEWTGENHSFNKDWLIGELRNRGGTPVVINIRAHQVSYTPGAPLFEFPGDLPNAYITLNIYADIYGRGGTGGVAYLGGNPGGDCIHNWIGNRLRINNQGWICGGGGGGGGFRVGHTEAGGGGGRPLGAGGVSSLNLNGDNATLGAPGRGYQLGNDYAGNGGDVGNPGSASSAEMGGGAAGRAVVGTSPQWINVGNIAGSWL

SEQ ID NO: 90 - protein, 204 aa, Bacteriophage S16
MGSSHHHHHHSQDPENLYFQGALGSASIAIGDNDTGLRWGGDGIVQIVANNAIVGGWNSTDIFTEAGKHITSNGNLNQWGGGAIYCRDLNVSSDRRIKKDIKAFENPVDILSTIGGYTYLIEKGFNEDGSQAYEESAGLIAQEVEAVLPRLVKISNDGTKDVKRLNYNGITALNTAAINVHTKEINELKKQLKELKDIVKFLTK

SEQ ID NO: 91 - protein, 184 aa, Human adenovirus 26 [sequence omitted]

SEQ ID NO: 92 - protein, 393 aa, Artificial Sequence
  Engineered fluorescent protein based on sfGFP, with ALFA-tags (SRLEEELRRRLT) inserted into loop region and at the termini
MGSRLEEELRRRLTQQQSRLEEELRRRLTQQQSRLEEELRRRLTGQVSKGEELFTGVVPILVELDGDVNGHKFSVRGEGEGDATNGKLTLKFICTTGKLPVPWPTLVTTLTYGVQCFSRYPDHMKRHDFFKSAMPEGYVQERTISFKDDGTYKTRAEVKFEGDTLVNRIELKGIDFKEDGNILGHKLEYNFNSHNVYITADKQKNGIKANFKIRHNVEGGSRLEEELRRRLTQQQSRLEEELRRRLTGGQQGGSRLEEELRRRLTQQQSRLEEELRRRLTGGDGSVQLADHYQQNTPIGDGPVLLPDNHYLSTQSVLSKDPNEKRDHMVLLEFVTAAGITHGMDELYKGQGSRLEEELRRRLTQQQSRLEEELRRRLTQQQSRLEEELRRRLT

SEQ ID NO: 93 - protein, 350 aa, Artificial Sequence
  Engineered fluorescent protein based on mGreenLantern, with HA-tags (YPYDVPDYA) inserted into loop region and at the termini
MGYPYDVPDYAGYPYDVPDYAGYPYDVPDYAGGVSKGEELFTGVVPILVELDGDVNGHKFSVRGEGEGDATNGKLTLKFICTTGKLPVPWPTLVTTLGYGVACFARYPDHMKQHDFFKSAMPEGYVQERTISFKDDGTYKTRAEVKFEGDTLVNRIVLKGIDFKEDGNILGHKLEYNFNSHKVYITADKQKNGIKANFKTRHNVEGGYPYDVPDYAGGYPYDVPDYAGGGGYPYDVPDYAGGYPYDVPDYAGGDGGVQLADHYQQNTPIGDGPVLLPDNHYLSHQSKLSKDPNEKRDHMVLKERVTAAGITHDMDELYKGGYPYDVPDYAGYPYDVPDYAGYPYDVPDYA

SEQ ID NO: 94 - protein, 369 aa, Artificial Sequence
  Engineered fluorescent protein based on mGreenLantern, with Moon-Tags(KNEQELLELDKWASL) inserted into loop region and at the termini
MVSKGEELFTGVVPILVELDGDVNGHKFSVRGEGEGDATNGKLTLKFICTTGKLPVPWPTLVTTLGYGVACFARYPDHMKQHDFFKSAMPEGYVQERTISFKDDGTYKTRAEVKFEGDTLVNRIVLKGIDFKEDGNILGHKLEYNFNSHKVYITADKQKNGIKANFKTRHNVEGGKNEQELLELDKWASLQQQKNEQELLELDKWASLGGQQGGKNEQELLELDKWASLQQQKNEQELLELDKWASLGGDGGVQLADHYQQNTPIGDGPVLLPDNHYLSHQSKLSKDPNEKRDHMVLKERVTAAGITHDMDELYKGQGKNEQELLELDKWASLQQQKNEQELLELDKWASLQQQKNEQELLELDKWASL

SEQ ID NO: 95 - protein, 422 aa, Artificial Sequence
  Engineered fluorescent protein based on mScarlet-I,with PepTags (AVERYLKDQQLLGIW) inserted into loop region and at the termini
MGTGSAVERYLKDQQLLGIWQQQAVERYLKDQQLLGIWQQQAVERYLKDQQLLGIWGQVSKGEAVIKEFMRFKVHMEGSMNGHEFEIEGEGEGRPYEGTQTAKLKVTKGGPLPFSWDILSPQFMYGSRAFIKHPADIPDYYKQSFPEGFKWERVMNFEDGGAVTVTQDTSLEDGTLIYKVKLRGTNFPPDGPVMQKKTMGWEASTERLYPEDGVLKGDIKMALRLKGGAVERYLKDQQLLGIWQQQAVERYLKDQQLLGIWGGQQGGAVERYLKDQQLLGIWQQQAVERYLKDQQLLGIWGGDGGRYLADFKTTYKAKKPVQMPGAYNVDRKLDITSHNEDYTVVEQYERSEGRHSTGGMDELYKGQGAVERYLKDQQLLGIWQQQAVERYLKDQQLLGIWQQQAVERYLKDQQLLGIWGPG

SEQ ID NO: 96 - protein, 457 aa, Artificial Sequence
  Engineered fluorescent protein based on mEosEM, with MoonTags (EELLSKNYHLENEVARLKK) inserted inserted into loop region and at the termini
MGTGSEELLSKNYHLENEVARLKKQQQEELLSKNYHLENEVARLKKQQQEELLSKNYHLENEVARLKKGQVSAIKPDMRIKLRMEGNVNGHHFVIDGEGTGKPYEGKQTMDLEVKEGGPLPFAFDILTTAFHYGNRVFVKYPDNIQDYFKQSFPKGYSWERSMTFEDGGICNARNDITMEGDTFYNKVRFYGTNFPANGPVMQKKTLKWEPSTEKMYVRDGVLTGDIEMALLLEGGEELLSKNYHLENEVARLKKQQQEELLSKNYHLENEVARLKKGGQQGGEELLSKNYHLENEVARLKKQQQEELLSKNYHLENEVARLKKGGGGAHYRCDFRTTYKAKEKGVKLPGAHFVDHAIEILSHDKDYNKVKLYEHAVAHSGLPDNARRGQGEELLSKNYHLENEVARLKKQQQEELLSKNYHLENEVARLKKQQQEELLSKNYHLENEVARLKKGPG

SEQ ID NO: 97 - protein, 339 aa, Artificial Sequence
  Engineered fluorescent protein based on mScarlet-I, with triple FLAG-tags (DYKDHDGDYKDHDIDYKDDDDK) inserted into loop region and at the termini
MGTGSDYKDHDGDYKDHDIDYKDDDDKGQVSKGEAVIKEFMRFKVHMEGSMNGHEFEIEGEGEGRPYEGTQTAKLKVTKGGPLPFSWDILSPQFMYGSRAFIKHPADIPDYYKQSFPEGFKWERVMNFEDGGAVTVTQDTSLEDGTLIYKVKLRGTNFPPDGPVMQKKTMGWEASTERLYPEDGVLKGDIKMALRLKGGDYKDHDGDYKDHDIDYKDDDDKGGGDYKDHDGDYKDHDIDYKDDDDKGGDGGRYLADFKTTYKAKKPVQMPGAYNVDRKLDITSHNEDYTVVEQYERSEGRHSTGGMDELYKGQGDYKDHDGDYKDHDIDYKDDDDKGPG

SEQ ID NO: 98 - protein, 1511 aa, Artificial Sequence
  Engineered fluorescent protein based on emFPv4 with 24x SunTags on both termini
MEELLSKNYHLENEVARLKKGSGSGEELLSKNYHLENEVARLKKGSGSGEELLSKNYHLENEVARLKKGSGSGEELLSKNYHLENEVARLKKGSGSGEELLSKNYHLENEVARLKKGSGSGEELLSKNYHLENEVARLKKGSGSGEELLSKNYHLENEVARLKKGSGSGEELLSKNYHLENEVARLKKGSGSGEELLSKNYHLENEVARLKKGSGSGEELLSKNYHLENEVARLKKGSGSGEELLSKNYHLENEVARLKKGSGSGEELLSKNYHLENEVARLKKGSGSGEELLSKNYHLENEVARLKKGSGSGEELLSKNYHLENEVARLKKGSGSGEELLSKNYHLENEVARLKKGSGSGEELLSKNYHLENEVARLKKGSGSGEELLSKNYHLENEVARLKKGSGSGEELLSKNYHLENEVARLKKGSGSGEELLSKNYHLENEVARLKKGSGSGEELLSKNYHLENEVARLKKGSGSGEELLSKNYHLENEVARLKKGSGSGEELLSKNYHLENEVARLKKGSGSGEELLSKDYHLENEVARLKKGSGSGEELLSKNYHLENEVARLKKVSKGEELFTGVVPILVELDGDVNGHKFSVRGEGEGDATNGKLTLKFICTTGKLPVPWPTLVTTLGYGVACFARYPDHMKQHDFFKSAMPEGYVQERTISFKDDGTYKTRAEVKFEGDTLVNRIVLKGIDFKEDGNILGHKLEYNFNSHKVYITADKQKNGIKANFKTRHNVEGGKNEQELLELDKWASLQQQKNEQELLELDKWASLGGQQGGKNEQELLELDKWASLQQQKNEQELLELDKWASLGGDGGVQLADHYQQNTPIGDGPVLLPDNHYLSHQSKLSKDPNEKRDHMVLKERVTAAGITHDMDELYKGQGKNEQELLELDKWASLQQQKNEQELLELDKWASLQQQKNEQELLELDKWASLEELLSKNYHLENEVARLKKGSGSGEELLSKNYHLENEVARLKKGSGSGEELLSKNYHLENEVARLKKGSGSGEELLSKNYHLENEVARLKKGSGSGEELLSKNYHLENEVARLKKGSGSGEELLSKNYHLENEVARLKKGSGSGEELLSKNYHLENEVARLKKGSGSGEELLSKNYHLENEVARLKKGSGSGEELLSKNYHLENEVARLKKGSGSGEELLSKNYHLENEVARLKKGSGSGEELLSKNYHLENEVARLKKGSGSGEELLSKNYHLENEVARLKKGSGSGEELLSKNYHLENEVARLKKGSGSGEELLSKNYHLENEVARLKKGSGSGEELLSKNYHLENEVARLKKGSGSGEELLSKNYHLENEVARLKKGSGSGEELLSKNYHLENEVARLKKGSGSGEELLSKNYHLENEVARLKKGSGSGEELLSKNYHLENEVARLKKGSGSGEELLSKNYHLENEVARLKKGSGSGEELLSKNYHLENEVARLKKGSGSGEELLSKNYHLENEVARLKKGSGSGEELLSKDYHLENEVARLKKGSGSGEELLSKNYHLENEVARLKK

SEQ ID NO: 99 - protein, 1167 aa, Artificial Sequence
  Engineered fluorescent protein based on emFPv4 with 10x P3 CCC tags on each terminus
MSPEDEIQQLEEEIAQLEQKNAALKEKNQALKYGLKSGPGSGSPEDEIQQLEEEIAQLEQKNAALKEKNQALKYGTGSGPGSGSPEDEIQQLEEEIAQLEQKNAALKEKNQALKYGASSGPGSGSPEDEIQQLEEEIAQLEQKNAALKEKNQALKYGLESGPGSGSPEDEIQQLEEEIAQLEQKNAALKEKNQALKYGSGPGSGSPEDEIQQLEEEIAQLEQKNAALKEKNQALKYLESGPGSGSPEDEIQQLEEEIAQLEQKNAALKEKNQALKYGASSGPGSGSPEDEIQQLEEEIAQLEQKNAALKEKNQALKYGTGSGPGSGSPEDEIQQLEEEIAQLEQKNAALKEKNQALKYGLKSGPGSGSPEDEIQQLEEEIAQLEQKNAALKEKNQALKYGVSKGEELFTGVVPILVELDGDVNGHKFSVRGEGEGDATNGKLTLKFICTTGKLPVPWPTLVTTLGYGVACFARYPDHMKQHDFFKSAMPEGYVQERTISFKDDGTYKTRAEVKFEGDTLVNRIVLKGIDFKEDGNILGHKLEYNFNSHKVYITADKQKNGIKANFKTRHNVEGGKNEQELLELDKWASLQQQKNEQELLELDKWASLGGQQGGKNEQELLELDKWASLQQQKNEQELLELDKWASLGGDGGVQLADHYQQNTPIGDGPVLLPDNHYLSHQSKLSKDPNEKRDHMVLKERVTAAGITHDMDELYKGQGKNEQELLELDKWASLQQQKNEQELLELDKWASLQQQKNEQELLELDKWASLSPEDEIQQLEEEIAQLEQKNAALKEKNQALKYGLKSGPGSGSPEDEIQQLEEEIAQLEQKNAALKEKNQALKYGTGSGPGSGSPEDEIQQLEEEIAQLEQKNAALKEKNQALKYGASSGPGSGSPEDEIQQLEEEIAQLEQKNAALKEKNQALKYGLESGPGSGSPEDEIQQLEEEIAQLEQKNAALKEKNQALKYGSGPGSGSPEDEIQQLEEEIAQLEQKNAALKEKNQALKYLESGPGSGSPEDEIQQLEEEIAQLEQKNAALKEKNQALKYGASSGPGSGSPEDEIQQLEEEIAQLEQKNAALKEKNQALKYGTGSGPGSGSPEDEIQQLEEEIAQLEQKNAALKEKNQALKYGLKSGPGSGSPEDEIQQLEEEIAQLEQKNAALKEKNQALKYG

SEQ ID NO: 100 - protein, 130 aa, Bacteriophage MS2
MASNFTQFVLVDNGGTGDVTVAPSNFANGVAEWISSNSRSQAYKVTCSVRQSSAQNRKYTIKVEVPKVATQTVGGVELPVAAWRSYLNMELTIPIFATNSDCELIVKAMQGLLKDGNPIPSAIAANSGIY

SEQ ID NO: 101 - protein, 393 aa, Bacteriophage MS2
MRAFSTLDRENETFVPSVRVYADGETEDNSFSLKYRSNWTPGRFNSTGAKTKQWHYPSPYSRGALSVTSIDQGAYKRSGSSWGRPYEEKAGFGFSLDARSCYSLFPVSQNLTYIEVPQNVANRASTEVLQKVTQGNFNLGVALAEARSTASQLATQTIALVKAYTAARRGNWRQALRYLALNEDRKFRSKHVAGRWLELQFGWLPLMSDIQGAYEMLTKVHLQEFLPMRAVRQVGTNIKLDGRLSYPAANFQTTCNISRRIVIWFYINDARLAWLSSLGILNPLGIVWEKVPFSFVVDWLLPVGNMLEGLTAPVGCSYMSGTVTDVITGESIISVDAPYGWTVERQGTAKAQISAMHRGVQSVWPTTGAYVKSPFSMVHTLDALALIRQRLSR

SEQ ID NO: 102 - protein, 133 aa, Bacteriophage Q-beta
MAKLETVTLGNIGKDGKQTLVLNPRGVNPTNGVASLSQAGAVPALEKRVTVSVSQPSRNRKNYKVQVKIQNPTACTANGSCDPSVTRQAYADVTFSFTQYSTDEERAFVRTELAALLASPLLIDAIDQLNPAY

SEQ ID NO: 103 - protein, 420 aa, Bacteriophage Q-beta
MPKLPRGLRFGADNEILNDFQELWFPDLFIESSDTHPWYTLKGRVLNAHLDDRLPNVGGRQVRRTPHRVTVPIASSGLRPVTTVQYDPAALSFLLNARVDWDFGNGDSANLVINDFLFRTFAPKEFDFSNSLVPRYTQAFSAFNAKYGTMIGEGLETIKYLGLLLRRLREGYRAVKRGDLRALRRVIQSYHNGKWKPATAGNLWLEFRYGLMPLFYDIRDVMLDWQNRHDKIQRLLRFSVGHGEDYVVEFDNLYPAVAYFKLKGEITLERRHRHGISYANREGYAVFDNGSLRPVSDWKELATAFINPHEVAWELTPYSFVVDWFLNVGDILAQQGQLYHNIDIVDGFDRRDIRLKSFTIKGERNGRPVNVSASLSAVDLFYSRLHTSNLPFATLDLDTTFSSFKHVLDSIFLLTQRVKR

SEQ ID NO: 104 - protein, 294 aa, Artificial Sequence
  Capsid forming monomer from the encapsulin system of Q.thermotolerans tagged with C-termina FLAG epitope
MMNKSQLYPDSPLTDQDFNQLDQTVIEAARRQLVGRRFIELYGPLGRGMQSVFNDIFMESHEAKMDFQGSFDTEVESSRRVNYTIPMLYKDFVLYWRDLEQSKALDIPIDFSVAANAARDVAFLEDQMIFHGSKEFDIPGLMNVKGRLTHLIGNWYESGNAFQDIVEARNKLLEMNHNGPYALVLSPELYSLLHRVHKDTNVLEIEHVRELITAGVFQSPVLKGKSGVIVNTGRNNLDLAISEDFETAYLGEEGMNHPFRVYETVVLRIKRPAAICTLIDPEEGSGDYKDDDDK

SEQ ID NO: 105 - protein, 209 aa, Artificial Sequence
  Fusion of G51-E1-G52 domains of S.aureus protein SasG (amino acids 419-629) and mCherry
APKTITELEKKVEEIPFKKERKFNPDLAPGTEKVTREGQKGEKTITTPTLKNPLTGVIISKGEPKEEITKDPINELTEYGPETIAPGHRDEFDPKLPTGEKEEVPGKPGIKNPETGDVVRPPVDSVTKYGPVKGDSIVEKEEIPFEKERKFNPDLAPGTEKVTREGQKGEKTITTPTLKNPLTGEIISKGESKEEITKDPINELTEYGP

SEQ ID NO: 106 - protein, 407 aa, Artificial Sequence
  Capsid forming monomer from the encapsulin system of Q.thermotolerans tagged with a C-terminal anti-GFP intrabody
MNKSQLYPDSPLTDQDFNQLDQTVIEAARRQLVGRRFIELYGPLGRGMQSVFNDIFMESHEAKMDFQGSFDTEVESSRRVNYTIPMLYKDFVLYWRDLEQSKALDIPIDFSVAANAARDVAFLEDQMIFHGSKEFDIPGLMNVKGRLTHLIGNWYESGNAFQDIVEARNKLLEMNHNGPYALVLSPELYSLLHRVHKDTNVLEIEHVRELITAGVFQSPVLKGKSGVIVNTGRNNLDLAISEDFETAYLGEEGMNHPFRVYETVVLRIKRPAAICTLIDPEEGGGGSGPGGSGVQLVESGGALVQPGGSLRLSCAASGFPVNRYSMRWYRQAPGKEREWVAGMSSAGDRSSYEDSVKGRFTISRDDARNTVYLQMNSLKPEDTAVYYCNVNVGFEYWGQGTQVTVSS

SEQ ID NO: 107 - protein, 298 aa, Artificial Sequence
  Capsid forming monomer from the encapsulin system of M.xanthus tagged with C-terminal FLAG epitope
MPDFLGHAENPLREEEWARLNETVIQVARRSLVGRRILDIYGPLGAGVQTVPYDEFQGVSPGAVDIVGEQETAMVFTDARKFKTIPIIYKDFLLHWRDIEAARTHNMPLDVSAAAGAAALCAQQEDELIFYGDARLGYEGLMTANGRLTVPLGDWTSPGGGFQAIVEATRKLNEQGHFGPYAVVLSPRLYSQLHRIYEKTGVLEIETIRQLASDGVYQSNRLRGESGVVVSTGRENMDLAVSMDMVAAYLGASRMNHPFRVLEALLLRIKHPDAICTLEGAGATERRGSGDYKDDDDK

SEQ ID NO: 108 - protein, 283 aa, Artificial Sequence
  Capsid forming monomer from the encapsulin system of T.maritima (amino acids 1-264) tagged with C-termina BC2 epitope
MEFLKRSFAPLTEKQWQEIDNRAREIFKTQLYGRKFVDVEGPYGWEYAAHPLGEVEVLSDENEVVKWGLRKSLPLIELRATFTLDLWELDNLERGKPNVDLSSLEETVRKVAEFEDEVIFRGCEKSGVKGLLSFEERKIECGSTPKDLLEAIVRALSIFSKDGIEGPYTLVINTDRWINFLKEEAGHYPLEKRVEECLRGGKIITTPRIEDALVVSERGGDFKLILGQDLSIGYEDREKDAVRLFITETFTFQVVNPEALILLKGGGSGPGPDRKAAVSHWQQ

SEQ ID NO: 109 - protein, 439 aa, Artificial Sequence
  Capsid forming monomer from the encapsulin system of T.maritima (amino acids 1-264) N-terminally fused to a synthetic coiled-coil domain 'P2' and C-terminally fused to an anti-mCherry Intrabody (LaM-4)
MSPEDKIAQLKEKNAALKEKNQQLKEKIQALKYGGGGGSGPGEFLKRSFAPLTEKQWQEIDNRAREIFKTQLYGRKFVDVEGPYGWEYAAHPLGEVEVLSDENEVVKWGLRKSLPLIELRATFTLDLWELDNLERGKPNVDLSSLEETVRKVAEFEDEVIFRGCEKSGVKGLLSFEERKIECGSTPKDLLEAIVRALSIFSKDGIEGPYTLVINTDRWINFLKEEAGHYPLEKRVEECLRGGKIITTPRIEDALVVSERGGDFKLILGQDLSIGYEDREKDAVRLFITETFTFQVVNPEALILLKGSGSGSETTGAQVQLVESGGSLVQPGGSLRLSCAASGRFAESSSMGWFRQAPGKEREFVAAISWSGGATNYADSAKGRFTLSRDNTKNTVYLQMNSLKPDDTAVYYCAANLGNYISSNQRLYGYWGQGTQVTVS

SEQ ID NO: 110 - protein, 551 aa, Artificial Sequence
  Fusion protein consisting of MT3, a de novo designed fibril forming protein and GFP
MDPNCSCATDGSCSCAGSCKCKQCKCTSCKKSCCSCCPVGCAKCSQGCICKEASDKCSCCAGSGGSGGSGGMGPEDELKRVEKLVKEAEALLIVAKIKGSKRDLEKALRTAEEAAREAVKVLVQALLEGDPEVALRAVELVVRVAELLLRIAKESGSREALLRALIVAEEAAKLAKMVLELAEKQGDPEVALRAVELVVRVAELLLRIAKESGSEEALERALRVAEEAARLAKRVLELAEEQGDPLVAKMAVELVKRVAELLERIARESGSEEAKERAERVREEARELQERVKELREREGSGSGSGSGSKGEELFTGVVPILVELDGDVNGHKFSVRGEGEGDATNGKLTLKFICTTGKLPVPWPTLVTTLTYGVQCFARYPDHMKQHDFFKSAMPEGYVQERTISFKDDGTYKTRAEVKFEGDTLVNRIELKGIDFKEDGNILGHKLEYNFNSHNVYITADKQKNGIKANFKIRHNVEDGSVQLADHYQQNTPIGDGPVLLPDNHYLSTQSVLSKDPNEKRDHMVLLEFVTAAGITHGMDELYKGSGSLE

SEQ ID NO: 111 - protein, 420 aa, Artificial Sequence
  Fusion protein consisting of hexa-Histidine Tag, a SpyCatcher domain, a de novo designed, single component icosahedron and an MT3 domain
MRGSHHHHHHENLYFQGAVDTLSGLSSEQGQSGDMTIEEDSATHIKFSKRDEDGKELAGATMELRDSSGKTISTWISDGQVKDFYLYPGKYTFVETAAPDGYEVATAITFTVNEQGQVTVNGKATKGDAHIGGSGGSGGEKAAKAEEAARKMEELFKKHKIVAVLRANSVEEAKKKALAVFLGGVHLIEITFTVPDADTVIKELSFLKEMGAIIGAGTVTSVEQCRKAVESGAEFIVSPHLDEEISQFCKEKGVFYMPGVMTPTELVKAMKLGHTILKLFPGEVVGPQFVKAMKGPFPNVKFVPTGGVNLDNVCEWFKAGVLAVGVGSALVKGTPVEVAEKAKAFVEKIRGCTEGSGSGMDPNCSCATDGSCSCAGSCKCKQCKCTSCKKSCCSCCPVGCAKCSQGCICKEASDKCSCCA

SEQ ID NO: 112 - protein, 129 aa, Artificial Sequence
  Fusion protein of E.coli CsgA where the secretion peptide and N22 were deleted (amino acids 36-144) and SpyTag peptide
MSELNIYQYGGGNSALALQTDARNSDLTITQHGGGNGADVGQGSDDSSIDLTQRGFGNSATLDQWNGKNSEMTVKQFGGGNGAAVDQTASNSSVNVTQVGFGNNATAHQYGSGGSGAHIVMVDAYKPTK

SEQ ID NO: 113 - protein, 304 aa, Artificial Sequence
  Fusion protein of capsid forming monomer of the Encapsulin system of Q.thermotolerans and a synthetic peptide interacting with motor proteins
MNKSQLYPDSPLTDQDFNQLDQTVIEAARRQLVGRRFIELYGPLGRGMQSVFNDIFMESHEAKMDFQGSFDTEVESSRRVNYTIPMLYKDFVLYWRDLEQSKALDIPIDFSVAANAARDVAFLEDQMIFHGSKEFDIPGLMNVKGRLTHLIGNWYESGNAFQDIVEARNKLLEMNHNGPYALVLSPELYSLLHRVHKDTNVLEIEHVRELITAGVFQSPVLKGKSGVIVNTGRNNLDLAISEDFETAYLGEEGMNHPFRVYETVVLRIKRPAAICTLIDPEEGSGSAGTVFTTEDIYEWDDSAI

SEQ ID NO: 114 - protein, 697 aa, Artificial Sequence
  Fusion protein consisting of super-folder GFP, the G51-E1-G52 domains of S.aureus protein SasG (amino acids 419-629) and mCherry
MSKGEELFTGVVPILVELDGDVNGHKFSVRGEGEGDATNGKLTLKFICTTGKLPVPWPTLVTTLTYGVQCFSRYPDHMKRHDFFKSAMPEGYVQERTISFKDDGTYKTRAEVKFEGDTLVNRIELKGIDFKEDGNILGHKLEYNFNSHNVYITADKQKNGIKANFKIRHNVEDGSVQLADHYQQNTPIGDGPVLLPDNHYLSTQSVLSKDPNEKRDHMVLLEFVTAAGITHGMDELYKGGTGGSAPKTITELEKKVEEIPFKKERKFNPDLAPGTEKVTREGQKGEKTITTPTLKNPLTGVIISKGEPKEEITKDPINELTEYGPETIAPGHRDEFDPKLPTGEKEEVPGKPGIKNPETGDVVRPPVDSVTKYGPVKGDSIVEKEEIPFEKERKFNPDLAPGTEKVTREGQKGEKTITTPTLKNPLTGEIISKGESKEEITKDPINELTEYGPETGSGATGSVSKGEEDNMAIIKEFMRFKVHMEGSVNGHEFEIEGEGEGRPYEGTQTAKLKVTKGGPLPFAWDILSPQFMYGSKAYVKHPADIPDYLKLSFPEGFKWERVMNFEDGGVVTVTQDSSLQDGEFIYKVKLRGTNFPSDGPVMQKKTMGWEASSERMYPEDGALKGEIKQRLKLKDGGHYDAEVKTTYKAKKPVQLPGAYNVNIKLDITSHNEDYTIVEQYERAEGRHSTGGMDELYK

SEQ ID NO: 115 - protein, 876 aa, Artificial Sequence
  Fusion protein consisting of Gp41-1 C-intein, superfolder GFP, SasG (comprising 4 G5 domains yielding GEGEGEG), and engineered SpyCatcher003
MMLKKILKIEELDERELIDIEVSGNHLFYANDILTHNSSSGTGSGGSKGEELFTGVVPILVELDGDVNGHKFSVRGEGEGDATNGKLTLKFICTTGKLPVPWPTLVTTLTYGVQCFSRYPDHMKRHDFFKSAMPEGYVQERTISFKDDGTYKTRAEVKFEGDTLVNRIELKGIDFKEDGNILGHKLEYNFNSHNVYITADKQKNGIKANFKIRHNVEDGSVQLADHYQQNTPIGDGPVLLPDNHYLSTQSVLSKDPNEKRDHMVLLEFVTAAGITHGMDELYKGGTGGSAPKTITELEKKVEEIPFKKERKFNPDLAPGTEKVTREGQKGEKTITTPTLKNPLTGVIISKGEPKEEITKDPINELTEYGPETIAPGHRDEFDPKLPTGEKEEVPGKPGIKNPETGDVVRPPVDSVTKYGPVKGDSIVEKEEIPFEKERKFNPDLAPGTEKVTREGQKGEKTITTPTLKNPLTGEIISKGESKEEITKDPINELTEYGPETIAPGHRDEFDPKLPTGEKEEVPGKPGIKNPETGDVVRPPVDSVTKYGPVKGDSIVEKEEIPFEKERKFNPDLAPGTEKVTREGQKGEKTITTPTLKNPLTGEIISKGESKEEITKDPINELTEYGPETIAPGHRDEFDPKLPTGEKEEVPGKPGIKNPETGDVVRPPVDSVTKYGPVKGDSIVEKEEIPFEKERKFNPDLAPGTEKVTREGQKGEKTITTPTLKNPLTGEIISKGESKEEITKDPINELTEYGPETGSGATGSVTTLSGLSGEQGPSGDMTTEEDSATHIKFSKRDEDGRELAGATMELRDSSGKTISTWISDGHVKDFYLYPGKYTFVETAAPDGYEVATPIEFTVNEDGQVTVDGEATEGDAHT

SEQ ID NO: 116 - protein, 829 aa, Artificial Sequence
  Fusion protein consisting of a SnoopTag, mTurquoise2, SasG (comprising 4 G5 domains yielding GEGEGEG) and the N-intein split fragment of Gp41-1
MGKLGDIEFIKVNKSGGGSGVSKGEELFTGVVPILVELDGDVNGHKFSVSGEGEGDATYGKLTLKFICTTGKLPVPWPTLVTTLSWGVQCFARYPDHMKQHDFFKSAMPEGYVQERTIFFKDDGNYKTRAEVKFEGDTLVNRIELKGIDFKEDGNILGHKLEYNYFSDNVYITADKQKNGIKANFKIRHNIEDGGVQLADHYQQNTPIGDGPVLLPDNHYLSTQSKLSKDPNEKRDHMVLLEFVTAAGITLGMDELYKGGTGGSAPKTITELEKKVEEIPFKKERKFNPDLAPGTEKVTREGQKGEKTITTPTLKNPLTGVIISKGEPKEEITKDPINELTEYGPETIAPGHRDEFDPKLPTGEKEEVPGKPGIKNPETGDVVRPPVDSVTKYGPVKGDSIVEKEEIPFEKERKFNPDLAPGTEKVTREGQKGEKTITTPTLKNPLTGEIISKGESKEEITKDPINELTEYGPETIAPGHRDEFDPKLPTGEKEEVPGKPGIKNPETGDVVRPPVDSVTKYGPVKGDSIVEKEEIPFEKERKFNPDLAPGTEKVTREGQKGEKTITTPTLKNPLTGEIISKGESKEEITKDPINELTEYGPETIAPGHRDEFDPKLPTGEKEEVPGKPGIKNPETGDVVRPPVDSVTKYGPVKGDSIVEKEEIPFEKERKFNPDLAPGTEKVTREGQKGEKTITTPTLKNPLTGEIISKGESKEEITKDPINELTEYGPETGSGATGSSGYCLDLKTQVQTPQGMKEISNIQVGDLVLSNTGYNEVLNVFPKSKKKSYKITLEDGKEIICSEEHLFPTQTGEMNISGGLKEGMCLYVKE

SEQ ID NO: 117 - protein, 858 aa, Artificial Sequence
  Fusion protein consisting of SpyTag003, the red fluorescent protein mCherry, SasG (comprising 4 G5 domains yielding GEGEGEG) and a SnoopCatcher domain
MGRGVPHIVMVDAYKRYKSGGGSGVSKGEEDNMAIIKEFMRFKVHMEGSVNGHEFEIEGEGEGRPYEGTQTAKLKVTKGGPLPFAWDILSPQFMYGSKAYVKHPADIPDYLKLSFPEGFKWERVMNFEDGGVVTVTQDSSLQDGEFIYKVKLRGTNFPSDGPVMQKKTMGWEASSERMYPEDGALKGEIKQRLKLKDGGHYDAEVKTTYKAKKPVQLPGAYNVNIKLDITSHNEDYTIVEQYERAEGRHSTGGMDELYKGGTGGSAPKTITELEKKVEEIPFKKERKFNPDLAPGTEKVTREGQKGEKTITTPTLKNPLTGVIISKGEPKEEITKDPINELTEYGPETIAPGHRDEFDPKLPTGEKEEVPGKPGIKNPETGDVVRPPVDSVTKYGPVKGDSIVEKEEIPFEKERKFNPDLAPGTEKVTREGQKGEKTITTPTLKNPLTGEIISKGESKEEITKDPINELTEYGPETIAPGHRDEFDPKLPTGEKEEVPGKPGIKNPETGDVVRPPVDSVTKYGPVKGDSIVEKEEIPFEKERKFNPDLAPGTEKVTREGQKGEKTITTPTLKNPLTGEIISKGESKEEITKDPINELTEYGPETIAPGHRDEFDPKLPTGEKEEVPGKPGIKNPETGDVVRPPVDSVTKYGPVKGDSIVEKEEIPFEKERKFNPDLAPGTEKVTREGQKGEKTITTPTLKNPLTGEIISKGESKEEITKDPINELTEYGPETGSGATGSLEKGSHMKPLRGAVFSLQKQHPDYPDIYGAIDQNGTYQNVRTGEDGKLTFKNLSDGKYRLFENSEPAGYKPVQNKPIVAFQIVNGEVRDVTSIVPQDIPATYEFTNGKHYITNEPIPPK

SEQ ID NO: 118 - protein, 426 aa, Artificial Sequence
  Fusion protein consisting of superfolder GFP, the G51 domain of SasG and the Npu DnaE N-intein split part
MSKGEELFTGVVPILVELDGDVNGHKFSVRGEGEGDATNGKLTLKFICTTGKLPVPWPTLVTTLTYGVQCFSRYPDHMKRHDFFKSAMPEGYVQERTISFKDDGTYKTRAEVKFEGDTLVNRIELKGIDFKEDGNILGHKLEYNFNSHNVYITADKQKNGIKANFKIRHNVEDGSVQLADHYQQNTPIGDGPVLLPDNHYLSTQSVLSKDPNEKRDHMVLLEFVTAAGITHGMDELYKGGTGGSAPKTITELEKKVEEIPFKKERKFNPDLAPGTEKVTREGQKGEKTITTPTLKNPLTGVIISKGEPKEEITKDPINELTEYGCLSYETEILTVEYGLLPIGKIVEKRIECTVYSVDNNGNIYTQPVAQWHDRGEQEVFEYCLEDGSLIRATKDHKFMTVDGQMLPIDEIFERELDLMRVDNLPN

SEQ ID NO: 119 - protein, 409 aa, Artificial Sequence
  Fusion protein consisting of Npu DnaE GEP C-Intein split fragment, SasG EG domains, where the proline residue in the G51-E junction was mutated to Cysteine to serve as nucleophile in the splicing reaction, and mCherry
MIKIATRKYLGKQNVYDIGVGEPHNFALKNGFIASNCETIAPGHRDEFDPKLPTGEKEEVPGKPGIKNPETGDVVRPPVDSVTKYGPVKGDSIVEKEEIPFEKERKFNPDLAPGTEKVTREGQKGEKTITTPTLKNPLTGEIISKGESKEEITKDPINELTEYGPETGSGATGSVSKGEEDNMAIIKEFMRFKVHMEGSVNGHEFEIEGEGEGRPYEGTQTAKLKVTKGGPLPFAWDILSPQFMYGSKAYVKHPADIPDYLKLSFPEGFKWERVMNFEDGGVVTVTQDSSLQDGEFIYKVKLRGTNFPSDGPVMQKKTMGWEASSERMYPEDGALKGEIKQRLKLKDGGHYDAEVKTTYKAKKPVQLPGAYNVNIKLDITSHNEDYTIVEQYERAEGRHSTGGMDELYK

SEQ ID NO: 120 - protein, 266 aa, Artificial Sequence
  Fusion protein consisting of Npu DnaE GEP C-Intein split fragment, SasG EG domains and the Npu DnaE N-intein split part on its C-terminus. This yields a self-growing fragment which can be capped off with NpuDnaE_GEP_C-Int_SasG_EG_mCherry_V2
MIKIATRKYLGKQNVYDIGVGEPHNFALKNGFIASNCETIAPGHRDEFDPKLPTGEKEEVPGKPGIKNPETGDVVRPPVDSVTKYGPVKGDSIVEKEEIPFEKERKFNPDLAPGTEKVTREGQKGEKTITTPTLKNPLTGEIISKGESKEEITKDPINELTEYGCLSYETEILTVEYGLLPIGKIVEKRIECTVYSVDNNGNIYTQPVAQWHDRGEQEVFEYCLEDGSLIRATKDHKFMTVDGQMLPIDEIFERELDLMRVDNLPN

SEQ ID NO: 121 - protein, 340 aa, Artificial Sequence
  Fusion protein consisting of superfolder GFP, the G51 domain of SasG and the VidaL N-Intein split part
MSKGEELFTGVVPILVELDGDVNGHKFSVRGEGEGDATNGKLTLKFICTTGKLPVPWPTLVTTLTYGVQCFSRYPDHMKRHDFFKSAMPEGYVQERTISFKDDGTYKTRAEVKFEGDTLVNRIELKGIDFKEDGNILGHKLEYNFNSHNVYITADKQKNGIKANFKIRHNVEDGSVQLADHYQQNTPIGDGPVLLPDNHYLSTQSVLSKDPNEKRDHMVLLEFVTAAGITHGMDELYKGGTGGSAPKTITELEKKVEEIPFKKERKFNPDLAPGTEKVTREGQKGEKTITTPTLKNPLTGVIISKGEPKEEITKDPINELTEYGCLPKEAVVQIRLTKKG

SEQ ID NO: 122 - protein, 496 aa, Artificial Sequence
  Fusion protein consisting of VidaL C-Intein split part, SasG EG domains and mCherry
MIEEKKVTVQELRELYLSGEYTIEIDTPDGYQTIGKWFDKGVLSMVRVATATYETVCAFNHMIQLADNTWVQACELDVGVDIQTAAGIQPVMLVEDTSDAECYDFEVMHPNHRYYGDGIVSHNSETIAPGHRDEFDPKLPTGEKEEVPGKPGIKNPETGDVVRPPVDSVTKYGPVKGDSIVEKEEIPFEKERKFNPDLAPGTEKVTREGQKGEKTITTPTLKNPLTGEIISKGESKEEITKDPINELTEYGPETGSGATGSVSKGEEDNMAIIKEFMRFKVHMEGSVNGHEFEIEGEGEGRPYEGTQTAKLKVTKGGPLPFAWDILSPQFMYGSKAYVKHPADIPDYLKLSFPEGFKWERVMNFEDGGVVTVTQDSSLQDGEFIYKVKLRGTNFPSDGPVMQKKTMGWEASSERMYPEDGALKGEIKQRLKLKDGGHYDAEVKTTYKAKKPVQLPGAYNVNIKLDITSHNEDYTIVEQYERAEGRHSTGGMDELYK

SEQ ID NO: 123 - protein, 267 aa, Artificial Sequence
  Fusion protein consisting of VidaL C-Intein split part, SasG EG domains and VidaL N-Intein split part. This building block is a self-growing unit and can be capped off with VidaL-C-Int_SasG_EG_mCherry
MIEEKKVTVQELRELYLSGEYTIEIDTPDGYQTIGKWFDKGVLSMVRVATATYETVCAFNHMIQLADNTWVQACELDVGVDIQTAAGIQPVMLVEDTSDAECYDFEVMHPNHRYYGDGIVSHNSETIAPGHRDEFDPKLPTGEKEEVPGKPGIKNPETGDVVRPPVDSVTKYGPVKGDSIVEKEEIPFEKERKFNPDLAPGTEKVTREGQKGEKTITTPTLKNPLTGEIISKGESKEEITKDPINELTEYGCLPKEAVVQIRLTKKG

SEQ ID NO: 124 - protein, 255 aa, Tobacco etch virus
MEQKLISEEDLGESLFKGPRDYNPISSTICHLTNESDGHTTSLYGIGFGPFIITNKHLFRRNNGTLLVQSLHGVFKVKNTTTLQQHLIDGRDMIIIRMPKDFPPFPQKLKFREPQREERICLVTTNFQTKSMSSMVSDTSCTFPSSDGIFWKHWIQTKDGQCGSPLVSTRDGFIVGIHSASNFTNTNNYFTSVPKNFMELLTNQEAQQWVSGWRLNADSVLWGGHKVFMSKPEEPFQPVKEATQLMSELVYSQYP

SEQ ID NO: 125 - protein, 244 aa, Plum pox virus
MSKSLFRGLRDYNPIASSICQLNNSSGARQSEMFGLGFGGLIVTNQHLFKRNDGELTIRSHHGEFVVKDTKTLKLLPCKGRDIVIIRLPKDFPPFPKRLQFRTPTTEDRVCLIGSNFQTKSISSTMSETSATYPVDNSHFWKHWISTKDGHCGLPIVSTRDGSILGLHSLANSTNTQNFYAAFPDNFETTYLSNQDNDNWIKQWRYNPDEVCWGSLQLKRDIPQSPFTICKLLTDLDGEFVYTQ

SEQ ID NO: 126 - protein, 244 aa, Soybean mosaic virus
MSKSVYKGLRDYSGISTLICQLTNSSDGHKETMFGVGYGSFIITNGHLFRRNNGMLTVKTWHGEFVIHNTTQLKIHFIQGRDVILIRMPKDFPPFGKRNLFRQPKREERVCMVGTNFQEKSLRATVSESSMILPEGKGSFWIHWITTQDGFCGLPLVSVNDGHIVGIHGLTSNDSEKNFFVPLTDGFEKEYLENADNLSWDKHWFWEPSKIAWGSLNLVEEQPKEEFKISKLVSDLFGNTVTVQ

SEQ ID NO: 127 - protein, 242 aa, sunflower mild mosaic virus
MGVSLSRGVRDYNAISSMVCRVTNDSGSSSTTMYGIGYGCYIITNKHLFRENNGRLLITSHHGEYICKNSASLKLSLVPGRDMLLIRLPKDCPPFPSKLKFREPTSEEKAVLVVTNFQEKHLSSMVSESSCVVQREDSPIWRHWISTKDGHCGAPIVSIRDGYIIGSHCGENPMTSNFFTSIPKDFQNLLNGKEANEWVSGWKYNIDAVCWGGLSVVNDAPSEPFITAKVVSALDTEGIKVQ

SEQ ID NO: 128 - protein, 458 aa, Artificial Sequence
  Fusion protein consisting of a triple engineered Lanthanide binding domain (LBT15), a TEV cleavage site, the capsid forming monomer of the Encapsulin system of Q.thermotolerans and a FLAG epitope
MFIDTNNDGWIEGDELLLEEGGSGGGGSFIDTNNDGWIEGDELLLEEGGSGGGGSFIDTNNDGWIEGDELLLEEGGSGGGGSENLYFQSGSGPGMDPETCPCPTGGSCTCSDKCKCKGCKCTNCKKSCCSCCPAGCEKCAKDCVCKGEEGAKAEAEKCSCCQGSGGNKSQLYPDSPLTDQDFNQLDQTVIEAARRQLVGRRFIELYGPLGRGMQSVFNDIFMESHEAKMDFQGSFDTEVESSRRVNYTIPMLYKDFVLYWRDLEQSKALDIPIDFSVAANAARDVAFLEDQMIFHGSKEFDIPGLMNVKGRLTHLIGNWYESGNAFQDIVEARNKLLEMNHNGPYALVLSPELYSLLHRVHKDTNVLEIEHVRELITAGVFQSPVLKGKSGVIVNTGRNNLDLAISEDFETAYLGEEGMNHPFRVYETVVLRIKRPAAICTLIDPEEGSGDYKDDDDK

SEQ ID NO: 129 - protein, 150 aa, Artificial Sequence
  Fusion protein consisting of a FLAG epitope, the N-terminal fragment of the Tobacco etch virus protease (TEV) (amino acids 1-118 and a C-terminal M13 calmodulin-binding peptide
MDYKDDDDKTGGESLFKGPRDYNPISSTICHLTNESDGHTTSLYGIGFGPFIITNKHLFRRNNGTLVVQSLHGVFKVKNTTTLQQHLIDGRDMIIIRMPKDFPPFPQKLKFREPQREERICLVTTNFQTSAGRRKWNKGHAVRAIGRLSS

SEQ ID NO: 130 - protein, 266 aa, Artificial Sequence
  Fusion protein consisting of a Myc epitope, Calmodulin and the C-terminal split fragment of Tobacco etch virus protease (amino acids 119-219, S153N
MASMQKLISEEDLTGDQLTEEQIAEFKEAFSLFDKDGDGTITTKELGTVMRSLGQNPTEAELQDMINEVDADGDGTIDFPEFLTMMARKMKDTDSEEEIREAFRVFDKDGNGYISAAELRHVMTNLGEKLTDEEVDEMIREADIDGDGQVNYEEFVQMMTAKSAGKSMSSMVSDTSCTFPSGDGIFWKHWIQTKDGQCGNPLVSTRDGFIVGIHSASNFTNTNNYFTSVPKNFMELLTNQEAQQWVSGWRLNADSVLWGGHKVFMV

SEQ ID NO: 131 - protein, 315 aa, Artificial Sequence
  Fusion of Encapsulin forming monomer of the Encapsulin system M.xanthus and the Calmodulin binding peptide RS20
MADFLGHAENPLREEEWARLNETVIQVARRSLVGRRILDIYGPLGAGVQTVPYDEFQGVSPGAVDIVGEQETAMVFTDARKFKTIPIIYKDFLLHWRDIEAARTHNMPLDVSAAAGAAALCAQQEDELIFYGDARLGYEGLMTANGRLTVPLGDWTSPGGGFQAIVEATRKLNEQGHFGPYAVVLSPRLYSQLHRIYEKTGVLEIETIRQLASDGVYQSNRLRGESGVVVSTGRENMDLAVSMDMVAAYLGASRMNHPFRVLEALLLRIKHPDAICTLEGAGATERRGSSEGGSGRRKWQKTGHAVRAIGRLSSS

SEQ ID NO: 132 - protein, 305 aa, Artificial Sequence
  Fusion of Encapsulin forming monomer of the Encapsulin system Q.thermotolerans and the Calmodulin binding peptide RS20
MNKSQLYPDSPLTDQDFNQLDQTVIEAARRQLVGRRFIELYGPLGRGMQSVFNDIFMESHEAKMDFQGSFDTEVESSRRVNYTIPMLYKDFVLYWRDLEQSKALDIPIDFSVAANAARDVAFLEDQMIFHGSKEFDIPGLMNVKGRLTHLIGNWYESGNAFQDIVEARNKLLEMNHNGPYALVLSPELYSLLHRVHKDTNVLEIEHVRELITAGVFQSPVLKGKSGVIVNTGRNNLDLAISEDFETAYLGEEGMNHPFRVYETVVLRIKRPAAICTLIDPEEGSGRRKWQKTGHAVRAIGRLSSS

SEQ ID NO: 133 - protein, 287 aa, Artificial Sequence
  Fusion of Encapsulin forming monomer of the Encapsulin system T.maritima and the Calmodulin binding peptide RS20
MEFLKRSFAPLTEKQWQEIDNRAREIFKTQLYGRKFVDVEGPYGWEYAAHPLGEVEVLSDENEVVKWGLRKSLPLIELRATFTLDLWELDNLERGKPNVDLSSLEETVRKVAEFEDEVIFRGCEKSGVKGLLSFEERKIECGSTPKDLLEAIVRALSIFSKDGIEGPYTLVINTDRWINFLKEEAGHYPLEKRVEECLRGGKIITTPRIEDALVVSERGGDFKLILGQDLSIGYEDREKDAVRLFITETFTFQVVNPEALILLKGSGRRKWQKTGHAVRAIGRLSSS

SEQ ID NO: 134 - protein, 315 aa, Artificial Sequence
  Fusion protein of human calmodulin and H.pylori ferritin (AA 5-167, N19Q)
MADQLTEEQIAEFKEAFSLFDKDGDGTITTKELGTVMRSLGQNPTEAELQDMINEVDADGNGTIDFPEFLTMMARKMKDTDSEEEIREAFRVFDKDGNGYISAAELRHVMTNLGEKLTDEEVDEMIREADIDGDGQVNYEEFVQMMTAKSGGDIIKLLNEQVNKEMQSSNLYMSMSSWCYTHSLDGAGLFLFDHAAEEYEHAKKLIIFLNENNVPVQLTSISAPEHKFEGLTQIFQKAYEHEQHISESINNIVDHAIKSKDHATFNFLQWYVAEQHEEEVLFKDILDKIELIGNENHGLYLADQYVKGIAKSRKS

SEQ ID NO: 135 - protein, 235 aa, Artificial Sequence
  Fusion of human Calmodulin and MmMT3 which will be recruited to the scaffold (Enc) to form a contrast halo around the element when elevated Ca2+ levels are present
MDIIKLLNEQVNKEMQSSNLYMSMSSWCYTHSLDGAGLFLFDHAAEEYEHAKKLIIFLNENNVPVQLTSISAPEHKFEGLTQIFQKAYEHEQHISESINNIVDHAIKSKDHATFNFLQWYVAEQHEEEVLFKDILDKIELIGNENHGLYLADQYVKGIAKSRKSGSGMDPETCPCPTGGSCTCSDKCKCKGCKCTNCKKSCCSCCPAGCEKCAKDCVCKGEEGAKAEAEKCSCCQ

SEQ ID NO: 136 - protein, 170 aa, Artificial Sequence
  Fusion protein of MT3, an engineered minimal Troponin C domain of Opsanus tau and the Encapsulin signal of the Encapsulin system of Q.thermotolerans
MDPETCPCPTGGSCTCSDKCKCKGCKCTNCKKSCCSCCPAGCEKCAKDCVCKGEEGAKAEAEKCSCCQTGRMQVADASEEELSECFRIFDFDGNGFIDREEFGDIIRLTGEQLTDEDVDEIFGDSDTDKNGRIDFDEFLKMVENVQPIYPGGGGSGGGGSKGFTVGSLIQ

SEQ ID NO: 137 - protein, 443 aa, Artificial Sequence
  Fusion protein MT3-TnCmin-QtEnc-FLAG
MDPETCPCPTGGSCTCSDKCKCKGCKCTNCKKSCCSCCPAGCEKCAKDCVCKGEEGAKAEAEKCSCCQTGRMQVADASEEELSECFRIFDFDGNGFIDREEFGDIIRLTGEQLTDEDVDEIFGDSDTDKNGRIDFDEFLKMVENVQPIYPGGGGSGGGGSVMNKSQLYPDSPLTDQDFNQLDQTVIEAARRQLVGRRFIELYGPLGRGMQSVFNDIFMESHEAKMDFQGSFDTEVESSRRVNYTIPMLYKDFVLYWRDLEQSKALDIPIDFSVAANAARDVAFLEDQMIFHGSKEFDIPGLMNVKGRLTHLIGNWYESGNAFQDIVEARNKLLEMNHNGPYALVLSPELYSLLHRVHKDTNVLEIEHVRELITAGVFQSPVLKGKSGVIVNTGRNNLDLAISEDFETAYLGEEGMNHPFRVYETVVLRIKRPAAICTLIDPEE

SEQ ID NO: 138 - protein, 723 aa, Artificial Sequence
  Fusion of E3 ubiquitin-protein ligase TRIM21, with inactivating mutations  I79R and  S80A, and mCherry fluorescence protein
TGSGATGSVSKGEEDNMAIIKEFMRFKVHMEGSVNGHEFEIEGEGEGRPYEGTQTAKLKVTKGGPLPFAWDILSPQFMYGSKAYVKHPADIPDYLKLSFPEGFKWERVMNFEDGGVVTVTQDSSLQDGEFIYKVKLRGTNFPSDGPVMQKKTMGWEASSERMYPEDGALKGEIKQRLKLKDGGHYDAEVKTTYKAKKPVQLPGAYNVNIKLDITSHNEDYTIVEQYERAEGRHSTGGMDELYKGGGSGMASAARLTMMWEEVTCPICLDPFVEPVSIECGHSFCQECISQVGKGGGSVCPVCRQRFLLKNLRPNRQLANMVNNLKERAQEAREGTQGERCAVHGERLHLFCEKDGKALCWVCAQSRKHRDHAMVPLEEAAQEYQEKLQVALGELRRKQELAEKLEVEIAIKRADWKKTVETQKSRIHAEFVQQKNFLVEEEQRQLQELEKDEREQLRILGEKEAKLAQQSQALQELISELDRRCHSSALELLQEVIIVLERSESWNLKDLDITSPELRSVCHVPGLKKMLRTCAVHITLDPDTANPWLILSEDRRQVRLGDTQQSIPGNEERFDSYPMVLGAQHFHSGKHYWEVDVTGKEAWDLGVCRDSVRRKGHFLLSSKSGFWTIWLWNKQKYEAGTYPQTPLHLQVPPCQVGIFLDYEAGMVSFYNITDHGSLIYSFSECAFTGPLRPFFSPGFNDGGKNTAPLTLCPLNIGSQGSTDY

SEQ ID NO: 139 - protein, 806 aa, Artificial Sequence
  Fusion of E3 ubiquitin-protein ligase TRIM21, with inactivating mutations  I79R and  S80A, and superfolder GFP
MSKGEELFTGVVPILVELDGDVNGHKFSVRGEGEGDATNGKLTLKFICTTGKLPVPWPTLVTTLTYGVQCFSRYPDHMKRHDFFKSAMPEGYVQERTISFKDDGTYKTRAEVKFEGDTLVNRIELKGIDFKEDGNILGHKLEYNFNSHNVYITADKQKNGIKANFKIRHNVEDGSVQLADHYQQNTPIGDGPVLLPDNHYLSTQSVLSKDPNEKRDHMVLLEFVTAAGITHGMDELYKGGTGGSAPKTITELEKKVEEIPFKKERKFNPDLAPGTEKVTREGQKGEKTITTPTLKNPLTGVIISKGEPKEEITKDPINELTEYGPEGGGSGMASAARLTMMWEEVTCPICLDPFVEPVSIECGHSFCQECISQVGKGGGSVCPVCRQRFLLKNLRPNRQLANMVNNLKERAQEAREGTQGERCAVHGERLHLFCEKDGKALCWVCAQSRKHRDHAMVPLEEAAQEYQEKLQVALGELRRKQELAEKLEVEIAIKRADWKKTVETQKSRIHAEFVQQKNFLVEEEQRQLQELEKDEREQLRILGEKEAKLAQQSQALQELISELDRRCHSSALELLQEVIIVLERSESWNLKDLDITSPELRSVCHVPGLKKMLRTCAVHITLDPDTANPWLILSEDRRQVRLGDTQQSIPGNEERFDSYPMVLGAQHFHSGKHYWEVDVTGKEAWDLGVCRDSVRRKGHFLLSSKSGFWTIWLWNKQKYEAGTYPQTPLHLQVPPCQVGIFLDYEAGMVSFYNITDHGSLIYSFSECAFTGPLRPFFSPGFNDGGKNTAPLTLCPLNIGSQGSTDY

SEQ ID NO: 140 - DNA, 4955 bp, Artificial Sequence
  expression vector pcDNA 3.1 (+) Zeocin containing elements from different organisms
aatggatgagctgtacaagtgataagcggccgctcgagtctagagggcccgtttaaacccgctgatcagcctcgactgtgccttctagttgccagccatctgttgtttgcccctcccccgtgccttccttgaccctggaaggtgccactcccactgtcctttcctaataaaatgaggaaattgcatcgcattgtctgagtaggtgtcattctattctggggggtggggtggggcaggacagcaagggggaggattgggaagacaatagcaggcatgctggggatgcggtgggctctatggcttctgaggcggaaagaaccagctggggctctagggggtatccccacgcgccctgtagcggcgcattaagcgcggcgggtgtggtggttacgcgcagcgtgaccgctacacttgccagcgccctagcgcccgctcctttcgctttcttcccttcctttctcgccacgttcgccggctttccccgtcaagctctaaatcggggcatccctttagggttccgatttagtgctttacggcacctcgaccccaaaaaacttgattagggtgatggttcacgtagtgggccatcgccctgatagacggtttttcgccctttgacgttggagtccacgttctttaatagtggactcttgttccaaactggaacaacactcaaccctatctcggtctattcttttgatttataagggattttggggatttcggcctattggttaaaaaatgagctgatttaacaaaaatttaacgcgaattaattctgtggaatgtgtgtcagttagggtgtggaaagtccccaggctccccaggcaggcagaagtatgcaaagcatgcatctcaattagtcagcaaccaggtgtggaaagtccccaggctccccagcaggcagaagtatgcaaagcatgcatctcaattagtcagcaaccatagtcccgcccctaactccgcccatcccgcccctaactccgcccagttccgcccattctccgccccatggctgactaattttttttatttatgcagaggccgaggccgcctctgcctctgagctattccagaagtagtgaggaggcttttttggaggcctaggcttttgcaaaaagctcccgggagcttgtatatccattttcggatctgatcagcacgtgttgacaattaatcatcggcatagtatatcggcatagtataatacgacaaggtgaggaactaaaccatggccaagttgaccagtgccgttccggtgctcaccgcgcgcgacgtcgccggagcggtcgagttctggaccgaccggctcgggttctcccgggacttcgtggaggacgacttcgccggtgtggtccgggacgacgtgaccctgttcatcagcgcggtccaggaccaggtggtgccggacaacaccctggcctgggtgtgggtgcgcggcctggacgagctgtacgccgagtggtcggaggtcgtgtccacgaacttccgggacgcctccgggccggccatgaccgagatcggcgagcagccgtgggggcgggagttcgccctgcgcgacccggccggcaactgcgtgcacttcgtggccgaggagcaggactgacacgtgctacgagatttcgattccaccgccgccttctatgaaaggttgggcttcggaatcgttttccgggacgccggctggatgatcctccagcgcggggatctcatgctggagttcttcgcccaccccaacttgtttattgcagcttataatggttacaaataaagcaatagcatcacaaatttcacaaataaagcatttttttcactgcattctagttgtggtttgtccaaactcatcaatgtatcttatcatgtctgtataccgtcgacctctagctagagcttggcgtaatcatggtcatagctgtttcctgtgtgaaattgttatccgctcacaattccacacaacatacgagccggaagcataaagtgtaaagcctggggtgcctaatgagtgagctaactcacattaattgcgttgcgctcactgcccgctttccagtcgggaaacctgtcgtgccagctgcattaatgaatcggccaacgcgcggggagaggcggtttgcgtattgggcgctcttccgcttcctcgctcactgactcgctgcgctcggtcgttcggctgcggcgagcggtatcagctcactcaaaggcggtaatacggttatccacagaatcaggggataacgcaggaaagaacatgtgagcaaaaggccagcaaaaggccaggaaccgtaaaaaggccgcgttgctggcgtttttccataggctccgcccccctgacgagcatcacaaaaatcgacgctcaagtcagaggtggcgaaacccgacaggactataaagataccaggcgtttccccctggaagctccctcgtgcgctctcctgttccgaccctgccgcttaccggatacctgtccgcctttctcccttcgggaagcgtggcgctttctcaatgctcacgctgtaggtatctcagttcggtgtaggtcgttcgctccaagctgggctgtgtgcacgaaccccccgttcagcccgaccgctgcgccttatccggtaactatcgtcttgagtccaacccggtaagacacgacttatcgccactggcagcagccactggtaacaggattagcagagcgaggtatgtaggcggtgctacagagttcttgaagtggtggcctaactacggctacactagaaggacagtatttggtatctgcgctctgctgaagccagttaccttcggaaaaagagttggtagctcttgatccggcaaacaaaccaccgctggtagcggtggtttttttgtttgcaagcagcagattacgcgcagaaaaaaaggatctcaagaagatcctttgatcttttctacggggtctgacgctcagtggaacgaaaactcacgttaagggattttggtcatgagattatcaaaaaggatcttcacctagatccttttaaattaaaaatgaagttttaaatcaatctaaagtatatatgagtaaacttggtctgacagttaccaatgcttaatcagtgaggcacctatctcagcgatctgtctatttcgttcatccatagttgcctgactccccgtcgtgtagataactacgatacgggagggcttaccatctggccccagtgctgcaatgataccgcgagacccacgctcaccggctccagatttatcagcaataaaccagccagccggaagggccgagcgcagaagtggtcctgcaactttatccgcctccatccagtctattaattgttgccgggaagctagagtaagtagttcgccagttaatagtttgcgcaacgttgttgccattgctacaggcatcgtggtgtcacgctcgtcgtttggtatggcttcattcagctccggttcccaacgatcaaggcgagttacatgatcccccatgttgtgcaaaaaagcggttagctccttcggtcctccgatcgttgtcagaagtaagttggccgcagtgttatcactcatggttatggcagcactgcataattctcttactgtcatgccatccgtaagatgcttttctgtgactggtgagtactcaaccaagtcattctgagaatagtgtatgcggcgaccgagttgctcttgcccggcgtcaatacgggataataccgcgccacatagcagaactttaaaagtgctcatcattggaaaacgttcttcggggcgaaaactctcaaggatcttaccgctgttgagatccagttcgatgtaacccactcgtgcacccaactgatcttcagcatcttttactttcaccagcgtttctgggtgagcaaaaacaggaaggcaaaatgccgcaaaaaagggaataagggcgacacggaaatgttgaatactcatactcttcctttttcaatattattgaagcatttatcagggttattgtctcatgagcggatacatatttgaatgtatttagaaaaataaacaaataggggttccgcgcacatttccccgaaaagtgccacctgacgtcgacggatcgggagatctcccgatcccctatggtcgactctcagtacaatctgctctgatgccgcatagttaagccagtatctgctccctgcttgtgtgttggaggtcgctgagtagtgcgcgagcaaaatttaagctacaacaaggcaaggcttgaccgacaattgcatgaagaatctgcttagggttaggcgttttgcgctgcttcgcgatgtacgggccagatatacgcgttgacattgattattgactagttattaatagtaatcaattacggggtcattagttcatagcccatatatggagttccgcgttacataacttacggtaaatggcccgcctggctgaccgcccaacgacccccgcccattgacgtcaataatgacgtatgttcccatagtaacgccaatagggactttccattgacgtcaatgggtggactatttacggtaaactgcccacttggcagtacatcaagtgtatcatatgccaagtacgccccctattgacgtcaatgacggtaaatggcccgcctggcattatgcccagtacatgaccttatgggactttcctacttggcagtacatctacgtattagtcatcgctattaccatggtgatgcggttttggcagtacatcaatgggcgtggatagcggtttgactcacggggatttccaagtctccaccccattgacgtcaatgggagtttgttttggcaccaaaatcaacgggactttccaaaatgtcgtaacaactccgccccattgacgcaaatgggcggtaggcgtgtacggtgggaggtctatataagcagagctctctggctaactagagaacccactgcttactggcttatcgaaattaatacgactcactatagggagacccaagc

SEQ ID NO: 141 - DNA, 6098 bp, Artificial Sequence
  pIRES
tcaatattggccattagccatattattcattggttatatagcataaatcaatattggctattggccattgcatacgttgtatctatatcataatatgtacatttatattggctcatgtccaatatgaccgccatgttggcattgattattgactagttattaatagtaatcaattacggggtcattagttcatagcccatatatggagttccgcgttacataacttacggtaaatggcccgcctggctgaccgcccaacgacccccgcccattgacgtcaataatgacgtatgttcccatagtaacgccaatagggactttccattgacgtcaatgggtggagtatttacggtaaactgcccacttggcagtacatcaagtgtatcatatgccaagtccgccccctattgacgtcaatgacggtaaatggcccgcctggcattatgcccagtacatgaccttacgggactttcctacttggcagtacatctacgtattagtcatcgctattaccatggtgatgcggttttggcagtacaccaatgggcgtggatagcggtttgactcacggggatttccaagtctccaccccattgacgtcaatgggagtttgttttggcaccaaaatcaacgggactttccaaaatgtcgtaacaactgcgatcgcccgccccgttgacgcaaatgggcggtaggcgtgtacggtgggaggtctatataagcagagctcgtttagtgaaccgtcagatcactagaagctttattgcggtagtttatcacagttaaattgctaacgcagtcagtgcttctgacacaacagtctcgaacttaagctgcagtgactctcttaaggtagccttgcagaagttggtcgtgaggcactgggcaggtaagtatcaaggttacaagacaggtttaaggagaccaatagaaactgggcttgtcgagacagagaagactcttgcgtttctgataggcacctattggtcttactgacatccactttgcctttctctccacaggtgtccactcccagttcaattacagctcttaaggctagagtacttaatacgactcactataggctagcctcgagaattcacgcgtcgagcatgcatctagggcggccaattccgcccctctcccccccccccctctccctcccccccccctaacgttactggccgaagccgcttggaataaggccggtgtgcgtttgtctatatgttattttccaccatattgccgtcttttggcaatgtgagggcccggaaacctggccctgtcttcttgacgagcattcctaggggtctttcccctctcgccaaaggaatgcaaggtctgttgaatgtcgtgaaggaagcagttcctctggaagcttcttgaagacaaacaacgtctgtagcgaccctttgcaggcagcggaaccccccacctggcgacaggtgcctctgcggccaaaagccacgtgtataagatacacctgcaaaggcggcacaaccccagtgccacgttgtgagttggatagttgtggaaagagtcaaatggctctcctcaagcgtattcaacaaggggctgaaggatgcccagaaggtaccccattgtatgggatctgatctggggcctcggtgcacatgctttacatgtgtttagtcgaggttaaaaaaacgtctaggccccccgaaccacggggacgtggttttcctttgaaaaacacgatgataagcttgccacaacccgggatcctctagagtcgacccgggcggccgcttccctttagtgagggttaatgcttcgagcagacatgataagatacattgatgagtttggacaaaccacaactagaatgcagtgaaaaaaatgctttatttgtgaaatttgtgatgctattgctttatttgtaaccattataagctgcaataaacaagttaacaacaacaattgcattcattttatgtttcaggttcagggggagatgtgggaggttttttaaagcaagtaaaacctctacaaatgtggtaaaatccgataaggatcgatccgggctggcgtaatagcgaagaggcccgcaccgatcgcccttcccaacagttgcgcagcctgaatggcgaatggacgcgccctgtagcggcgcattaagcgcggcgggtgtggtggttacgcgcagcgtgaccgctacacttgccagcgccctagcgcccgctcctttcgctttcttcccttcctttctcgccacgttcgccggctttccccgtcaagctctaaatcgggggctccctttagggttccgatttagtgctttacggcacctcgaccccaaaaaacttgattagggtgatggttcacgtagtgggccatcgccctgatagacggtttttcgccctttgacgttggagtccacgttctttaatagtggactcttgttccaaactggaacaacactcaaccctatctcggtctattcttttgatttataagggattttgccgatttcggcctattggttaaaaaatgagctgatttaacaaaaatttaacgcgaattttaacaaaatattaacgcttacaatttcctgatgcggtattttctccttacgcatctgtgcggtatttcacaccgcatacgcggatctgcgcagcaccatggcctgaaataacctctgaaagaggaacttggttaggtaccttctgaggcggaaagaaccagctgtggaatgtgtgtcagttagggtgtggaaagtccccaggctccccagcaggcagaagtatgcaaagcatgcatctcaattagtcagcaaccaggtgtggaaagtccccaggctccccagcaggcagaagtatgcaaagcatgcatctcaattagtcagcaaccatagtcccgcccctaactccgcccatcccgcccctaactccgcccagttccgcccattctccgccccatggctgactaattttttttatttatgcagaggccgaggccgcctcggcctctgagctattccagaagtagtgaggaggcttttttggaggcctaggcttttgcaaaaagcttgattcttctgacacaacagtctcgaacttaaggctagagccaccatgattgaacaagatggattgcacgcaggttctccggccgcttgggtggagaggctattcggctatgactgggcacaacagacaatcggctgctctgatgccgccgtgttccggctgtcagcgcaggggcgcccggttctttttgtcaagaccgacctgtccggtgccctgaatgaactgcaggacgaggcagcgcggctatcgtggctggccacgacgggcgttccttgcgcagctgtgctcgacgttgtcactgaagcgggaagggactggctgctattgggcgaagtgccggggcaggatctcctgtcatctcaccttgctcctgccgagaaagtatccatcatggctgatgcaatgcggcggctgcatacgcttgatccggctacctgcccattcgaccaccaagcgaaacatcgcatcgagcgagcacgtactcggatggaagccggtcttgtcgatcaggatgatctggacgaagagcatcaggggctcgcgccagccgaactgttcgccaggctcaaggcgcgcatgcccgacggcgaggatctcgtcgtgacccatggcgatgcctgcttgccgaatatcatggtggaaaatggccgcttttctggattcatcgactgtggccggctgggtgtggcggaccgctatcaggacatagcgttggctacccgtgatattgctgaagagcttggcggcgaatgggctgaccgcttcctcgtgctttacggtatcgccgctcccgattcgcagcgcatcgccttctatcgccttcttgacgagttcttctgagcgggactctggggttcgaaatgaccgaccaagcgacgcccaacctgccatcacgatggccgcaataaaatatctttattttcattacatctgtgtgttggttttttgtgtgaatcgatagcgataaggatccgcgtatggtgcactctcagtacaatctgctctgatgccgcatagttaagccagccccgacacccgccaacacccgctgacgcgccctgacgggcttgtctgctcccggcatccgcttacagacaagctgtgaccgtctccgggagctgcatgtgtcagaggttttcaccgtcatcaccgaaacgcgcgagacgaaagggcctcgtgatacgcctatttttataggttaatgtcatgataataatggtttcttagacgtcaggtggcacttttcggggaaatgtgcgcggaacccctatttgtttatttttctaaatacattcaaatatgtatccgctcatgagacaataaccctgataaatgcttcaataatattgaaaaaggaagagtatgagtattcaacatttccgtgtcgcccttattcccttttttgcggcattttgccttcctgtttttgctcacccagaaacgctggtgaaagtaaaagatgctgaagatcagttgggtgcacgagtgggttacatcgaactggatctcaacagcggtaagatccttgagagttttcgccccgaagaacgttttccaatgatgagcacttttaaagttctgctatgtggcgcggtattatcccgtattgacgccgggcaagagcaactcggtcgccgcatacactattctcagaatgacttggttgagtactcaccagtcacagaaaagcatcttacggatggcatgacagtaagagaattatgcagtgctgccataaccatgagtgataacactgcggccaacttacttctgacaacgatcggaggaccgaaggagctaaccgcttttttgcacaacatgggggatcatgtaactcgccttgatcgttgggaaccggagctgaatgaagccataccaaacgacgagcgtgacaccacgatgcctgtagcaatggcaacaacgttgcgcaaactattaactggcgaactacttactctagcttcccggcaacaattaatagactggatggaggcggataaagttgcaggaccacttctgcgctcggcccttccggctggctggtttattgctgataaatctggagccggtgagcgtgggtctcgcggtatcattgcagcactggggccagatggtaagccctcccgtatcgtagttatctacacgacggggagtcaggcaactatggatgaacgaaatagacagatcgctgagataggtgcctcactgattaagcattggtaactgtcagaccaagtttactcatatatactttagattgatttaaaacttcatttttaatttaaaaggatctaggtgaagatcctttttgataatctcatgaccaaaatcccttaacgtgagttttcgttccactgagcgtcagaccccgtagaaaagatcaaaggatcttcttgagatcctttttttctgcgcgtaatctgctgcttgcaaacaaaaaaaccaccgctaccagcggtggtttgtttgccggatcaagagctaccaactctttttccgaaggtaactggcttcagcagagcgcagataccaaatactgttcttctagtgtagccgtagttaggccaccacttcaagaactctgtagcaccgcctacatacctcgctctgctaatcctgttaccagtggctgctgccagtggcgataagtcgtgtcttaccgggttggactcaagacgatagttaccggataaggcgcagcggtcgggctgaacggggggttcgtgcacacagcccagcttggagcgaacgacctacaccgaactgagatacctacagcgtgagctatgagaaagcgccacgcttcccgaagggagaaaggcggacaggtatccggtaagcggcagggtcggaacaggagagcgcacgagggagcttccagggggaaacgcctggtatctttatagtcctgtcgggtttcgccacctctgacttgagcgtcgatttttgtgatgctcgtcaggggggcggagcctatggaaaaacgccagcaacgcggcctttttacggttcctggccttttgctggccttttgctcacatggctcga

SEQ ID NO: 142 - protein, 293 aa, Artificial Sequence
  Shell forming monomer of the Encapsulin system of Quasibacillus thermotolerans with a C-terminally appended FLAG epitope connected via a short GSG linker.
MNKSQLYPDSPLTDQDFNQLDQTVIEAARRQLVGRRFIELYGPLGRGMQSVFNDIFMESHEAKMDFQGSFDTEVESSRRVNYTIPMLYKDFVLYWRDLEQSKALDIPIDFSVAANAARDVAFLEDQMIFHGSKEFDIPGLMNVKGRLTHLIGNWYESGNAFQDIVEARNKLLEMNHNGPYALVLSPELYSLLHRVHKDTNVLEIEHVRELITAGVFQSPVLKGKSGVIVNTGRNNLDLAISEDFETAYLGEEGMNHPFRVYETVVLRIKRPAAICTLIDPEEGSGDYKDDDDK

SEQ ID NO: 143 - protein, 444 aa, Artificial Sequence
  A tandem of the Mus musculus Metallothionein 3 connected via GGGGSGGGGS linker fused to the shell forming monomer of the Encapsulin system of Quasibacillus thermotolerans with a C-terminally appended FLAG epitope connected via a short GSG
MDPETCPCPTGGSCTCSDKCKCKGCKCTNCKKSCCSCCPAGCEKCAKDCVCKGEEGAKAEAEKCSCCQGGGSGGGSGGSADPETCPCPTGGSCTCSDKCKCKGCKCTNCKKSCCSCCPAGCEKCAKDCVCKGEEGAKAEAEKCSCCQGSGPGNKSQLYPDSPLTDQDFNQLDQTVIEAARRQLVGRRFIELYGPLGRGMQSVFNDIFMESHEAKMDFQGSFDTEVESSRRVNYTIPMLYKDFVLYWRDLEQSKALDIPIDFSVAANAARDVAFLEDQMIFHGSKEFDIPGLMNVKGRLTHLIGNWYESGNAFQDIVEARNKLLEMNHNGPYALVLSPELYSLLHRVHKDTNVLEIEHVRELITAGVFQSPVLKGKSGVIVNTGRNNLDLAISEDFETAYLGEEGMNHPFRVYETVVLRIKRPAAICTLIDPEEGSGDYKDDDDK

SEQ ID NO: 144 - protein, 355 aa, Artificial Sequence
  Fusion of Mus musculus Metallothionein 3 fused to the shell forming monomer of the Encapsulin system of Thermotoga maritima fused to a C-terminal BC2-Tag
MDPETCPCPTGGSCTCSDKCKCKGCKCTNCKKSCCSCCPAGCEKCAKDCVCKGEEGAKAEAEKCSCCQGSGPGEFLKRSFAPLTEKQWQEIDNRAREIFKTQLYGRKFVDVEGPYGWEYAAHPLGEVEVLSDENEVVKWGLRKSLPLIELRATFTLDLWELDNLERGKPNVDLSSLEETVRKVAEFEDEVIFRGCEKSGVKGLLSFEERKIECGSTPKDLLEAIVRALSIFSKDGIEGPYTLVINTDRWINFLKEEAGHYPLEKRVEECLRGGKIITTPRIEDALVVSERGGDFKLILGQDLSIGYEDREKDAVRLFITETFTFQVVNPEALILLKGGGSGPGPDRKAAVSHWQQ

SEQ ID NO: 145 - protein, 318 aa, Artificial Sequence
  Synthetic Lanthanide-bindering tag 15 fused to the shell forming monomer of the Encapsulin system of Quasibacillus thermotolerans fused to a C-terminal FLAG tag-
MFIDTNNDGWIEGDELLLEEGGSGPGNKSQLYPDSPLTDQDFNQLDQTVIEAARRQLVGRRFIELYGPLGRGMQSVFNDIFMESHEAKMDFQGSFDTEVESSRRVNYTIPMLYKDFVLYWRDLEQSKALDIPIDFSVAANAARDVAFLEDQMIFHGSKEFDIPGLMNVKGRLTHLIGNWYESGNAFQDIVEARNKLLEMNHNGPYALVLSPELYSLLHRVHKDTNVLEIEHVRELITAGVFQSPVLKGKSGVIVNTGRNNLDLAISEDFETAYLGEEGMNHPFRVYETVVLRIKRPAAICTLIDPEEGSGDYKDDDDK

SEQ ID NO: 146 - protein, 380 aa, Artificial Sequence
  Engineered tandem Lanthanide-binding tag fused to the shell forming monomer of the Encapsulin system of Quasibacillus thermotolerans fused to a C-terminal FLAG tag
MGPGYIDTNNDGWIEGDELYIDTNNDGWIEGDELLAGGGSGGGSGGSAGPGYIDTNNDGWIEGDELYIDTNNDGWIEGDELLAGSGPGNKSQLYPDSPLTDQDFNQLDQTVIEAARRQLVGRRFIELYGPLGRGMQSVFNDIFMESHEAKMDFQGSFDTEVESSRRVNYTIPMLYKDFVLYWRDLEQSKALDIPIDFSVAANAARDVAFLEDQMIFHGSKEFDIPGLMNVKGRLTHLIGNWYESGNAFQDIVEARNKLLEMNHNGPYALVLSPELYSLLHRVHKDTNVLEIEHVRELITAGVFQSPVLKGKSGVIVNTGRNNLDLAISEDFETAYLGEEGMNHPFRVYETVVLRIKRPAAICTLIDPEEGSGDYKDDDDK

SEQ ID NO: 147 - protein, 304 aa, Artificial Sequence
  Capsid forming monomer from the encapsulin system of Q.thermotolerans tagged with C-terminal SpyTag003
MNKSQLYPDSPLTDQDFNQLDQTVIEAARRQLVGRRFIELYGPLGRGMQSVFNDIFMESHEAKMDFQGSFDTEVESSRRVNYTIPMLYKDFVLYWRDLEQSKALDIPIDFSVAANAARDVAFLEDQMIFHGSKEFDIPGLMNVKGRLTHLIGNWYESGNAFQDIVEARNKLLEMNHNGPYALVLSPELYSLLHRVHKDTNVLEIEHVRELITAGVFQSPVLKGKSGVIVNTGRNNLDLAISEDFETAYLGEEGMNHPFRVYETVVLRIKRPAAICTLIDPEEGGGGSGRGVPHIVMVDAYKRYK

SEQ ID NO: 148 - protein, 434 aa, Artificial Sequence
  Designed Uranyl-binding protein MUP2 fused to the shell forming monomer of the Encapsulin system of Quasibacillus thermotolerans
MVSRLEERVRDLEAEVDKLRERLDRLEETVQAKGGGGSGGGGSGGGGSGGGGSGGVSRLEERVRDLEAEVDKLRERLDRLEETVQAKGGGGSGGGGSGGGGSGGGGSGGVSRLEERVRDLEAEVDKLRERLDRLEETVQAKPPPPRPPPPRTGNKSQLYPDSPLTDQDFNQLDQTVIEAARRQLVGRRFIELYGPLGRGMQSVFNDIFMESHEAKMDFQGSFDTEVESSRRVNYTIPMLYKDFVLYWRDLEQSKALDIPIDFSVAANAARDVAFLEDQMIFHGSKEFDIPGLMNVKGRLTHLIGNWYESGNAFQDIVEARNKLLEMNHNGPYALVLSPELYSLLHRVHKDTNVLEIEHVRELITAGVFQSPVLKGKSGVIVNTGRNNLDLAISEDFETAYLGEEGMNHPFRVYETVVLRIKRPAAICTLIDPEE

SEQ ID NO: 149 - protein, 515 aa, Artificial Sequence
  Designed Uranyl-binding protein MUP5 fused to the shell forming monomer of the Encapsulin system of Quasibacillus thermotolerans
MQLEDKVEELLSKVYHLENEVDRLRKLIENKGGGGSGGGGSQLEDKVEELESEVDHLRNEVARLKKLVGGGGSGGGGSQLEDKVEELLSKVYHLENEVDRLRKLIENKGGGGSGGGGSQLEDKVEELESEVDHLRNEVARLKKLVGGGGSGGGGSQLEDKVEELLSKVYHLENEVDRLRKLIENKGGGGSGGGGSQLEDKVEELESEVDHLRNEVARLKKLVPPPPRPPPPRTGNKSQLYPDSPLTDQDFNQLDQTVIEAARRQLVGRRFIELYGPLGRGMQSVFNDIFMESHEAKMDFQGSFDTEVESSRRVNYTIPMLYKDFVLYWRDLEQSKALDIPIDFSVAANAARDVAFLEDQMIFHGSKEFDIPGLMNVKGRLTHLIGNWYESGNAFQDIVEARNKLLEMNHNGPYALVLSPELYSLLHRVHKDTNVLEIEHVRELITAGVFQSPVLKGKSGVIVNTGRNNLDLAISEDFETAYLGEEGMNHPFRVYETVVLRIKRPAAICTLIDPEE

SEQ ID NO: 150 - protein, 257 aa, Artificial Sequence
  Engineered SpyCatcher 003 domain fused to fatty acid binding protein FABP
MVEAFCATWKLTNSQNFDEYMKALGVGFATRQVGNVTKPTVIISQEGDKVVIRTLSTFKNTEISFQLGEEFDETTADDRNCKSVVSLDGDKLVHIQKWDGKETNFVREIKDGKMVMTLTFGDVVAVRHYEKAPPPPRTGPPPPRVTTLSGLSGEQGPSGDMTTEEDSATHIKFSKRDEDGRELAGATMELRDSSGKTISTWISDGHVKDFYLYPGKYTFVETAAPDGYEVATPIEFTVNEDGQVTVDGEATEGDAHT

SEQ ID NO: 151 - protein, 581 aa, Artificial Sequence
  Heme binding domain BM3h fused to engineered SpyCatcher 003 domain
MTIKEMPQPKTFGELKNLPLLNTDKPVQALMKIADELGEIFKFEAPGRVTRYLSSQRLIKEACDESRFDKNLSQALKFVRDFAGDGLFTSWTHEKNWKKAHNILLPSFSQQAMKGYHAMMVDIAVQLVQKWERLNADEHIEVPEDMTRLTLDTIGLCGFNYRFNSFYRDQPHPFITSMVRALDEAMNKLQRANPDDPAYDENKRQFQEDIKVMNDLVDKIIADRKASGEQSDDLLTHMLNGKDPETGEPLDDENIRYQIITFLIAGHETTSGLLSFALYFLVKNPHVLQKAAEEAARVLVDPVPSYKQVKQLKYVGMVLNEALRLWPTAPAFSLYAKEDTVLGGEYPLEKGDELMVLIPQLHRDKTIWGDDVEEFRPERFENPSAIPQHAFKPFGNGQRACIGQQFALHEATLVLGMMLKHFDFEDHTNYELDIKETLTLKPEGFVVKAKSKKIPLPPPPRTGPPPPRVTTLSGLSGEQGPSGDMTTEEDSATHIKFSKRDEDGRELAGATMELRDSSGKTISTWISDGHVKDFYLYPGKYTFVETAAPDGYEVATPIEFTVNEDGQVTVDGEATEGDAHT

SEQ ID NO: 152 - RNA, 21 nt, Bacteriophage MS2
aaacaugaggauuacccaugu

SEQ ID NO: 153 - protein, 10 aa, Artificial Sequence
  2xGGGGS linker
GGGGSGGGGS

SEQ ID NO: 154 - protein, 107 aa, Artificial Sequence
  Engineered FKBP-derived degron
GVQVETISPGDGRTFPKRGQTCVVHYTGMLEDGKKVDSSRDRNKPFKFMLGKQEVIRGWEEGVAQMSVGQRAKLTISPDYAYGATGHPGIIPPHATLVFDVELLKPE

SEQ ID NO: 155 - protein, 509 aa, Artificial Sequence
  Fusion of engineered ultrasmall fluorescent protein eUnaG followed by MT3, QtEnc and a FLAG-tag
MLEKFVGTWKIADSHNFGEYLKAIGAPKELSDGGDATTPTLYISQKDGDKMSVKIENGPPTFLDTQVKFKLGEEFDEFPSDRRKGVKSVVNLVGEKLVYVQKWDGKETTYVREIKDGKLVVTLTMGDVVAVRSYRRATEGGTGGSDPETCPCPTGGSCTCSDKCKCKGCKCTNCKKSCCSCCPAGCEKCAKDCVCKGEEGAKAEAEKCSCCQGSGPGNKSQLYPDSPLTDQDFNQLDQTVIEAARRQLVGRRFIELYGPLGRGMQSVFNDIFMESHEAKMDFQGSFDTEVESSRRVNYTIPMLYKDFVLYWRDLEQSKALDIPIDFSVAANAARDVAFLEDQMIFHGSKEFDIPGLMNVKGRLTHLIGNWYESGNAFQDIVEARNKLLEMNHNGPYALVLSPELYSLLHRVHKDTNVLEIEHVRELITAGVFQSPVLKGKSGVIVNTGRNNLDLAISEDFETAYLGEEGMNHPFRVYETVVLRIKRPAAICTLIDPEEGSGDYKDDDDK

SEQ ID NO: 156 - protein, 588 aa, Artificial Sequence
  Fusion of engineered ultrasmall fluorescent protein eUnaG followed by 2xMT3, QtEnc and a FLAG-tag
MLEKFVGTWKIADSHNFGEYLKAIGAPKELSDGGDATTPTLYISQKDGDKMSVKIENGPPTFLDTQVKFKLGEEFDEFPSDRRKGVKSVVNLVGEKLVYVQKWDGKETTYVREIKDGKLVVTLTMGDVVAVRSYRRATEGGTGGSDPETCPCPTGGSCTCSDKCKCKGCKCTNCKKSCCSCCPAGCEKCAKDCVCKGEEGAKAEAEKCSCCQGGGSGGGSGGSADPETCPCPTGGSCTCSDKCKCKGCKCTNCKKSCCSCCPAGCEKCAKDCVCKGEEGAKAEAEKCSCCQGSGPGNKSQLYPDSPLTDQDFNQLDQTVIEAARRQLVGRRFIELYGPLGRGMQSVFNDIFMESHEAKMDFQGSFDTEVESSRRVNYTIPMLYKDFVLYWRDLEQSKALDIPIDFSVAANAARDVAFLEDQMIFHGSKEFDIPGLMNVKGRLTHLIGNWYESGNAFQDIVEARNKLLEMNHNGPYALVLSPELYSLLHRVHKDTNVLEIEHVRELITAGVFQSPVLKGKSGVIVNTGRNNLDLAISEDFETAYLGEEGMNHPFRVYETVVLRIKRPAAICTLIDPEEGSGDYKDDDDK

SEQ ID NO: 157 - protein, 609 aa, Artificial Sequence
  Fusion of the engineered green fluorescent protein mGreenLantern, MT3, QtEnc and a FLAG epitope
MVSKGEELFTGVVPILVELDGDVNGHKFSVRGEGEGDATNGKLTLKFICTTGKLPVPWPTLVTTLGYGVACFARYPDHMKQHDFFKSAMPEGYVQERTISFKDDGTYKTRAEVKFEGDTLVNRIVLKGIDFKEDGNILGHKLEYNFNSHKVYITADKQKNGIKANFKTRHNVEDGGVQLADHYQQNTPIGDGPVLLPDNHYLSHQSKLSKDPNEKRDHMVLKERVTAAGITHDMDELYKGGTGGSDPETCPCPTGGSCTCSDKCKCKGCKCTNCKKSCCSCCPAGCEKCAKDCVCKGEEGAKAEAEKCSCCQGSGPGNKSQLYPDSPLTDQDFNQLDQTVIEAARRQLVGRRFIELYGPLGRGMQSVFNDIFMESHEAKMDFQGSFDTEVESSRRVNYTIPMLYKDFVLYWRDLEQSKALDIPIDFSVAANAARDVAFLEDQMIFHGSKEFDIPGLMNVKGRLTHLIGNWYESGNAFQDIVEARNKLLEMNHNGPYALVLSPELYSLLHRVHKDTNVLEIEHVRELITAGVFQSPVLKGKSGVIVNTGRNNLDLAISEDFETAYLGEEGMNHPFRVYETVVLRIKRPAAICTLIDPEEGSGDYKDDDDK

SEQ ID NO: 158 - protein, 778 aa, Artificial Sequence
  Fusion of the engineered fluorescent Calcium integrator CaMPARI2, MT3, QtEnc and a FLAG tag
MGSDQLTEEQIAEFKEAFSLFDKDGDGTITTKELGTVMRSLGQNPTEAELQDMINEVDADGDGTIDFPEFLTMMARKMKDTDSEEEIREAFRVFDKDGNGYISAAELRHVMTNLGEKLTDEEVDEMIREADIDGDGQVNYEEFVVMMTAKLECEKIYVRDGVLTGDIHMILLLEGNAHYRCDFRTTYKAKEKGVKLPGVHYVDHTIEILSHDKDYNKVKIYEYAVAHSGLPDNARRGGTGGSMVSAIKPDMKIKLRMEGNVNGHHFVIDGDGTGKPYEGKQTMDLEVKEGGPLPFAFDILTTAFHYGNRVFVKYPDNIQDYFKQSFPKGYSWERSMTFEDGGICYARSDITMEGDTFYNKVRFYGTNFPANGPVMQKKTLKWMPSWTRSSRRKFNKTGHALRAIGRLSGGTGGSDPETCPCPTGGSCTCSDKCKCKGCKCTNCKKSCCSCCPAGCEKCAKDCVCKGEEGAKAEAEKCSCCQGSGPGNKSQLYPDSPLTDQDFNQLDQTVIEAARRQLVGRRFIELYGPLGRGMQSVFNDIFMESHEAKMDFQGSFDTEVESSRRVNYTIPMLYKDFVLYWRDLEQSKALDIPIDFSVAANAARDVAFLEDQMIFHGSKEFDIPGLMNVKGRLTHLIGNWYESGNAFQDIVEARNKLLEMNHNGPYALVLSPELYSLLHRVHKDTNVLEIEHVRELITAGVFQSPVLKGKSGVIVNTGRNNLDLAISEDFETAYLGEEGMNHPFRVYETVVLRIKRPAAICTLIDPEEGSGDYKDDDDK

SEQ ID NO: 159 - protein, 324 aa, Artificial Sequence
  Synthetic coiled-coil domain P2 (partner of P1) fused to the TmEnc (AA 1-264) with a C-terminal BC2-Tag
MSPEDKIAQLKEKNAALKEKNQQLKEKIQALKYGGGGGSGPGEFLKRSFAPLTEKQWQEIDNRAREIFKTQLYGRKFVDVEGPYGWEYAAHPLGEVEVLSDENEVVKWGLRKSLPLIELRATFTLDLWELDNLERGKPNVDLSSLEETVRKVAEFEDEVIFRGCEKSGVKGLLSFEERKIECGSTPKDLLEAIVRALSIFSKDGIEGPYTLVINTDRWINFLKEEAGHYPLEKRVEECLRGGKIITTPRIEDALVVSERGGDFKLILGQDLSIGYEDREKDAVRLFITETFTFQVVNPEALILLKGGGSGPGPDRKAAVSHWQQ

SEQ ID NO: 160 - protein, 385 aa, Artificial Sequence
  Synthetic coiled-coil domain DHD13a (partner of DHD13b) fused to MxEnc with a StrepTagII
MGTKEDILERQRKIIERAQEIHRRQQEILEELERIIRKPGSSEEAMKRMLKLLEESLRLLKELLELSEESAQLLYEQRGGGGSGPGPDFLGHAENPLREEEWARLNETVIQVARRSLVGRRILDIYGPLGAGVQTVPYDEFQGVSPGAVDIVGEQETAMVFTDARKFKTIPIIYKDFLLHWRDIEAARTHNMPLDVSAAAGAAALCAQQEDELIFYGDARLGYEGLMTANGRLTVPLGDWTSPGGGFQAIVEATRKLNEQGHFGPYAVVLSPRLYSQLHRIYEKTGVLEIETIRQLASDGVYQSNRLRGESGVVVSTGRENMDLAVSMDMVAAYLGASRMNHPFRVLEALLLRIKHPDAICTLEGAGATERRGSGSAWSHPQFEK

SEQ ID NO: 161 - protein, 334 aa, Artificial Sequence
  Synthetic coiled-coil domain P3 (partner of P4) fused to QtEnc with a FLAG-Tag
MSPEDEIQQLEEEIAQLEQKNAALKEKNQALKYGGGGGSGPGNKSQLYPDSPLTDQDFNQLDQTVIEAARRQLVGRRFIELYGPLGRGMQSVFNDIFMESHEAKMDFQGSFDTEVESSRRVNYTIPMLYKDFVLYWRDLEQSKALDIPIDFSVAANAARDVAFLEDQMIFHGSKEFDIPGLMNVKGRLTHLIGNWYESGNAFQDIVEARNKLLEMNHNGPYALVLSPELYSLLHRVHKDTNVLEIEHVRELITAGVFQSPVLKGKSGVIVNTGRNNLDLAISEDFETAYLGEEGMNHPFRVYETVVLRIKRPAAICTLIDPEEGSGDYKDDDDK

SEQ ID NO: 162 - protein, 389 aa, Artificial Sequence
  Fusion of DD-N degron with mScarlet-I and synthetic coiled-coil domain P1 (partner of P2)
GVQVETISPGDGRTFPKRGQTCVVHYTGMLEDGKKVDSSRDRNKPFKFMLGKQEVIRGWEEGVAQMSVGQRAKLTISPDYAYGATGHPGIIPPHATLVFDVELLKPEGSGVSKGEAVIKEFMRFKVHMEGSMNGHEFEIEGEGEGRPYEGTQTAKLKVTKGGPLPFSWDILSPQFMYGSRAFIKHPADIPDYYKQSFPEGFKWERVMNFEDGGAVTVTQDTSLEDGTLIYKVKLRGTNFPPDGPVMQKKTMGWEASTERLYPEDGVLKGDIKMALRLKDGGRYLADFKTTYKAKKPVQMPGAYNVDRKLDITSHNEDYTVVEQYERSEGRHSTGGMDELYKGGGGSGGGGSGPGTGSPEDEIQALEEENAQLEQENAALEEEIAQLEYG

SEQ ID NO: 163 - protein, 444 aa, Artificial Sequence
  Fusion of DD-N degron with mTagBFP2 and synthetic coiled-coil domain DHD13b (partner of DHD13a)
GVQVETISPGDGRTFPKRGQTCVVHYTGMLEDGKKVDSSRDRNKPFKFMLGKQEVIRGWEEGVAQMSVGQRAKLTISPDYAYGATGHPGIIPPHATLVFDVELLKPEGSGVSKGEELIKENMHMKLYMEGTVDNHHFKCTSEGEGKPYEGTQTMRIKVVEGGPLPFAFDILATSFLYGSKTFINHTQGIPDFFKQSFPEGFTWERVTTYEDGGVLTATQDTSLQDGCLIYNVKIRGVNFTSNGPVMQKKTLGWEAFTETLYPADGGLEGRNDMALKLVGGSHLIANAKTTYRSKKPAKNLKMPGVYYVDYRLERIKEANNETYVEQHEVAVARYCDLPSKLGHKLNGGGGSGGGGSGPGTGGTEKRLLEEAERAHREQKEIIKKAQELHRRLEEIVRQSGSSEEAKKEAKKILEEIRELSKRSLELLREILYLSQEQKGSLVPR

SEQ ID NO: 164 - protein, 396 aa, Artificial Sequence
  Fusion of DD-N degron with mGreenLantern and synthetic coiled-coil domain P4 (partner of P3)
GVQVETISPGDGRTFPKRGQTCVVHYTGMLEDGKKVDSSRDRNKPFKFMLGKQEVIRGWEEGVAQMSVGQRAKLTISPDYAYGATGHPGIIPPHATLVFDVELLKPEGSGVSKGEELFTGVVPILVELDGDVNGHKFSVRGEGEGDATNGKLTLKFICTTGKLPVPWPTLVTTLGYGVACFARYPDHMKQHDFFKSAMPEGYVQERTISFKDDGTYKTRAEVKFEGDTLVNRIVLKGIDFKEDGNILGHKLEYNFNSHKVYITADKQKNGIKANFKTRHNVEDGGVQLADHYQQNTPIGDGPVLLPDNHYLSHQSKLSKDPNEKRDHMVLKERVTAAGITHDMDELYKGGGGSGGGGSGPGTGSPEDKIAQLKQKIQALKQENQQLEEENAALEYG

SEQ ID NO: 165 - protein, 365 aa, Artificial Sequence
  Fusion of Mus musculus Metallothionein 3, the shell forming monomer of the Encapsulin system of Quasibacillus thermotolerans and a C-terminal FLAG-Tag
MDPETCPCPTGGSCTCSDKCKCKGCKCTNCKKSCCSCCPAGCEKCAKDCVCKGEEGAKAEAEKCSCCQGSGPGNKSQLYPDSPLTDQDFNQLDQTVIEAARRQLVGRRFIELYGPLGRGMQSVFNDIFMESHEAKMDFQGSFDTEVESSRRVNYTIPMLYKDFVLYWRDLEQSKALDIPIDFSVAANAARDVAFLEDQMIFHGSKEFDIPGLMNVKGRLTHLIGNWYESGNAFQDIVEARNKLLEMNHNGPYALVLSPELYSLLHRVHKDTNVLEIEHVRELITAGVFQSPVLKGKSGVIVNTGRNNLDLAISEDFETAYLGEEGMNHPFRVYETVVLRIKRPAAICTLIDPEEGSGDYKDDDDK

SEQ ID NO: 166 - protein, 370 aa, Artificial Sequence
  Fusion of Mus musculus Metallothionein 3, the shell forming monomer of the Encapsulin system of Myxococcus xanthus and a C-terminal FLAG-Tag
MDPETCPCPTGGSCTCSDKCKCKGCKCTNCKKSCCSCCPAGCEKCAKDCVCKGEEGAKAEAEKCSCCQGSGPGPDFLGHAENPLREEEWARLNETVIQVARRSLVGRRILDIYGPLGAGVQTVPYDEFQGVSPGAVDIVGEQETAMVFTDARKFKTIPIIYKDFLLHWRDIEAARTHNMPLDVSAAAGAAALCAQQEDELIFYGDARLGYEGLMTANGRLTVPLGDWTSPGGGFQAIVEATRKLNEQGHFGPYAVVLSPRLYSQLHRIYEKTGVLEIETIRQLASDGVYQSNRLRGESGVVVSTGRENMDLAVSMDMVAAYLGASRMNHPFRVLEALLLRIKHPDAICTLEGAGATERRGSGDYKDDDDK

SEQ ID NO: 167 - protein, 381 aa, Artificial Sequence
  Fusion of Mus musculus Metallothionein 3, the shell forming monomer of the Encapsulin system of Myxococcus xanthus and a C-terminal FLAG-Tag followed by a cMyc-derived nuclear localization signal (NLS)
MDPETCPCPTGGSCTCSDKCKCKGCKCTNCKKSCCSCCPAGCEKCAKDCVCKGEEGAKAEAEKCSCCQGSGPGPDFLGHAENPLREEEWARLNETVIQVARRSLVGRRILDIYGPLGAGVQTVPYDEFQGVSPGAVDIVGEQETAMVFTDARKFKTIPIIYKDFLLHWRDIEAARTHNMPLDVSAAAGAAALCAQQEDELIFYGDARLGYEGLMTANGRLTVPLGDWTSPGGGFQAIVEATRKLNEQGHFGPYAVVLSPRLYSQLHRIYEKTGVLEIETIRQLASDGVYQSNRLRGESGVVVSTGRENMDLAVSMDMVAAYLGASRMNHPFRVLEALLLRIKHPDAICTLEGAGATERRGSGDYKDDDDKGGPAAKRVKLD

SEQ ID NO: 168 - protein, 376 aa, Artificial Sequence
  Fusion of Mus musculus Metallothionein 3, the shell forming monomer of the Encapsulin system of Quasibacillus thermotolerans and a C-terminal FLAG-Tag followed by a cMyc-derived nuclear localization signal (NLS)
MDPETCPCPTGGSCTCSDKCKCKGCKCTNCKKSCCSCCPAGCEKCAKDCVCKGEEGAKAEAEKCSCCQGSGPGNKSQLYPDSPLTDQDFNQLDQTVIEAARRQLVGRRFIELYGPLGRGMQSVFNDIFMESHEAKMDFQGSFDTEVESSRRVNYTIPMLYKDFVLYWRDLEQSKALDIPIDFSVAANAARDVAFLEDQMIFHGSKEFDIPGLMNVKGRLTHLIGNWYESGNAFQDIVEARNKLLEMNHNGPYALVLSPELYSLLHRVHKDTNVLEIEHVRELITAGVFQSPVLKGKSGVIVNTGRNNLDLAISEDFETAYLGEEGMNHPFRVYETVVLRIKRPAAICTLIDPEEGSGDYKDDDDKGGPAAKRVKLD

SEQ ID NO: 169 - protein, 420 aa, Artificial Sequence
  Fusion of 3xMT with QtEnc and a C-terminal FLAG-Tag.
MDPETCPCPTGGSCTCSDKCKCKGCKCTNCKKSCCSCCPAGCEKCAKDCVCKGEEGAKAEAEKCSCCQGGTGGSTSTTLVKCACEPCLCNVDPSKAIDRNGLYYCSEACADGHTGGSKGCGHTGCNCHGSAGGCDDKCGCAVPCPGGTGCRCTSARSGAAAGEHTTCGCGEHCGCNPCACGREGTPSGRANRRANCSCGAACNCASCGSATAPGGGGSGGGSGGSANKSQLYPDSPLTDQDFNQLDQTVIEAARRQLVGRRFIELYGPLGRGMQSVFNDIFMESHEAKMDFQGSFDTEVESSRRVNYTIPMLYKDFVLYWRDLEQSKALDIPIDFSVAANAARDVAFLEDQMIFHGSKEFDIPGLMNVKGRLTHLIGNWYESGNAFQDIVEARNKLLEMNHNGPYALVLSPELYSLLHRV

SEQ ID NO: 170 - protein, 162 aa, Rattus norvegicus
GDDEGRQSPVSWTSLFALQTEDGFWKLTPELGLILKLNVNALLNSLEEKGIRSLGTKGRERLLDLIATLLVLQFLYTKLEQEGMAAKSLIKMDDVLISRNIPWAFENIKKAREWARRTEGQYPSICQRLELGKDWESATKQLLGIQHQGNTSLHRILHYSQG

SEQ ID NO: 171 - protein, 193 aa, Artificial Sequence
  MT3 fused to SpyCatcher003
MDPETCPCPTGGSCTCSDKCKCKGCKCTNCKKSCCSCCPAGCEKCAKDCVCKGEEGAKAEAEKCSCCQPPPPRTGPPPPRVTTLSGLSGEQGPSGDMTTEEDSATHIKFSKRDEDGRELAGATMELRDSSGKTISTWISDGHVKDFYLYPGKYTFVETAAPDGYEVATPIEFTVNEDGQVTVDGEATEGDAHT

SEQ ID NO: 172 - protein, 359 aa, Artificial Sequence
  Fusion of antiALFATag intrabody with a MT3 tandem, GB1 domain, a FLAG-Tag and C-terminal RXXG degron.
MEVQLQESGGGLVQPGGSLRLSCTASGVTISALNAMAMGWYRQAPGERRVMVAAVSERGNAMYRESVQGRFTVTRDFTNKMVSLQMDNLKPEDTAVYYCHVLEDRVDSFHDYWGQGTQVTVSSGAPGFSSISASGGTGGSDPETCPCPTGGSCTCSDKCKCKGCKCTNCKKSCCSCCPAGCEKCAKDCVCKGEEGAKAEAEKCSCCQGGGSGGGSGGSADPETCPCPTGGSCTCSDKCKCKGCKCTNCKKSCCSCCPAGCEKCAKDCVCKGEEGAKAEAEKCSCCQGSGPGYKLILNGKTLKGETTTEAVDAATAEKVFKQYANDNGVDGEWTYDDATKTFTVTEGDYKDDDDKGRRVG

SEQ ID NO: 173 - protein, 560 aa, Artificial Sequence
  Fusion of antiHA frankenbody with a MeLanM tandem, GB1 domain, a FLAG-Tag and C-terminal RXXG degron.
MAEVKLVESGGGLVKPGGSLKLSCAASGFTFSSYGMSWVRQTPEKRLEWVATISRGGSYTYYPDSVKGRFTISRDNAKNTLYLQMSSLRSEDTAIYYCARRETYDEKGFAYWGQGTTLTVSSGGGGSGGGGSGGGGSDIVLTQSPASLTVSLGQRATISCKSSQSLLNSGNQKNYLTWYQQKPGQPPKLLIYWASTRESGIPARFSGSGSGTDFTLNIHPVEEEDAATYYCQNDNSHPLTFGAGTKLEIGGTGGSPTTTTKVDIAAFDPDKDGTIDLKEALAAGSAAFDKLDPDKDGTLDAKELKGRVSEADLKKLDPDNDGTLDKKEYLAAVEAQFKAANPDNDGTIDARELASPAGSALVNLIRGGGGSGGGGSPTTTTKVDIAAFDPDKDGTIDLKEALAAGSAAFDKLDPDKDGTLDAKELKGRVSEADLKKLDPDNDGTLDKKEYLAAVEAQFKAANPDNDGTIDARELASPAGSALVNLIRGSGPGYKLILNGKTLKGETTTEAVDAATAEKVFKQYANDNGVDGEWTYDDATKTFTVTEGDYKDDDDKGRRVG

SEQ ID NO: 174 - protein, 450 aa, Artificial Sequence
  Fusion of antiMoonTag intrabody with a AssVanabin2 tandem, GB1 domain, a FLAG-Tag and C-terminal RXXG degron.
MEVQLVESGGGLVQPGGSLRLSCAASGSISSVDVMSWYRQAPGKQRELVAFITDRGRTNYKVSVKGRFTISRDNSKNMVYLQMNSLKPEDTADYLCRAESRTSWSSPSPLDVWGRGTQVTVSSGGTGGSSKVIFALVLVVVLVACINATYVEFEEAYAPVDCKGQCTTPCEPLTACKEKCAESCETSADKKTCRRNCKKADCEPQDKVCDACRMKCHKACRAANCASECPKHEHKSDTCRACMKTNCKGGGGSGGGGSSKVIFALVLVVVLVACINATYVEFEEAYAPVDCKGQCTTPCEPLTACKEKCAESCETSADKKTCRRNCKKADCEPQDKVCDACRMKCHKACRAANCASECPKHEHKSDTCRACMKTNCKGSGPGYKLILNGKTLKGETTTEAVDAATAEKVFKQYANDNGVDGEWTYDDATKTFTVTEGDYKDDDDKGRRVG

SEQ ID NO: 175 - protein, 434 aa, Artificial Sequence
  Fusion of antiMoonTag intrabody with a MeLanM tandem, GB1 domain, a FLAG-Tag and C-terminal RXXG degron.
MEVQLVESGGGLVQPGGSLRLSCAASGSISSVDVMSWYRQAPGKQRELVAFITDRGRTNYKVSVKGRFTISRDNSKNMVYLQMNSLKPEDTADYLCRAESRTSWSSPSPLDVWGRGTQVTVSSGGTGGSPTTTTKVDIAAFDPDKDGTIDLKEALAAGSAAFDKLDPDKDGTLDAKELKGRVSEADLKKLDPDNDGTLDKKEYLAAVEAQFKAANPDNDGTIDARELASPAGSALVNLIRGGGGSGGGGSPTTTTKVDIAAFDPDKDGTIDLKEALAAGSAAFDKLDPDKDGTLDAKELKGRVSEADLKKLDPDNDGTLDKKEYLAAVEAQFKAANPDNDGTIDARELASPAGSALVNLIRGSGPGYKLILNGKTLKGETTTEAVDAATAEKVFKQYANDNGVDGEWTYDDATKTFTVTEGDYKDDDDKGRRVG

SEQ ID NO: 176 - protein, 358 aa, Artificial Sequence
  Fusion of antiMoonTag intrabody with a 4xP3 CCC-Tag, GB1 domain, a FLAG-Tag and C-terminal RXXG degron.
MEVQLVESGGGLVQPGGSLRLSCAASGSISSVDVMSWYRQAPGKQRELVAFITDRGRTNYKVSVKGRFTISRDNSKNMVYLQMNSLKPEDTADYLCRAESRTSWSSPSPLDVWGRGTQVTVSSGGTGGSSPEDEIQQLEEEIAQLEQKNAALKEKNQALKYGLKSGPGSGSPEDEIQQLEEEIAQLEQKNAALKEKNQALKYGTGSGPGSGSPEDEIQQLEEEIAQLEQKNAALKEKNQALKYGLKSGPGSGSPEDEIQQLEEEIAQLEQKNAALKEKNQALKYGGSGPGYKLILNGKTLKGETTTEAVDAATAEKVFKQYANDNGVDGEWTYDDATKTFTVTEGDYKDDDDKGRRVG

SEQ ID NO: 177 - protein, 348 aa, Artificial Sequence
  Fusion of antiMoonTag intrabody with a MT3 tandem, GB1 domain, a FLAG-Tag and C-terminal RXXG degron.
MEVQLVESGGGLVQPGGSLRLSCAASGSISSVDVMSWYRQAPGKQRELVAFITDRGRTNYKVSVKGRFTISRDNSKNMVYLQMNSLKPEDTADYLCRAESRTSWSSPSPLDVWGRGTQVTVSSGGTGGSDPETCPCPTGGSCTCSDKCKCKGCKCTNCKKSCCSCCPAGCEKCAKDCVCKGEEGAKAEAEKCSCCQGGGSGGGSGGSADPETCPCPTGGSCTCSDKCKCKGCKCTNCKKSCCSCCPAGCEKCAKDCVCKGEEGAKAEAEKCSCCQGSGPGYKLILNGKTLKGETTTEAVDAATAEKVFKQYANDNGVDGEWTYDDATKTFTVTEGDYKDDDDKGRRVG

SEQ ID NO: 178 - protein, 387 aa, Artificial Sequence
  Fusion of antiMoonTag intrabody with a EcCusF tandem, GB1 domain, a FLAG-Tag and C-terminal RXXG degron.
MEVQLVESGGGLVQPGGSLRLSCAASGSISSVDVMSWYRQAPGKQRELVAFITDRGRTNYKVSVKGRFTISRDNSKNMVYLQMNSLKPEDTADYLCRAESRTSWSSPSPLDVWGRGTQVTVSSGGTGGSDPETCPCPTGGSCTCSDKCKCKGCKCTNCKKSCCSCCPAGCEKCAKDCVCKGEEGAKAEAEKCSCCQMNEHHHETMSEAQPQVISATGEVKGIDLESKKITIHHDPIAAVNWPEMTMRFTITPQTKMSEIKTGDKVAFNFVQQGNLSLLQDIKVSQMNEHHHETMSEAQPQVISATGEVKGIDLESKKITIHHDPIAAVNWPEMTMRFTITPQTKMSEIKTGDKVAFNFVQQGNLSLLQDIKVSQDYKDDDDKGRRVG

SEQ ID NO: 179 - protein, 442 aa, Artificial Sequence
  Fusion of LifeAct-peptide to emFPv4
MGVADLIKKFESISKEEGTGSKNEQELLELDKWASLQQQKNEQELLELDKWASLQQQKNEQELLELDKWASLGQVSKGEELFTGVVPILVELDGDVNGHKFSVRGEGEGDATNGKLTLKFICTTGKLPVPWPTLVTTLGYGVACFARYPDHMKQHDFFKSAMPEGYVQERTISFKDDGTYKTRAEVKFEGDTLVNRIVLKGIDFKEDGNILGHKLEYNFNSHKVYITADKQKNGIKANFKTRHNVEGGKNEQELLELDKWASLQQQKNEQELLELDKWASLGGQQGGKNEQELLELDKWASLQQQKNEQELLELDKWASLGGDGGVQLADHYQQNTPIGDGPVLLPDNHYLSHQSKLSKDPNEKRDHMVLKERVTAAGITHDMDELYKGQGKNEQELLELDKWASLQQQKNEQELLELDKWASLQQQKNEQELLELDKWASL

SEQ ID NO: 180 - DNA, 1329 bp, Artificial Sequence
  DNA sequence encoding QtEnc-FLAG followed by a TGA stop codon, followed by the read-through promoting sequence "RT20s" followed by an anti-GFPintrabody with a C-terminal HiBit peptide.
atgaacaagagccagctgtaccctgacagccctctgaccgaccaggacttcaaccagctggaccagaccgtgattgaagccgccagaaggcagctcgtcggcagaagattcatcgagctgtacggccctctcggcagaggcatgcagagcgtgttcaacgacatcttcatggaaagccacgaggccaagatggacttccagggcagcttcgacaccgaggtggaaagcagcagaagagtgaactacacaatccccatgctgtacaaggacttcgtgctgtactggcgcgacctggaacagagcaaggccctggacatccccatcgatttttccgtggccgccaacgccgctagagatgtggcctttctggaagatcagatgatctttcacggcagcaaagagttcgacatccccggcctgatgaacgtgaagggcagactgacacacctgatcggcaattggtacgagagcggcaacgccttccaggacatcgtggaagcccggaacaagctgctggaaatgaaccacaacggcccctacgctctggtgctgagccctgagctgtatagcctgctgcacagagtgcacaaggacaccaacgtcctggaaatcgagcacgtgcgcgagctgattaccgccggtgtctttcagagccctgtgctgaagggaaagtccggcgtgatcgtgaacaccggcagaaacaacctggacctggccatcagcgaggacttcgagacagcctatctgggcgaagagggcatgaatcaccccttccgggtgtacgagacagtggtgctgcggattaagaggcctgccgccatctgcaccctgatcgatcctgaagaaggctccggcgactacaaggacgacgacgacaaatgacaattagctcatccagacattccgggcggaggtggcagcggacctggtggctccggcgtgcagctggtcgagtccggaggagctctggttcagcccggcggctctcttcgactcagttgtgccgcatctggcttccccgtgaaccgatattcaatgagatggtaccggcaggctcccggaaaggagcgcgaatgggttgccggaatgtcctccgccggcgaccgatcatcttacgaagactctgtcaaaggcagattcaccatcagcagagatgacgcccggaataccgtctatctccagatgaactctcttaagcctgaggatacagcagtctactactgcaacgtgaacgtgggattcgagtattggggacaggggacccaggtcactgtgtcctctggcagcggcggcgtgagcggctggcgcctgtttaaaaaaattagctaa

SEQ ID NO: 181 - DNA, 2742 bp, Artificial Sequence
  DNA sequence encoding QtEnc-FLAG followed by a TGA stop codon, followed by a read-through promoting sequence "RT20s", followed by an Ssp DnaE intein mutant (N159A) which exhibits hyperfast N-terminal cleavage, followed by a P2A peptide followed by a
atgaacaagagccagctgtaccctgacagccctctgaccgaccaggacttcaaccagctggaccagaccgtgattgaagccgccagaaggcagctcgtcggcagaagattcatcgagctgtacggccctctcggcagaggcatgcagagcgtgttcaacgacatcttcatggaaagccacgaggccaagatggacttccagggcagcttcgacaccgaggtggaaagcagcagaagagtgaactacacaatccccatgctgtacaaggacttcgtgctgtactggcgcgacctggaacagagcaaggccctggacatccccatcgatttttccgtggccgccaacgccgctagagatgtggcctttctggaagatcagatgatctttcacggcagcaaagagttcgacatccccggcctgatgaacgtgaagggcagactgacacacctgatcggcaattggtacgagagcggcaacgccttccaggacatcgtggaagcccggaacaagctgctggaaatgaaccacaacggcccctacgctctggtgctgagccctgagctgtatagcctgctgcacagagtgcacaaggacaccaacgtcctggaaatcgagcacgtgcgcgagctgattaccgccggtgtctttcagagccctgtgctgaagggaaagtccggcgtgatcgtgaacaccggcagaaacaacctggacctggccatcagcgaggacttcgagacagcctatctgggcgaagagggcatgaatcaccccttccgggtgtacgagacagtggtgctgcggattaagaggcctgccgccatctgcaccctgatcgatcctgaagaaggctccggcgactacaaggacgacgacgacaaatagcaattagctcatccagacattccgtgtctgtctttcggcaccgagatcctgaccgtggaatacggccctctgcctatcggcaagatcgtgtccgaagagatcaactgcagcgtgtacagcgtggacccagagggcagagtgtacacacaggctatcgcccagtggcacgacagaggcgaacaagaggtgctggaatacgagctggaagatggcagcgtgatcagagccaccagcgaccacagatttctgaccaccgactaccagctgctggccatcgaggaaatcttcgccagacagctggacctgctgaccctggaaaacatcaagcagaccgaggaagccctggacaaccacagactgccctttccactgctggatgccggcaccatcaagatggtcaaagtgatcggcagacgcagcctgggcgtgcagagaatcttcgatatcggactgccccaggaccacaactttctgctggctaacggcgctatcgccgctgcctgttcttgtggctctggatctagaggcggctctggcgccacaaacttcagcctgcttaaacaggccggcgacgtggaagagaaccccggacctaacaagagccagctgtaccctgacagccctctgaccgaccaggacttcaaccagctggaccagaccgtgattgaagccgccagaaggcagctcgtcggcagaagattcatcgagctgtacggccctctcggcagaggcatgcagagcgtgttcaacgacatcttcatggaaagccacgaggccaagatggacttccagggcagcttcgacaccgaggtggaaagcagcagaagagtgaactacacaatccccatgctgtacaaggacttcgtgctgtactggcgcgacctggaacagagcaaggccctggacatccccatcgatttttccgtggccgccaacgccgctagagatgtggcctttctggaagatcagatgatctttcacggcagcaaagagttcgacatccccggcctgatgaacgtgaagggcagactgacacacctgatcggcaattggtacgagagcggcaacgccttccaggacatcgtggaagcccggaacaagctgctggaaatgaaccacaacggcccctacgctctggtgctgagccctgagctgtatagcctgctgcacagagtgcacaaggacaccaacgtcctggaaatcgagcacgtgcgcgagctgattaccgccggtgtctttcagagccctgtgctgaagggaaagtccggcgtgatcgtgaacaccggcagaaacaacctggacctggccatcagcgaggacttcgagacagcctatctgggcgaagagggcatgaatcaccccttccgggtgtacgagacagtggtgctgcggattaagaggcctgccgccatctgcaccctgatcgatcctgaagaaggcggaggtggcagcggacctggtggctccggcgtgcagctggtcgagtccggaggagctctggttcagcccggcggctctcttcgactcagttgtgccgcatctggcttccccgtgaaccgatattcaatgagatggtaccggcaggctcccggaaaggagcgcgaatgggttgccggaatgtcctccgccggcgaccgatcatcttacgaagactctgtcaaaggcagattcaccatcagcagagatgacgcccggaataccgtctatctccagatgaactctcttaagcctgaggatacagcagtctactactgcaacgtgaacgtgggattcgagtattggggacaggggacccaggtcactgtgtcctctggcagcggcggcgtgagcggctggcgcctgtttaaaaaaattagctaa

SEQ ID NO: 182 - protein, 19 aa, Porcine tescho virus
ATNFSLLKQAGDVEENPGP

SEQ ID NO: 183 - protein, 558 aa, Artificial Sequence
  Tandem MT3 fused to QtEnc which has a C-terminal anti GFP intrabody
MDPETCPCPTGGSCTCSDKCKCKGCKCTNCKKSCCSCCPAGCEKCAKDCVCKGEEGAKAEAEKCSCCQGGGSGGGSGGSADPETCPCPTGGSCTCSDKCKCKGCKCTNCKKSCCSCCPAGCEKCAKDCVCKGEEGAKAEAEKCSCCQGSGPGNKSQLYPDSPLTDQDFNQLDQTVIEAARRQLVGRRFIELYGPLGRGMQSVFNDIFMESHEAKMDFQGSFDTEVESSRRVNYTIPMLYKDFVLYWRDLEQSKALDIPIDFSVAANAARDVAFLEDQMIFHGSKEFDIPGLMNVKGRLTHLIGNWYESGNAFQDIVEARNKLLEMNHNGPYALVLSPELYSLLHRVHKDTNVLEIEHVRELITAGVFQSPVLKGKSGVIVNTGRNNLDLAISEDFETAYLGEEGMNHPFRVYETVVLRIKRPAAICTLIDPEEGGGGSGPGGSGVQLVESGGALVQPGGSLRLSCAASGFPVNRYSMRWYRQAPGKEREWVAGMSSAGDRSSYEDSVKGRFTISRDDARNTVYLQMNSLKPEDTAVYYCNVNVGFEYWGQGTQVTVSS

SEQ ID NO: 184 - protein, 238 aa, Aequorea victoria
MSKGEELFTGVVPILVELDGDVNGHKFSVRGEGEGDATNGKLTLKFICTTGKLPVPWPTLVTTLTYGVQCFSRYPDHMKRHDFFKSAMPEGYVQERTISFKDDGTYKTRAEVKFEGDTLVNRIELKGIDFKEDGNILGHKLEYNFNSHNVYITADKQKNGIKANFKIRHNVEDGSVQLADHYQQNTPIGDGPVLLPDNHYLSTQSVLSKDPNEKRDHMVLLEFVTAAGITHGMDELYK

SEQ ID NO: 185 - protein, 235 aa, Anaplasma marginale
VSKGEEDNMAIIKEFMRFKVHMEGSVNGHEFEIEGEGEGRPYEGTQTAKLKVTKGGPLPFAWDILSPQFMYGSKAYVKHPADIPDYLKLSFPEGFKWERVMNFEDGGVVTVTQDSSLQDGEFIYKVKLRGTNFPSDGPVMQKKTMGWEASSERMYPEDGALKGEIKQRLKLKDGGHYDAEVKTTYKAKKPVQLPGAYNVNIKLDITSHNEDYTIVEQYERAEGRHSTGGMDELYK

SEQ ID NO: 186 - protein, 114 aa, Artificial Sequence
  antiGFP-intrabody
VQLVESGGALVQPGGSLRLSCAASGFPVNRYSMRWYRQAPGKEREWVAGMSSAGDRSSYEDSVKGRFTISRDDARNTVYLQMNSLKPEDTAVYYCNVNVGFEYWGQGTQVTVSS

SEQ ID NO: 187 - protein, 124 aa, Artificial Sequence
  antimCherry intrabody (LaM-4)
AQVQLVESGGSLVQPGGSLRLSCAASGRFAESSSMGWFRQAPGKEREFVAAISWSGGATNYADSAKGRFTLSRDNTKNTVYLQMNSLKPDDTAVYYCAANLGNYISSNQRLYGYWGQGTQVTVS

SEQ ID NO: 188 - protein, 953 aa, Artificial Sequence
  Fusion of sfGFP-SasG-G51-G54-mCherry
MSKGEELFTGVVPILVELDGDVNGHKFSVRGEGEGDATNGKLTLKFICTTGKLPVPWPTLVTTLTYGVQCFSRYPDHMKRHDFFKSAMPEGYVQERTISFKDDGTYKTRAEVKFEGDTLVNRIELKGIDFKEDGNILGHKLEYNFNSHNVYITADKQKNGIKANFKIRHNVEDGSVQLADHYQQNTPIGDGPVLLPDNHYLSTQSVLSKDPNEKRDHMVLLEFVTAAGITHGMDELYKGGTGGSAPKTITELEKKVEEIPFKKERKFNPDLAPGTEKVTREGQKGEKTITTPTLKNPLTGVIISKGEPKEEITKDPINELTEYGPETIAPGHRDEFDPKLPTGEKEEVPGKPGIKNPETGDVVRPPVDSVTKYGPVKGDSIVEKEEIPFEKERKFNPDLAPGTEKVTREGQKGEKTITTPTLKNPLTGEIISKGESKEEITKDPINELTEYGPETIAPGHRDEFDPKLPTGEKEEVPGKPGIKNPETGDVVRPPVDSVTKYGPVKGDSIVEKEEIPFEKERKFNPDLAPGTEKVTREGQKGEKTITTPTLKNPLTGEIISKGESKEEITKDPINELTEYGPETIAPGHRDEFDPKLPTGEKEEVPGKPGIKNPETGDVVRPPVDSVTKYGPVKGDSIVEKEEIPFEKERKFNPDLAPGTEKVTREGQKGEKTITTPTLKNPLTGEIISKGESKEEITKDPINELTEYGPETGSGATGSVSKGEEDNMAIIKEFMRFKVHMEGSVNGHEFEIEGEGEGRPYEGTQTAKLKVTKGGPLPFAWDILSPQFMYGSKAYVKHPADIPDYLKLSFPEGFKWERVMNFEDGGVVTVTQDSSLQDGEFIYKVKLRGTNFPSDGPVMQKKTMGWEASSERMYPEDGALKGEIKQRLKLKDGGHYDAEVKTTYKAKKPVQLPGAYNVNIKLDITSHNEDYTIVEQYERAEGRHSTGGMDELYK

SEQ ID NO: 189 - protein, 479 aa, Artificial Sequence
  MT3 fused to QtEnc with a C-terminal anti GFP intrabody
MDPETCPCPTGGSCTCSDKCKCKGCKCTNCKKSCCSCCPAGCEKCAKDCVCKGEEGAKAEAEKCSCCQGSGPGNKSQLYPDSPLTDQDFNQLDQTVIEAARRQLVGRRFIELYGPLGRGMQSVFNDIFMESHEAKMDFQGSFDTEVESSRRVNYTIPMLYKDFVLYWRDLEQSKALDIPIDFSVAANAARDVAFLEDQMIFHGSKEFDIPGLMNVKGRLTHLIGNWYESGNAFQDIVEARNKLLEMNHNGPYALVLSPELYSLLHRVHKDTNVLEIEHVRELITAGVFQSPVLKGKSGVIVNTGRNNLDLAISEDFETAYLGEEGMNHPFRVYETVVLRIKRPAAICTLIDPEEGGGGSGPGGSGVQLVESGGALVQPGGSLRLSCAASGFPVNRYSMRWYRQAPGKEREWVAGMSSAGDRSSYEDSVKGRFTISRDDARNTVYLQMNSLKPEDTAVYYCNVNVGFEYWGQGTQVTVSS

SEQ ID NO: 190 - protein, 402 aa, Artificial Sequence
  Fusion of BmTyr and synthetic coiled-coil domain P2 (partner of P1)
MGHSNKYRVRKNVLHLTDTEKRDFVRTVLILKEKGIYDRYIAWHGAAGKFHTPPGSDRNAAHMSSAFLPWHREYLLRFERDLQSINPEVTLPYWEWETDAQMQDPSQSQIWSADFMGGNGNPIKDFIVDTGPFAAGRWTTIDEQGNPSGGLKRNFGATKEAPTLPTRDDVLNALKITQYDTPPWDMTSQNSFRNQLEGFINGPQLHNRVHRWVGGQMGVVPTAPNDPVFFLHHANVDRIWAVWQIIHRNQNYQPMKNGPFGQNFRDPMYPWNTTPEDVMNHRKLGYVYDIELRKSKRSSGGGGSGGGGSTGSPEDEIQALEEENAQLEQENAALEEEIAQLEYGSGSETPGTSESATPESAISHGFPPEVEEQAAGTLPMSCAQESGMDRHPAACASARINV

SEQ ID NO: 191 - protein, 375 aa, Artificial Sequence
  Fusion of Brain FABP and superfolder GFP
VEAFCATWKLTNSQNFDEYMKALGVGFATRQVGNVTKPTVIISQEGDKVVIRTLSTFKNTEISFQLGEEFDETTADDRNCKSVVSLDGDKLVHIQKWDGKETNFVREIKDGKMVMTLTFGDVVAVRHYEKAPPPPRTGSKGEELFTGVVPILVELDGDVNGHKFSVRGEGEGDATNGKLTLKFICTTGKLPVPWPTLVTTLTYGVQCFSRYPDHMKRHDFFKSAMPEGYVQERTISFKDDGTYKTRAEVKFEGDTLVNRIELKGIDFKEDGNILGHKLEYNFNSHNVYITADKQKNGIKANFKIRHNVEDGSVQLADHYQQNTPIGDGPVLLPDNHYLSTQSVLSKDPNEKRDHMVLLEFVTAAGITHGMDELYK

SEQ ID NO: 192 - protein, 699 aa, Artificial Sequence
  Fusion of BM3h and superfolder GFP
TIKEMPQPKTFGELKNLPLLNTDKPVQALMKIADELGEIFKFEAPGRVTRYLSSQRLIKEACDESRFDKNLSQALKFVRDFAGDGLFTSWTHEKNWKKAHNILLPSFSQQAMKGYHAMMVDIAVQLVQKWERLNADEHIEVPEDMTRLTLDTIGLCGFNYRFNSFYRDQPHPFITSMVRALDEAMNKLQRANPDDPAYDENKRQFQEDIKVMNDLVDKIIADRKASGEQSDDLLTHMLNGKDPETGEPLDDENIRYQIITFLIAGHETTSGLLSFALYFLVKNPHVLQKAAEEAARVLVDPVPSYKQVKQLKYVGMVLNEALRLWPTAPAFSLYAKEDTVLGGEYPLEKGDELMVLIPQLHRDKTIWGDDVEEFRPERFENPSAIPQHAFKPFGNGQRACIGQQFALHEATLVLGMMLKHFDFEDHTNYELDIKETLTLKPEGFVVKAKSKKIPLPPPPRTGSKGEELFTGVVPILVELDGDVNGHKFSVRGEGEGDATNGKLTLKFICTTGKLPVPWPTLVTTLTYGVQCFSRYPDHMKRHDFFKSAMPEGYVQERTISFKDDGTYKTRAEVKFEGDTLVNRIELKGIDFKEDGNILGHKLEYNFNSHNVYITADKQKNGIKANFKIRHNVEDGSVQLADHYQQNTPIGDGPVLLPDNHYLSTQSVLSKDPNEKRDHMVLLEFVTAAGITHGMDELYK

SEQ ID NO: 193 - protein, 135 aa, Homo sapiens
FATRQVGNVTKPTVIISQEGDKVVIRTLSTFKNTEISFQLGEEFDETTADDRNCKSVVSLDGDKLVHIQKWDGKETNFVREIKDGKMVMTLTFGDVVAVRHYEKAGGGSGMVEAFCATWKLTNSQNFDEYMKALG

SEQ ID NO: 194 - protein, 955 aa, Artificial Sequence
  Fusion of six B-FABP flanked by DnaE split intein fragments C-intein (AA 103-137) on the N-term and N-Intein (AA 1-102)
MIKIATRKYLGKQNVYDIGVGEPHNFALKNGFIASNGGGVEAFCATWKLTNSQNFDEYMKALGVGFATRQVGNVTKPTVIISQEGDKVVIRTLSTFKNTEISFQLGEEFDETTADDRNCKSVVSLDGDKLVHIQKWDGKETNFVREIKDGKMVMTLTFGDVVAVRHYEKAGGGSGVEAFCATWKLTNSQNFDEYMKALGVGFATRQVGNVTKPTVIISQEGDKVVIRTLSTFKNTEISFQLGEEFDETTADDRNCKSVVSLDGDKLVHIQKWDGKETNFVREIKDGKMVMTLTFGDVVAVRHYEKAGGGSGVEAFCATWKLTNSQNFDEYMKALGVGFATRQVGNVTKPTVIISQEGDKVVIRTLSTFKNTEISFQLGEEFDETTADDRNCKSVVSLDGDKLVHIQKWDGKETNFVREIKDGKMVMTLTFGDVVAVRHYEKAGGGSGVEAFCATWKLTNSQNFDEYMKALGVGFATRQVGNVTKPTVIISQEGDKVVIRTLSTFKNTEISFQLGEEFDETTADDRNCKSVVSLDGDKLVHIQKWDGKETNFVREIKDGKMVMTLTFGDVVAVRHYEKAGGGSGVEAFCATWKLTNSQNFDEYMKALGVGFATRQVGNVTKPTVIISQEGDKVVIRTLSTFKNTEISFQLGEEFDETTADDRNCKSVVSLDGDKLVHIQKWDGKETNFVREIKDGKMVMTLTFGDVVAVRHYEKAGGGSGVEAFCATWKLTNSQNFDEYMKALGVGFATRQVGNVTKPTVIISQEGDKVVIRTLSTFKNTEISFQLGEEFDETTADDRNCKSVVSLDGDKLVHIQKWDGKETNFVREIKDGKMVMTLTFGDVVAVRHYEKAGGGCLSYETEILTVEYGLLPIGKIVEKRIECTVYSVDNNGNIYTQPVAQWHDRGEQEVFEYCLEDGSLIRATKDHKFMTVDGQMLPIDEIFERELDLMRVDNLPN

SEQ ID NO: 195 - protein, 651 aa, Artificial Sequence
  Fusion of three repeats of B-FABP fused to MmMT3 flanked by DnaE split intein fragments C-intein (AA 103-137) on the N-term and N-Intein (AA 1-102)
MIKIATRKYLGKQNVYDIGVGEPHNFALKNGFIASNGGGVEAFCATWKLTNSQNFDEYMKALGVGFATRQVGNVTKPTVIISQEGDKVVIRTLSTFKNTEISFQLGEEFDETTADDRNCKSVVSLDGDKLVHIQKWDGKETNFVREIKDGKMVMTLTFGDVVAVRHYEKAGGGMDPETCPCPTGGSCTCSDKCKCKGCKCTNCKKSCCSCCPAGCEKCAKDCVCKGEEGAKAEAEKCSCCQGGGVEAFCATWKLTNSQNFDEYMKALGVGFATRQVGNVTKPTVIISQEGDKVVIRTLSTFKNTEISFQLGEEFDETTADDRNCKSVVSLDGDKLVHIQKWDGKETNFVREIKDGKMVMTLTFGDVVAVRHYEKAGGGMDPETCPCPTGGSCTCSDKCKCKGCKCTNCKKSCCSCCPAGCEKCAKDCVCKGEEGAKAEAEKCSCCQVEAFCATWKLTNSQNFDEYMKALGVGFATRQVGNVTKPTVIISQEGDKVVIRTLSTFKNTEISFQLGEEFDETTADDRNCKSVVSLDGDKLVHIQKWDGKETNFVREIKDGKMVMTLTFGDVVAVRHYEKAGGGMDPETCPCPTGGSCTCSDKCKCKGCKCTNCKKSCCSCCPAGCEKCAKDCVCKGEEGAKAEAEKCSCCQGGG

SEQ ID NO: 196 - protein, 1094 aa, Artificial Sequence
  Fusion of three repeats of 2x B-FABP intermixed by SpyTag003 and Spycatcher003 and flanked by DnaE split intein fragments C-intein (AA 103-137) on the N-term and N-Intein (AA 1-102)
MIKIATRKYLGKQNVYDIGVGEPHNFALKNGFIASNGGGVEAFCATWKLTNSQNFDEYMKALGVGFATRQVGNVTKPTVIISQEGDKVVIRTLSTFKNTEISFQLGEEFDETTADDRNCKSVVSLDGDKLVHIQKWDGKETNFVREIKDGKMVMTLTFGDVVAVRHYEKAGGGSGVEAFCATWKLTNSQNFDEYMKALGVGFATRQVGNVTKPTVIISQEGDKVVIRTLSTFKNTEISFQLGEEFDETTADDRNCKSVVSLDGDKLVHIQKWDGKETNFVREIKDGKMVMTLTFGDVVAVRHYEKAGGGSGRGVPHIVMVDAYKRYKGGGSGVEAFCATWKLTNSQNFDEYMKALGVGFATRQVGNVTKPTVIISQEGDKVVIRTLSTFKNTEISFQLGEEFDETTADDRNCKSVVSLDGDKLVHIQKWDGKETNFVREIKDGKMVMTLTFGDVVAVRHYEKAGGGSGVEAFCATWKLTNSQNFDEYMKALGVGFATRQVGNVTKPTVIISQEGDKVVIRTLSTFKNTEISFQLGEEFDETTADDRNCKSVVSLDGDKLVHIQKWDGKETNFVREIKDGKMVMTLTFGDVVAVRHYEKAGGGSGVTTLSGLSGEQGPSGDMTTEEDSATHIKFSKRDEDGRELAGATMELRDSSGKTISTWISDGHVKDFYLYPGKYTFVETAAPDGYEVATPIEFTVNEDGQVTVDGEATEGDAHTGGGSGVEAFCATWKLTNSQNFDEYMKALGVGFATRQVGNVTKPTVIISQEGDKVVIRTLSTFKNTEISFQLGEEFDETTADDRNCKSVVSLDGDKLVHIQKWDGKETNFVREIKDGKMVMTLTFGDVVAVRHYEKAGGGSGVEAFCATWKLTNSQNFDEYMKALGVGFATRQVGNVTKPTVIISQEGDKVVIRTLSTFKNTEISFQLGEEFDETTADDRNCKSVVSLDGDKLVHIQKWDGKETNFVREIKDGKMVMTLTFGDVVAVRHYEKAGGGCLSYETEILTVEYGLLPIGKIVEKRIECTVYSVDNNGNIYTQPVAQWHDRGEQEVFEYCLEDGSLIRATKDHKFMTVDGQMLPIDEIFERELDLMRVDNLPN

SEQ ID NO: 197 - protein, 317 aa, Artificial Sequence
  Fusion of QtEncapsulin and M13 a synthetic peptide binding Calmodulin
NKSQLYPDSPLTDQDFNQLDQTVIEAARRQLVGRRFIELYGPLGRGMQSVFNDIFMESHEAKMDFQGSFDTEVESSRRVNYTIPMLYKDFVLYWRDLEQSKALDIPIDFSVAANAARDVAFLEDQMIFHGSKEFDIPGLMNVKGRLTHLIGNWYESGNAFQDIVEARNKLLEMNHNGPYALVLSPELYSLLHRVHKDTNVLEIEHVRELITAGVFQSPVLKGKSGVIVNTGRNNLDLAISEDFETAYLGEEGMNHPFRVYETVVLRIKRPAAICTLIDPEEPPPPRPPPPRKRRWKKNFIAVSAANRFKKISSSGAL

SEQ ID NO: 198 - protein, 283 aa, Homo sapiens
VEAFCATWKLTNSQNFDEYMKALGVGFATRQVGNVTKPTVIISQEGDKVVIRTLSTFKNTEISFQLGEEFDETTADDRNCKSVVSLDGDKLVHIQKWDGKETNFVREIKDGKMVMTLTFGDVVAVRHYEKPPPPRADQLTDEQIAEFKEAFSLFDKDGDGTITTKELGTVMRSLGQNPTEAELQDMINEVDADGNGTIDFPEFLNLMARKMKDTDSEEKLKEAFRVFDKDGNGFISAAELRHVMTNLGEKLTDEEVDEMIREADVDGDGQVNYEEFVQVMMAK

SEQ ID NO: 199 - protein, 13 aa, Artificial Sequence
  Synthetic Silver mineralizing peptide 4
MNPSSLFRYLPSD

SEQ ID NO: 200 - protein, 1020 aa, Prevotella sp.
MKRTADGSEFESPKKKRKVNIPALVENQKKYFGTYSVMAMLNAQTVLDHIQKVADIEGEQNENNENLWFHPVMSHLYNAKNGYDKQPEKTMFIIERLQSYFPFLKIMAENQREYSNGKYKQNRVEVNSNDIFEVLKRAFGVLKMYRDLTNAYKTYEEKLNDGCEFLTSTEQPLSGMINNYYTVALRNMNERYGYKTEDLAFIQDKRFKFVKDAYGKKKSQVNTGFFLSLQDYNGDTQKKLHLSGVGIALLICLFLDKQYINIFLSRLPIFSSYNAQSEERRIIIRSFGINSIKLPKDRIHSEKSNKSVAMDMLNEVKRCPDELFTTLSAEKQSRFRIISDDHNEVLMKRSSDRFVPLLLQYIDYGKLFDHIRFHVNMGKLRYLLKADKTCIDGQTRVRVIEQPLNGFGRLEEAETMRKQENGTFGNSGIRIRDFENMKRDDANPANYPYIVDTYTHYILENNKVEMFINDKEDSAPLLPVIEDDRYVVKTIPSCRMSTLEIPAMAFHMFLFGSKKTEKLIVDVHNRYKRLFQAMQKEEVTAENIASFGIAESDLPQKILDLISGNAHGKDVDAFIRLTVDDMLTDTERRIKRFKDDRKSIRSADNKMGKRGFKQISTGKLADFLAKDIVLFQPSVNDGENKITGLNYRIMQSAIAVYDSGDDYEAKQQFKLMFEKARLIGKGTTEPHPFLYKVFARSIPANAVEFYERYLIERKFYLTGLSNEIKKGNRVDVPFIRRDQNKWKTPAMKTLGRIYSEDLPVELPRQMFDNEIKSHLKSLPQMEGIDFNNANVTYLIAEYMKRVLDDDFQTFYQWNRNYRYMDMLKGEYDRKGSLQHCFTSVEEREGLWKERASRTERYRKQASNKIRSNRQMRNASSEEIETILDKRLSNSRNEYQKSEKVIRRYRVQDALLFLLAKKTLTELADFDGERFKLKEIMPDAEKGILSEIMPMSFTFEKGGKKYTITSEGMKLKNYGDFFVLASDKRIGNLLELVGSDIVSKEDGSKRTADGSEFEPKKKRKV

SEQ ID NO: 201 - protein, 1186 aa, Homo sapiens
MSVACVLKRKAVLWQDSFSPHLKHHPQEPANPNMPVVLTSGTGSQAQPQPAANQALAAGTHSSPVPGSIGVAGRSQDDAMVDYFFQRQHGEQLGGGGSGGGGYNNSKHRWPTGDNIHAEHQVRSMDELNHDFQALALEGRAMGEQLLPGKKFWETDESSKDGPKGIFLGDQWRDSAWGTSDHSVSQPIMVQRRPGQSFHVNSEVNSVLSPRSESGGLGVSMVEYVLSSSPGDSCLRKGGFGPRDADSDENDKGEKKNKGTFDGDKLGDLKEEGDVMDKTNGLPVQNGIDADVKDFSRTPGNCQNSANEVDLLGPNQNGSEGLAQLTSTNGAKPVEDFSNMESQSVPLDPMEHVGMEPLQFDYSGTQVPVDSAAATVGLFDYNSQQQLFQRPNALAVQQLTAAQQQQYALAAAHQPHIGLAPAAFVPNPYIISAAPPGTDPYTAGLAAAATLGPAVVPHQYYGVTPWGVYPASLFQQQAAAAAAATNSANQQTTPQAQQGQQQVLRGGASQRPLTPNQNQQGQQTDPLVAAAAVNSALAFGQGLAAGMPGYPVLAPAAYYDQTGALVVNAGARNGLGAPVRLVAPAPVIISSSAAQAAVAAAAASANGAAGGLAGTTNGPFRPLGTQQPQPQPQQQPNNNLASSSFYGNNSLNSNSQSSSLFSQGSAQPANTSLGFGSSSSLGATLGSALGGFGTAVANSNTGSGSRRDSLTGSSDLYKRTSSSLTPIGHSFYNGLSFSSSPGPVGMPLPSQGPGHSQTPPPSLSSHGSSSSLNLGGLTNGSGRYISAAPGAEAKYRSASSASSLFSPSSTLFSSSRLRYGMSDVMPSGRSRLLEDFRNNRYPNLQLREIAGHIMEFSQDQHGSRFIQLKLERATPAERQLVFNEILQAAYQLMVDVFGNYVIQKFFEFGSLEQKLALAERIRGHVLSLALQMYGCRVIQKALEFIPSDQQNEMVRELDGHVLKCVKDQNGNHVVQKCIECVQPQSLQFIIDAFKGQVFALSTHPYGCRVIQRILEHCLPDQTLPILEELHQHTEQLVQDQYGNYVIQHVLEHGRPEDKSKIVAEIRGNVLVLSQHKFASNVVEKCVTHASRTERAVLIDEVCTMNDGPHSALYTMMKDQYANYVVQKMIDVAEPGQRKIVMHKIRPHIATLRKYTYGKHILAKLEKYYMKNGVDLGPICGPPNGII

SEQ ID NO: 202 - protein, 139 aa, Anguilla anguilla
MLEKFVGTWKIADSHNFGEYLKAIGAPKELSDGGDATTPTLYISQKDGDKMSVKIENGPPTFLDTQVKFKLGEEFDEFPSDRRKGVKSVVNLVGEKLVYVQKWDGKETTYVREIKDGKLVVTLTMGDVVAVRSYRRATE

SEQ ID NO: 203 - protein, 239 aa, Aequorea victoria
MVSKGEELFTGVVPILVELDGDVNGHKFSVRGEGEGDATNGKLTLKFICTTGKLPVPWPTLVTTLGYGVACFARYPDHMKQHDFFKSAMPEGYVQERTISFKDDGTYKTRAEVKFEGDTLVNRIVLKGIDFKEDGNILGHKLEYNFNSHKVYITADKQKNGIKANFKTRHNVEDGGVQLADHYQQNTPIGDGPVLLPDNHYLSHQSKLSKDPNEKRDHMVLKERVTAAGITHDMDELYK

SEQ ID NO: 204 - protein, 408 aa, Artificial Sequence
  Engineered fluorescent Calcium integrator
MGSDQLTEEQIAEFKEAFSLFDKDGDGTITTKELGTVMRSLGQNPTEAELQDMINEVDADGDGTIDFPEFLTMMARKMKDTDSEEEIREAFRVFDKDGNGYISAAELRHVMTNLGEKLTDEEVDEMIREADIDGDGQVNYEEFVVMMTAKLECEKIYVRDGVLTGDIHMILLLEGNAHYRCDFRTTYKAKEKGVKLPGVHYVDHTIEILSHDKDYNKVKIYEYAVAHSGLPDNARRGGTGGSMVSAIKPDMKIKLRMEGNVNGHHFVIDGDGTGKPYEGKQTMDLEVKEGGPLPFAFDILTTAFHYGNRVFVKYPDNIQDYFKQSFPKGYSWERSMTFEDGGICYARSDITMEGDTFYNKVRFYGTNFPANGPVMQKKTLKWMPSWTRSSRRKFNKTGHALRAIGRLS

SEQ ID NO: 205 - protein, 225 aa, Discosoma sp.
MASSEDVIKEFMRFKVRMEGSVNGHEFEIEGEGEGRPYEGTQTAKLKVTKGGPLPFAWDILSPQFQYGSKAYVKHPADIPDYLKLSFPEGFKWERVMNFEDGGVVTVTQDSSLQDGEFIYKVKLRGTNFPSDGPVMQKKTMGWEASTERMYPEDGALKGEIKMRLKLKDGGHYDAEVKTTYMAKKPVQLPGAYKTDIKLDITSHNEDYTIVEQYERAEGRHSTGA

SEQ ID NO: 206 - protein, 121 aa, Artificial Sequence
  phostphopetptide binding Forkhead-associated domain
FLTLKPLPDSIIQESLEIQQGVNPFFIGRSEDCNCKIEDNRLSRVHCFIFKKRHAVGKSMYESPAQGLDDIWYCHTGTNVSYLNNNRMIQGTKFLLQDGDEIKIIWDKNNKFVIGFKVEIN

SEQ ID NO: 207 - protein, 131 aa, Artificial Sequence
  Coat protein
MANKPMQPITSTANKIVWSDPTRLSTTFSASLLRQRVKVGIAELNNVSGQYVSVYKRPAPKPEGCADACVIMPNENQSIRTVISGSAENLATLKAEWETHKRNVDTLFASGNAGLGFLDPTAAIVSSDTTA

SEQ ID NO: 208 - protein, 678 aa, Artificial Sequence
  Fusion of mEos4b together with APEX2 to a C-terminal minimal interaction domain (mINT)
MVSAIKPDMRIKLRMEGNVNGHHFVIDGDGTGKPYEGKQTMDLEVKEGGPLPFAFDILTTAFHYGNRVFVKYPDNIQDYFKQSFPKGYSWERSLTFEDGGICNARNDITMEGDTFYNKVRFYGTNFPANGPVMQKKTLKWEPSTEKMYVRDGVLTGDIEMALLLEGNAHYRCDFRTTYKAKEKGVKLPGAHFVDHAIEILSHDKDYNKVKLYEHAVAHSGLPDNARRGGGGSGGGGDYKDDDDKGKSYPTVSADYQDAVEKAKKKLRGFIAEKRCAPLMLRLAFHSAGTFDKGTKTGGPFGTIKHPAELAHSANNGLDIAVRLLEPLKAEFPILSYADFYQLAGVVAVEVTGGPKVPFHPGREDKPEPPPEGRLPDPTKGSDHLRDVFGKAMGLTDQDIVALSGGHTIGAAHKERSGFEGPWTSNPLIFDNSYFTELLSGEKEGLLQLPSDKALLSDPVFRPLVDKYAADEDAFFADYAEAHQKLSELGFADALQLPPLERLTLDGGGSGGGGSGGGDDEGRQSPVSWTSLFALQTEDGFWKLTPELGLILKLNVNALLNSLEEKGIRSLGTKGRERLLDLIATLLVLQFLYTKLEQEGMAAKSLIKMDDVLISRNIPWAFENIKKAREWARRTEGQYPSICQRLELGKDWESATKQLLGIQHQGNTSLHRILHYSQG

SEQ ID NO: 209 - protein, 880 aa, Artificial Sequence
  Fusion of mouse Gap43 palmitoylation signal to the N-terminus of the major vault protein (MVP).
MLCCMRRTKQVEKNDEDQKIATEEAIIRIPPYHYIHVLDQNSNVSRVEVGPKTYIRQDNERVLFAPVRMVTVPPRHYCIVANPVSRDTQSSVLFDITGQVRLRHADQEIRLAQDPFPLYPGEVLEKDITPLQVVLPNTALHLKALLDFEDKNGDKVMAGDEWLFEGPGTYIPQKEVEVVEIIQATVIKQNQALRLRARKECFDREGKGRVTGEEWLVRSVGAYLPAVFEEVLDLVDAVILTEKTALHLRALQNFRDLRGVLHRTGEEWLVTVQDTEAHVPDVYEEVLGVVPITTLGPRHYCVILDPMGPDGKNQLGQKRVVKGEKSFFLQPGERLERGIQDVYVLSEQQGLLLKALQPLEEGESEEKVSHQAGDCWLIRGPLEYVPSAKVEVVEERQAIPLDQNEGIYVQDVKTGKVRAVIGSTYMLTQDEVLWEKELPSGVEELLNLGHDPLADRGQKGTAKPLQPSAPRNKTRVVSYRVPHNAAVQVYDYRAKRARVVFGPELVTLDPEEQFTVLSLSAGRPKRPHARRALCLLLGPDFFTDVITIETADHARLQLQLAYNWHFELKNRNDPAEAAKLFSVPDFVGDACKAIASRVRGAVASVTFDDFHKNSARIIRMAVFGFEMSEDTGPDGTLLPKARDQAVFPQNGLVVSSVDVQSVEPVDQRTRDALQRSVQLAIEITTNSQEAAAKHEAQRLEQEARGRLERQKILDQSEAEKARKELLELEAMSMAVESTGNAKAEAESRAEAARIEGEGSVLQAKLKAQALAIETEAELERVKKVREMELIYARAQLELEVSKAQQLANVEAKKFKEMTEALGPGTIRDLAVAGPEMQVKLLQSLGLKSTLITDGSSPINLFSTAFGLLGLGSDGQPPAQK

SEQ ID NO: 210 - protein, 485 aa, Artificial Sequence
  N-terminal fusion of SNAP-tag connected via GS linker to QtEnc with a C-terminal FLAG epitope
MDKDCEMKRTTLDSPLGKLELSGCEQGLHRIIFLGKGTSAADAVEVPAPAAVLGGPEPLMQATAWLNAYFHQPEAIEEFPVPALHHPVFQQESFTRQVLWKLLKVVKFGEVISYSHLAALAGNPAATAAVKTALSGNPVPILIPCHRVVQGDLDVGGYEGGLAVKEWLLAHEGHRLGKPGLGGGTGGSGSGPGNKSQLYPDSPLTDQDFNQLDQTVIEAARRQLVGRRFIELYGPLGRGMQSVFNDIFMESHEAKMDFQGSFDTEVESSRRVNYTIPMLYKDFVLYWRDLEQSKALDIPIDFSVAANAARDVAFLEDQMIFHGSKEFDIPGLMNVKGRLTHLIGNWYESGNAFQDIVEARNKLLEMNHNGPYALVLSPELYSLLHRVHKDTNVLEIEHVRELITAGVFQSPVLKGKSGVIVNTGRNNLDLAISEDFETAYLGEEGMNHPFRVYETVVLRIKRPAAICTLIDPEEGSGDYKDDDDK

SEQ ID NO: 211 - protein, 600 aa, Artificial Sequence
  N-terminal fusion of Halo-tag connected via GS linker to QtEnc with a C-terminal FLAG epitope
MAEIGTGFPFDPHYVEVLGERMHYVDVGPRDGTPVLFLHGNPTSSYVWRNIIPHVAPTHRCIAPDLIGMGKSDKPDLGYFFDDHVRFMDAFIEALGLEEVVLVIHDWGSALGFHWAKRNPERVKGIAFMEFIRPIPTWDEWPEFARETFQAFRTTDVGRKLIIDQNVFIEGTLPMGVVRPLTEVEMDHYREPFLNPVDREPLWRFPNELPIAGEPANIVALVEEYMDWLHQSPVPKLLFWGTPGVLIPPAEAARLAKSLPNCKAVDIGPGLNLLQEDNPDLIGSEIARWLSTLEISGGGTGGSGSGPGNKSQLYPDSPLTDQDFNQLDQTVIEAARRQLVGRRFIELYGPLGRGMQSVFNDIFMESHEAKMDFQGSFDTEVESSRRVNYTIPMLYKDFVLYWRDLEQSKALDIPIDFSVAANAARDVAFLEDQMIFHGSKEFDIPGLMNVKGRLTHLIGNWYESGNAFQDIVEARNKLLEMNHNGPYALVLSPELYSLLHRVHKDTNVLEIEHVRELITAGVFQSPVLKGKSGVIVNTGRNNLDLAISEDFETAYLGEEGMNHPFRVYETVVLRIKRPAAICTLIDPEEGSGDYKDDDDK

SEQ ID NO: 212 - protein, 320 aa, Artificial Sequence
  Fusion of MT3 to AA 110-346 of Pyrococcus furiosus Encapsulin monomer with a C-terminal FLAG epitope.
MDPETCPCPTGGSCTCSDKCKCKGCKCTNCKKSCCSCCPAGCEKCAKDCVCKGEEGAKAEAEKCSCCQGSGPGVEYFEKLRSALLDGVNKGRSLLKHLPVTRIEGQSFRVDIIKFEDGVRVVKQEYKPIPLLKKKFYVGIRELNDGTYDVSIATKAGELLVKDEESLVIREILSTEGIKKMKLSSWDNPEEALNDLMNALQEASNASAGPFGLIINPKRYAKLLKIYEKSGKMLVEVLKEIFRGGIIVTLNIDENKVIIFANTPAVLDVVVGQDVTLQELGPEGDDVAFLVSEAIGIRIKNPEAIVVLEGSGDYKDDDDK

SEQ ID NO: 213 - protein, 320 aa, Pyrococcus furiosus; identical to SEQ ID NO: 212

SEQ ID NO: 214 - protein, 227 aa, Artificial Sequence
  mEos4b
MVSAIKPDMRIKLRMEGNVNGHHFVIDGDGTGKPYEGKQTMDLEVKEGGPLPFAFDILTTAFHYGNRVFVKYPDNIQDYFKQSFPKGYSWERSLTFEDGGICNARNDITMEGDTFYNKVRFYGTNFPANGPVMQKKTLKWEPSTEKMYVRDGVLTGDIEMALLLEGNAHYRCDFRTTYKAKEKGVKLPGAHFVDHAIEILSHDKDYNKVKLYEHAVAHSGLPDNARR

SEQ ID NO: 215 - protein, 227 aa, Artificial Sequence
  mEosEM
MVSAIKPDMRIKLRMEGNVNGHHFVIDGEGTGKPYEGKQTMDLEVKEGGPLPFAFDILTTAFHYGNRVFVKYPDNIQDYFKQSFPKGYSWERSMTFEDGGICNARNDITMEGDTFYNKVRFYGTNFPANGPVMQKKTLKWEPSTEKMYVRDGVLTGDIEMALLLEGGAHYRCDFRTTYKAKEKGVKLPGAHFVDHAIEILSHDKDYNKVKLYEHAVAHSGLPDNARR

SEQ ID NO: 216 - protein, 316 aa, Artificial Sequence
  iRFP713
MAEGSVARQPDLLTCDDEPIHIPGAIQPHGLLLALAADMTIVAGSDNLPELTGLAIGALIGRSAADVFDSETHNRLTIALAEPGAAVGAPITVGFTMRKDAGFIGSWHRHDQLIFLELEPPQRDVAEPQAFFRRTNSAIRRLQAAETLESACAAAAQEVRKITGFDRVMIYRFASDFSGEVIAEDRCAEVESKLGLHYPASTVPAQARRLYTINPVRIIPDINYRPVPVTPDLNPVTGRPIDLSFAILRSVSPVHLEFMRNIGMHGTMSISILRGERLWGLIVCHHRTPYYVDLDGRQACELVAQVLAWQIGVMEE

SEQ ID NO: 217 - protein, 132 aa, Artificial Sequence
  TeAPCalpha
MKTGEQRVKIATLLSENEKKIVDKASQDLWRRRPDFIAPGGNAFGQRERALCLRDYGWYLRLITYGLLAGDKDPIESIGLIGVREMYNSLGVPVPGMVESIRCLKEASLSLLDEEDAKETAPYFDYIIQAMS

SEQ ID NO: 218 - protein, 494 aa, Homo sapiens
DLSLSDINSTVEVPEGHSFWKTLLAYSGPGALVAVGYMDPGNWSTSITGGQNFQYLLLSIIVISSLLAMLLQNMAAKLGIVCQLDLAQAIRARTSRRLGFIFWILTELAIMATDIAEVIGAAIALYLLFKIPIFLAVVITVLDVFLLLLLNRIGFRKIEALVVCLIFVILFVFLYQIILSQPAWHQVAKGLIPSWASVQTSPKIGGQTPLSASLGIIGATIMPHNLFLHSAISQSRKIDRTDSSKVAEAVRFSNWDSNIQLSLAMVVNALLLIMGVAVFKSGAVQDPSFFGLYQALSNPDMVSNPVLAEAARSGVLSTLFAVALLASGQNSTITGTITGQVIMEGFIHLRLPLWLRRLVTRLIAIIPVVVCVAITSHQGSLDEHQALNNLMNNSQVFLALALPFSIVPLLMLTDSAAQMGNQFKNTRWVKVMGWLTVIILTLLNLISISSQIAGFFGDNPSSQDLLLSQVISIGIILAMIGLLIWTIIDIRRFT

SEQ ID NO: 219 - protein, 492 aa, Homo sapiens
MKLLLLHPAFQSCLLLTLLGLWRTTPEAHASSLGAPAISAASFLQDLIHRYGEGDSLTLQQLKALLNHLDVGVGRGNVTQHVQGHRNLSTCFSSGDLFTAHNFSEQSRIGSSELQEFCPTILQQLDSRACTSENQENEENEQTEEGRPSAVEVWGYGLLCVTVISLCSLLGASVVPFMKKTFYKRLLLYFIALAIGTLYSNALFQLIPEAFGFNPLEDYYVSKSAVVFGGFYLFFFTEKILKILLKQKNEHHHGHSHYASESLPSKKDQEEGVMEKLQNGDLDHMIPQHCSSELDGKAPMVDEKVIVGSLSVQDLQASQSACYWLKGVRYSDIGTLAWMITLSDGLHNFIDGLAIGASFTVSVFQGISTSVAILCEEFPHELGDFVILLNAGMSIQQALFFNFLSACCCYLGLAFGILAGSHFSANWIFALAGGMFLYISLADMFPEMNEVCQEDERKGSILIPFIIQNLGLLTGFTIMVVLTMYSGQIQIG

SEQ ID NO: 220 - protein, 425 aa, Artificial Sequence
  Fusion of Cystathionine gamma-lyase with QtSig
MQEKDASSQGFLPHFQHFATQAIHVGQDPEQWTSRAVVPPISLSTTFKQGAPGQHSGFEYSRSGNPTRNCLEKAVAALDGAKYCLAFASGLAATVTITHLLKAGDQIICMDDVYGGTNRYFRQVASEFGLKISFVDCSKIKLLEAAITPETKLVWIETPTNPTQKVIDIEGCAHIVHKHGDIILVVDNTFMSPYFQRPLALGADISMYSATKYMNGHSDVVMGLVSVNCESLHNRLRFLQNSLGAVPSPIDCYLCNRGLKTLHVRMEKHFKNGMAVAQFLESNPWVEKVIYPGLPSHPQHELVKRQCTGCTGMVTFYIKGTLQHAEIFLKNLKLFTLAESLGGFESLAELPAIMTHASVLKNDRDVLGISDTLIRLSVGLEDEEDLLEDLDQALKAAHPPSGSHSGGGGSGGGGSKGFTVGSLIQ

SEQ ID NO: 221 - protein, 1070 aa, Artificial Sequence
  Fusion of Seap, a secreted form of Human embryonic alkaline phosphatase, and QtSig
MLGPCMLLLLLLLGLRLQLSLGIIPVEEENPDFWNREAAEALGAAKKLQPAQTAAKNLIIFLGDGMGVSTVTAARILKGQKKDKLGPEIPLAMDRFPYVALSKTYNVDKHVPDSGATATAYLCGVKGNFQTIGLSAAARFNQCNTTRGNEVISVMNRAKKAGKSVGVVTTTRVQHASPAGTYAHTVNRNWYSDADVPASARQEGCQDIATQLISNMDIDVILGGGRKYMFRMGTPDPEYPDDYSQGGTRLDGKNLVQEWLAKRQGARYVWNRTELMQASLDPSVTHLMGLFEPGDMKYEIHRDSTLDPSLMEMTEAALRLLSRNPRGFFLFVEGGRIDHGHHESRAYRALTETIMFDDAIERAGQLTSEEDTLSLVTADHSHVFSFGGYPLRGSSIFGLAPGKARDRKAYTVLLYGNGPGYVLKDGARPDVTESESGSPEYRQQSAVPLDEETHAGEDVAVFARGPQAHLVHGVQEQTFIAHVMAFAACLEPYTACDLAPPAGTTDAAHPGRSVVPALLPLLAGTLLLLETATAPMLGPCMLLLLLLLGLRLQLSLGIIPVEEENPDFWNREAAEALGAAKKLQPAQTAAKNLIIFLGDGMGVSTVTAARILKGQKKDKLGPEIPLAMDRFPYVALSKTYNVDKHVPDSGATATAYLCGVKGNFQTIGLSAAARFNQCNTTRGNEVISVMNRAKKAGKSVGVVTTTRVQHASPAGTYAHTVNRNWYSDADVPASARQEGCQDIATQLISNMDIDVILGGGRKYMFRMGTPDPEYPDDYSQGGTRLDGKNLVQEWLAKRQGARYVWNRTELMQASLDPSVTHLMGLFEPGDMKYEIHRDSTLDPSLMEMTEAALRLLSRNPRGFFLFVEGGRIDHGHHESRAYRALTETIMFDDAIERAGQLTSEEDTLSLVTADHSHVFSFGGYPLRGSSIFGLAPGKARDRKAYTVLLYGNGPGYVLKDGARPDVTESESGSPEYRQQSAVPLDEETHAGEDVAVFARGPQAHLVHGVQEQTFIAHVMAFAACLEPYTACDLAPPAGTTDAAHPGRSVVPALLPLLAGTLLLLETATAP

SEQ ID NO: 222 - protein, 1237 aa, Artificial Sequence
  Fusion of MnxG, component of the Bacillus sp. Multimeric multicopper oxidase Mnx, and QtSig
MKRCFHVVAIPIRIVVNNFGDYNPNGMMYVLKENEHKVKRLVKKNPFSVVDLVQPLIIRANEGDEVEVLFENQLPFNTSMHFQEAEYDVLTSDGANVGFNPDTTVAPGCKILYRLRLPKEGAYIFSDLGNPSSSEQGSNSNGLFGALFVERRFSWWTDPVTGGPLNSGLYADVHHPILPSFREYAWLFSDEMEINDLTGNNPIDPVTGEPTESFHGVNYRYEPLHRRKQLIDEGVVCPDCDGEEVHHDSWVFGDPATPIFRGYVGDPAKIRLIHAGVKETHVFHYHVHQWFNDPDNLESEIFDSQAASPQSHYDIEPLYGLGSLQRAIGDAIIHCHLYPHFGIGMWGMNRVFDTLQDGSQSYPNGVKIDALQPLPDRPAPPRPTKEKPGFPNFIPGKPGFKAPRPPLGIVGGRGLTELEKNAAVPKARPGAVFADPCIENANVIEYNISLIELPLVYNKQGWHDPKGRIYILDEDIDDVCSGRKEPEPLIIHQPANTCIRINYTNRLPHILDGDAFQLVTRSYEAGMHIHFVKFDVLVNDGANVGWNYDSSILPGETMRYEYYADVELKAWFFHDHLFAVQHQQHGVFGSGVVHPRFTKFIDSNGGGEVGAGAQVTAVNPLIPDYRDFSLMVQDFSLLFDKKGNPIQPPEFPGSQDDPGLFGVNYKNEPLQFRLGPDCDPAYTFSSFVHGDPCTPILRAYEGDPIRIRLLQGAQEESHSFNVHGLRWSKERSDLDSMFREQQHIGISESFTFESYIPRAGDYLWAFETEEDLWNGLWGLIRAYDEVVPDLIPLTDRPRPLKRSRLLPYRTGKPPRKGDCFKDDLIIPHKRCVKEFDIVAFQVPIIYNEFGDVDQNGIVFSLREDMDDILSGLKNPEPLIIRANVGDEVRVKLTSLLEFDKFPFKDGIYPYPTVKEQAFYPPSLRISLHPQLIQYDVKTSSGETVGYNYDQTVGPGESITYKWYVDFPVGACGMWDMADIRNHKSQGAFGAFIAEPRGTEYLDPHTLKPVKTGASVVLRNNLLPDKREFVIIMHDGVRLHDKDGILITDPIDGILLGPDNPFEGDLVDTYDNGSRGFNYRSERLINRYRKHPVLHDLFSSKLFGDPSTPLFESYAGDPVTLRLIAPAERRRSHTFHLHGHYWRKDISDINSVTASFEGFNLAGSKQDFELFGGAGGFNQFPGDYMYRSGNIQWDIEQGMWGIMRVHGKRQPHLPPLEKGGGGSGGGGSKGFTVGSLIQ

SEQ ID NO: 223 - protein, 1237 aa, Bacillus sp.; identical to SEQ ID NO: 222

SEQ ID NO: 224 - protein, 103 aa, Bacillus sp.
MEALFPMSTDYSKMTDVNEIHDSAILEHFRNGIGHKTLVISPSYPYMFVGIIKELIGDTVMIDVETTHFAQLENREWYIHIHNIEVFYIERPGAPKIPKLEDY

SEQ ID NO: 225 - protein, 82 aa, Artificial Sequence
  Designed uranyl binder with femtomolar affinity
SNALDCRERIEKDLEDLEKELMEMKSIKLSDDEEAVVERALNYRDDSVYYLEKGDHITSFGCITYAEGLTDSLRMLHRIIEG

SEQ ID NO: 226 - protein, 388 aa, Artificial Sequence
  Coiled-coil adapter to recruit an encapsulated cargo, such as the fluorescent protein mEosEM fused to P4  to an encapsulin already harboring an MT3 for dual EM and fluorescence detection.
SPEDEIQQLEEEIAQLEQKNAALKEKNQALKYGSGMDPETCPCPTGGSCTCSDKCKCKGCKCTNCKKSCCSCCPAGCEKCAKDCVCKGEEGAKAEAEKCSCCQGSGGNKSQLYPDSPLTDQDFNQLDQTVIEAARRQLVGRRFIELYGPLGRGMQSVFNDIFMESHEAKMDFQGSFDTEVESSRRVNYTIPMLYKDFVLYWRDLEQSKALDIPIDFSVAANAARDVAFLEDQMIFHGSKEFDIPGLMNVKGRLTHLIGNWYESGNAFQDIVEARNKLLEMNHNGPYALVLSPELYSLLHRVHKDTNVLEIEHVRELITAGVFQSPVLKGKSGVIVNTGRNNLDLAISEDFETAYLGEEGMNHPFRVYETVVLRIKRPAAICTLIDPEE

SEQ ID NO: 227 - protein, 497 aa, Artificial Sequence
  Fusion of the fluorescent protein eUnaG to the outer surface of encapsulin
MDPETCPCPTGGSCTCSDKCKCKGCKCTNCKKSCCSCCPAGCEKCAKDCVCKGEEGAKAEAEKCSCCQGSGGNKSQLYPDSPLTDQDFNQLDQTVIEAARRQLVGRRFIELYGPLGRGMQSVFNDIFMESHEAKMDFQGSFDTEVESSRRVNYTIPMLYKDFVLYWRDLEQSKALDIPIDFSVAANAARDVAFLEDQMIFHGSKEFDIPGLMNVKGRLTHLIGNWYESGNAFQDIVEARNKLLEMNHNGPYALVLSPELYSLLHRVHKDTNVLEIEHVRELITAGVFQSPVLKGKSGVIVNTGRNNLDLAISEDFETAYLGEEGMNHPFRVYETVVLRIKRPAAICTLIDPEEGGGSGMLEKFVGTWKIADSHNFGEYLKAIGAPKELSDGGDATTPTLYISQKDGDKMSVKIENGPPTFLDTQVKFKLGEEFDEFPSDRRKGVKSVVNLVGEKLVYVQKWDGKETTYVREIKDGKLVVTLTMGDVVAVRSYRRATE

SEQ ID NO: 228 - protein, 312 aa, Artificial Sequence
  CGU for attaching to the outer surface of encapsulin via anti-GFP antibody
MDPETCPCPTGGSCTCSDKCKCKGCKCTNCKKSCCSCCPAGCEKCAKDCVCKGEEGAKAEAEKCSCCQPPPPRTGSKGEELFTGVVPILVELDGDVNGHKFSVRGEGEGDATNGKLTLKFICTTGKLPVPWPTLVTTLTYGVQCFSRYPDHMKRHDFFKSAMPEGYVQERTISFKDDGTYKTRAEVKFEGDTLVNRIELKGIDFKEDGNILGHKLEYNFNSHNVYITADKQKNGIKANFKIRHNVEDGSVQLADHYQQNTPIGDGPVLLPDNHYLSTQSVLSKDPNEKRDHMVLLEFVTAAGITHGMDELYK

SEQ ID NO: 229 - protein, 418 aa, Artificial Sequence
  Fusion of QtEnc and Brain FABP, embodiment of concentric barcodes added to the outer surface of encapsulins
NKSQLYPDSPLTDQDFNQLDQTVIEAARRQLVGRRFIELYGPLGRGMQSVFNDIFMESHEAKMDFQGSFDTEVESSRRVNYTIPMLYKDFVLYWRDLEQSKALDIPIDFSVAANAARDVAFLEDQMIFHGSKEFDIPGLMNVKGRLTHLIGNWYESGNAFQDIVEARNKLLEMNHNGPYALVLSPELYSLLHRVHKDTNVLEIEHVRELITAGVFQSPVLKGKSGVIVNTGRNNLDLAISEDFETAYLGEEGMNHPFRVYETVVLRIKRPAAICTLIDPEEGGGGSGVEAFCATWKLTNSQNFDEYMKALGVGFATRQVGNVTKPTVIISQEGDKVVIRTLSTFKNTEISFQLGEEFDETTADDRNCKSVVSLDGDKLVHIQKWDGKETNFVREIKDGKMVMTLTFGDVVAVRHYEKA

SEQ ID NO: 230 - protein, 742 aa, Artificial Sequence
  Fusion of QtEnc and Bm3h, embodiment of concentric barcodes added to the outer surface of encapsulins
NKSQLYPDSPLTDQDFNQLDQTVIEAARRQLVGRRFIELYGPLGRGMQSVFNDIFMESHEAKMDFQGSFDTEVESSRRVNYTIPMLYKDFVLYWRDLEQSKALDIPIDFSVAANAARDVAFLEDQMIFHGSKEFDIPGLMNVKGRLTHLIGNWYESGNAFQDIVEARNKLLEMNHNGPYALVLSPELYSLLHRVHKDTNVLEIEHVRELITAGVFQSPVLKGKSGVIVNTGRNNLDLAISEDFETAYLGEEGMNHPFRVYETVVLRIKRPAAICTLIDPEEGGGGSGTIKEMPQPKTFGELKNLPLLNTDKPVQALMKIADELGEIFKFEAPGRVTRYLSSQRLIKEACDESRFDKNLSQALKFVRDFAGDGLFTSWTHEKNWKKAHNILLPSFSQQAMKGYHAMMVDIAVQLVQKWERLNADEHIEVPEDMTRLTLDTIGLCGFNYRFNSFYRDQPHPFITSMVRALDEAMNKLQRANPDDPAYDENKRQFQEDIKVMNDLVDKIIADRKASGEQSDDLLTHMLNGKDPETGEPLDDENIRYQIITFLIAGHETTSGLLSFALYFLVKNPHVLQKAAEEAARVLVDPVPSYKQVKQLKYVGMVLNEALRLWPTAPAFSLYAKEDTVLGGEYPLEKGDELMVLIPQLHRDKTIWGDDVEEFRPERFENPSAIPQHAFKPFGNGQRACIGQQFALHEATLVLGMMLKHFDFEDHTNYELDIKETLTLKPEGFVVKAKSKKIPL

SEQ ID NO: 231 - protein, 355 aa, Artificial Sequence
  Fusion of QtEnc and MT3, embodiment of concentric barcodes added to the outer surface of encapsulins
NKSQLYPDSPLTDQDFNQLDQTVIEAARRQLVGRRFIELYGPLGRGMQSVFNDIFMESHEAKMDFQGSFDTEVESSRRVNYTIPMLYKDFVLYWRDLEQSKALDIPIDFSVAANAARDVAFLEDQMIFHGSKEFDIPGLMNVKGRLTHLIGNWYESGNAFQDIVEARNKLLEMNHNGPYALVLSPELYSLLHRVHKDTNVLEIEHVRELITAGVFQSPVLKGKSGVIVNTGRNNLDLAISEDFETAYLGEEGMNHPFRVYETVVLRIKRPAAICTLIDPEEGGGGSGMDPETCPCPTGGSCTCSDKCKCKGCKCTNCKKSCCSCCPAGCEKCAKDCVCKGEEGAKAEAEKCSCCQ

SEQ ID NO: 232 - protein, 380 aa, Artificial Sequence
  Fusion of Brain FABP and superfolder GFP, for attachment via anti-GFP intrabody attachment points, e.g. to the outer surface of Encapsulins.
VEAFCATWKLTNSQNFDEYMKALGVGFATRQVGNVTKPTVIISQEGDKVVIRTLSTFKNTEISFQLGEEFDETTADDRNCKSVVSLDGDKLVHIQKWDGKETNFVREIKDGKMVMTLTFGDVVAVRHYEKAPPPPRTGPPPPRSKGEELFTGVVPILVELDGDVNGHKFSVRGEGEGDATNGKLTLKFICTTGKLPVPWPTLVTTLTYGVQCFSRYPDHMKRHDFFKSAMPEGYVQERTISFKDDGTYKTRAEVKFEGDTLVNRIELKGIDFKEDGNILGHKLEYNFNSHNVYITADKQKNGIKANFKIRHNVEDGSVQLADHYQQNTPIGDGPVLLPDNHYLSTQSVLSKDPNEKRDHMVLLEFVTAAGITHGMDELYK

SEQ ID NO: 233 - protein, 704 aa, Artificial Sequence
  Fusion of Bm3h and superfolder GFP, or attachment via anti-GFP intrabody attachment points, e.g. to the outer surface of Encapsulins.
TIKEMPQPKTFGELKNLPLLNTDKPVQALMKIADELGEIFKFEAPGRVTRYLSSQRLIKEACDESRFDKNLSQALKFVRDFAGDGLFTSWTHEKNWKKAHNILLPSFSQQAMKGYHAMMVDIAVQLVQKWERLNADEHIEVPEDMTRLTLDTIGLCGFNYRFNSFYRDQPHPFITSMVRALDEAMNKLQRANPDDPAYDENKRQFQEDIKVMNDLVDKIIADRKASGEQSDDLLTHMLNGKDPETGEPLDDENIRYQIITFLIAGHETTSGLLSFALYFLVKNPHVLQKAAEEAARVLVDPVPSYKQVKQLKYVGMVLNEALRLWPTAPAFSLYAKEDTVLGGEYPLEKGDELMVLIPQLHRDKTIWGDDVEEFRPERFENPSAIPQHAFKPFGNGQRACIGQQFALHEATLVLGMMLKHFDFEDHTNYELDIKETLTLKPEGFVVKAKSKKIPLPPPPRTGPPPPRSKGEELFTGVVPILVELDGDVNGHKFSVRGEGEGDATNGKLTLKFICTTGKLPVPWPTLVTTLTYGVQCFSRYPDHMKRHDFFKSAMPEGYVQERTISFKDDGTYKTRAEVKFEGDTLVNRIELKGIDFKEDGNILGHKLEYNFNSHNVYITADKQKNGIKANFKIRHNVEDGSVQLADHYQQNTPIGDGPVLLPDNHYLSTQSVLSKDPNEKRDHMVLLEFVTAAGITHGMDELYK

SEQ ID NO: 234 - protein, 204 aa, Artificial Sequence
  Fusion of MT3 and Lam4, for attachment to mCherry, e.g. on SasG
MDPETCPCPTGGSCTCSDKCKCKGCKCTNCKKSCCSCCPAGCEKCAKDCVCKGEEGAKAEAEKCSCCQPPPPRTGPPPPRAQVQLVESGGSLVQPGGSLRLSCAASGRFAESSSMGWFRQAPGKEREFVAAISWSGGATNYADSAKGRFTLSRDNTKNTVYLQMNSLKPDDTAVYYCAANLGNYISSNQRLYGYWGQGTQVTVS

SEQ ID NO: 235 - protein, 267 aa, Artificial Sequence
  Fusion of Brain FABP and Lam4, , for attachment to mCherry, e.g. on SasG
VEAFCATWKLTNSQNFDEYMKALGVGFATRQVGNVTKPTVIISQEGDKVVIRTLSTFKNTEISFQLGEEFDETTADDRNCKSVVSLDGDKLVHIQKWDGKETNFVREIKDGKMVMTLTFGDVVAVRHYEKAPPPPRTGPPPPRAQVQLVESGGSLVQPGGSLRLSCAASGRFAESSSMGWFRQAPGKEREFVAAISWSGGATNYADSAKGRFTLSRDNTKNTVYLQMNSLKPDDTAVYYCAANLGNYISSNQRLYGYWGQGTQVTVS

SEQ ID NO: 236 - protein, 591 aa, Artificial Sequence
  Fusion of Bm3h and Lam4, , for attachment to mCherry, e.g. on SasG
TIKEMPQPKTFGELKNLPLLNTDKPVQALMKIADELGEIFKFEAPGRVTRYLSSQRLIKEACDESRFDKNLSQALKFVRDFAGDGLFTSWTHEKNWKKAHNILLPSFSQQAMKGYHAMMVDIAVQLVQKWERLNADEHIEVPEDMTRLTLDTIGLCGFNYRFNSFYRDQPHPFITSMVRALDEAMNKLQRANPDDPAYDENKRQFQEDIKVMNDLVDKIIADRKASGEQSDDLLTHMLNGKDPETGEPLDDENIRYQIITFLIAGHETTSGLLSFALYFLVKNPHVLQKAAEEAARVLVDPVPSYKQVKQLKYVGMVLNEALRLWPTAPAFSLYAKEDTVLGGEYPLEKGDELMVLIPQLHRDKTIWGDDVEEFRPERFENPSAIPQHAFKPFGNGQRACIGQQFALHEATLVLGMMLKHFDFEDHTNYELDIKETLTLKPEGFVVKAKSKKIPLPPPPRTGPPPPRAQVQLVESGGSLVQPGGSLRLSCAASGRFAESSSMGWFRQAPGKEREFVAAISWSGGATNYADSAKGRFTLSRDNTKNTVYLQMNSLKPDDTAVYYCAANLGNYISSNQRLYGYWGQGTQVTVS

SEQ ID NO: 237 - protein, 4 aa, Artificial Sequence
  General linker used for protein fusions, including direct fusions of CGUs to achieve the nanometer sizes of a structural element
GGSG

SEQ ID NO: 238 - protein, 201 aa, Artificial Sequence
  myristoyl switch motif for calicum-rependent relocalization a structural element such as vaults to the membrane
GNSKSGALSKEILEELQLNTKFTEEELSSWYQSFLKECPSGRITRQEFQTIYSKFFPEADPKAYAQHVFRSFDANSDGTLDFKEYVIALHMTSAGKTNQKLEWAFSLYDVDGNGTISKNEVLEIVTAIFKMISPEDTKHLPEDENTPEKRAEKIWGFFGKKDDDKLTEKEFIEGTLANKEILRLIQFEPQKVKEKLKEKKL

SEQ ID NO: 239 - protein, 15 aa, Artificial Sequence
  synthide-2 binding for FHA2
PLARALTVAGLPGKK